European Patent Specification EP 4 011 206 B1, published November 1, 2023. Title: DYSTROPHIN MEMBRANE-BINDING DOMAINS (MBDSs) AND R16/17-SYNTROPHIN PDZ FUSION PROTEINS. Applicant: University of Missouri-Columbia. The sequence listing filed with the application follows.

SEQUENCE LISTING (67 sequences)

SEQ ID NO: 1 - protein, 3685 aa, Homo sapiens
MLWWEEVEDCYEREDVQKKTFTKWVNAQFSKFGKQHIENLFSDLQDGRRLLDLLEGLTGQKLPKEKGSTRVHALNNVNKALRVLQNNNVDLVNIGSTDIVDGNHKLTLGLIWNIILHWQVKNVMKNIMAGLQQTNSEKILLSWVRQSTRNYPQVNVINFTTSWSDGLALNALIHSHRPDLFDWNSVVCQQSATQRLEHAFNIARYQLGIEKLLDPEDVDTTYPDKKSILMYITSLFQVLPQQVSIEAIQEVEMLPRPPKVTKEEHFQLHHQMHYSQQITVSLAQGYERTSSPKPRFKSYAYTQAAYVTTSDPTRSPFPSQHLEAPEDKSFGSSLMESEVNLDRYQTALEEVLSWLLSAEDTLQAQGEISNDVEVVKDQFHTHEGYMMDLTAHQGRVGNILQLGSKLIGTGKLSEDEETEVQEQMNLLNSRWECLRVASMEKQSNLHRVLMDLQNQKLKELNDWLTKTEERTRKMEEEPLGPDLEDLKRQVQQHKVLQEDLEQEQVRVNSLTHMVVVVDESSGDHATAALEEQLKVLGDRWANICRWTEDRWVLLQDILLKWQRLTEEQCLFSAWLSEKEDAVNKIHTTGFKDQNEMLSSLQKLAVLKADLEKKKQSMGKLYSLKQDLLSTLKNKSVTQKTEAWLDNFARCWDNLVQKLEKSTAQISQAVTTTQPSLTQTTVMETVTTVTTREQILVKHAQEELPPPPPQKKRQITVDSEIRKRLDVDITELHSWITRSEAVLQSPEFAIFRKEGNFSDLKEKVNAIEREKAEKFRKLQDASRSAQALVEQMVNEGVNADSIKQASEQLNSRWIEFCQLLSERLNWLEYQNNIIAFYNQLQQLEQMTTTAENWLKIQPTTPSEPTAIKSQLKICKDEVNRLSGLQPQIERLKIQSIALKEKGQGPMFLDADFVAFTNHFKQVFSDVQAREKELQTIFDTLPPMRYQETMSAIRTWVQQSETKLSIPQLSVTDYEIMEQRLGELQALQSSLQEQQSGLYYLSTTVKEMSKKAPSEISRKYQSEFEEIEGRWKKLSSQLVEHCQKLEEQMNKLRKIQNHIQTLKKWMAEVDVFLKEEWPALGDSEILKKQLKQCRLLVSDIQTIQPSLNSVNEGGQKIKNEAEPEFASRLETELKELNTQWDHMCQQVYARKEALKGGLEKTVSLQKDLSEMHEWMTQAEEEYLERDFEYKTPDELQKAVEEMKRAKEEAQQKEAKVKLLTESVNSVIAQAPPVAQEALKKELETLTTNYQWLCTRLNGKCKTLEEVWACWHELLSYLEKANKWLNEVEFKLKTTENIPGGAEEISEVLDSLENLMRHSEDNPNQIRILAQTLTDGGVMDELINEELETFNSRWRELHEEAVRRQKLLEQSIQSAQETEKSLHLIQESLTFIDKQLAAYIADKVDAAQMPQEAQKIQSDLTSHEISLEEMKKHNQGKEAAQRVLSQIDVAQKKLQDVSMKFRLFQKPANFELRLQESKMILDEVKMHLPALETKSVEQEVVQSQLNHCVNLYKSLSEVKSEVEMVIKTGRQIVQKKQTENPKELDERVTALKLHYNELGAKVTERKQQLEKCLKLSRKMRKEMNVLTEWLAATDMELTKRSAVEGMPSNLDSEVAWGKATQKEIEKQKVHLKSITEVGEALKTVLGKKETLVEDKLSLLNSNWIAVTSRAEEWLNLLLEYQKHMETFDQNVDHITKWIIQADTLLDESEKKKPQQKEDVLKRLKAELNDIRPKVDSTRDQAANLMANRGDHCRKLVEPQISELNHRFAAISHRIKTGKASIPLKELEQFNSDIQKLLEPLEAEIQQGVNLKEEDFNKDMNEDNEGTVKELLQRGDNLQQRITDERKREEIKIKQQLLQTKHNALKDLRSQRRKKALEISHQWYQYKRQADDLLKCLDDIEKKLASLPEPRDERKIKEIDRELQKKKEELNAVRRQAEGLSEDGAAMAVEPTQIQLSKRWREIESKFAQFRRLNFAQIHTVREETMMVMTEDMPLEISYVPSTYLTEITHVSQALLEVEQLLNAPDLCAKDFEDLFKQEESLKNIKDSLQQSSGRIDIIHSKKTAALQSATPVERVKLQEALSQLDFQWEKVNKMYKDRQGRFDRSVEKWRRFHYDIKIFNQWLTEAEQFLRKTQIPENWEHAKYKWYLKELQDGIGQRQTVVRTLNATGEEIIQQSSKTDASILQEKLGSLNLRWQEVCKQLSDRKKRLEEQKNILSEFQRDLNEFVLWLEEADNIASIPLEPGKEQQLKEKLEQVKLLVEELPLRQGILKQLNETGGPVLVSAPISPEEQDKLENKLKQTNLQWIKVSRALPEKQGEIEAQIKDLGQLEKKLEDLEEQLNHLLLWLSPIRNQLEIYNQPNQEGPFDVQETEIAVQAKQPDVEEILSKGQHLYKEKPATQPVKRKLEDLSSEWKAVNRLLQELRAKQPDLAPGLTTIGASPTQTVTLVTQPVVTKETAISKLEMPSSLMLEVPALADFNRAWTELTDWLSLLDQVIKSQRVMVGDLEDINEMIIKQKATMQDLEQRRPQLEELITAAQNLKNKTSNQEARTIITDRIERIQNQWDEVQEHLQNRRQQLNEMLKDSTQWLEAKEEAEQVLGQARAKLESWKEGPYTVDAIQKKITETKQLAKDLRQWQTNVDVANDLALKLLRDYSADDTRKVHMITENINASWRSIHKRVSEREAALEETHRLLQQFPLDLEKFLAWLTEAETTANVLQDATRKERLLEDSKGVKELMKQWQDLQGEIEAHTDVYHNLDENSQKILRSLEGSDDAVLLQRRLDNMNFKWSELRKKSLNIRSHLEASSDQWKRLHLSLQELLVWLQLKDDELSRQAPIGGDFPAVQKQNDVHRAFKRELKTKEPVIMSTLETVRIFLTEQPLEGLEKLYQEPRELPPEERAQNVTRLLRKQAEEVNTEWEKLNLHSADWQRKIDETLERLQELQEATDELDLKLRQAEVIKGSWQPVGDLLIDSLQDHLEKVKALRGEIAPLKENVSHVNDLARQLTTLGIQLSPYNLSTLEDLNTRWKLLQVAVEDRVRQLHEAHRDFGPASQHFLSTSVQGPWERAISPNKVPYYINHETQTTCWDHPKMTELYQSLADLNNVRFSAYRTAMKLRRLQKALCLDLLSLSAACDALDQHNLKQNDQPMDILQIINCLTTIYDRLEQEHNNLVNVPLCVDMCLNWLLNVYDTGRTGRIRVLSFKTGIISLCKAHLEDKYRYLFKQVASSTGFCDQRRLGLLLHDSIQIPRQLGEVASFGGSNIEPSVRSCFQFANNKPEIEAALFLDWMRLEPQSMVWLPVLHRVAAAETAKHQAKCNICKECPIIGFRYRSLKHFNYDICQSCFFSGRVAKGHKMHYPMVEYCTPTTSGEDVRDFAKVLKNKFRTKRYFAKHPRMGYLPVQTVLEGDNMETPVTLINFWPVDSAPASSPQLSHDDTHSRIEHYASRLAEMENSNGSYLNDSISPNESIDDEHLLIQHYCQSLNQDSPLSQPRSPAQILISLESEERGELERILADLEEENRNLQAEYDRLKQQHEHKGLSPLPSPPEMMPTSPQSPRDAELIAEAKLLRQHKGRLEARMQILEDHNKQLESQLHRLRQLLEQPQAEAKVNGTTVSSPSTSLQRSDSSQPMLLRVVGSQTSDSMGEEDLLSPPQDTSTGLEEVMEQLNNSFPSSRGRNTPGKPMREDTM

SEQ ID NO: 2 - DNA, 11058 bp, Homo sapiens
atgctttggtgggaagaagtagaggactgttatgaaagagaagatgttcaaaagaaaacattcacaaaatgggtaaatgcacaattttctaagtttgggaagcagcatattgagaacctcttcagtgacctacaggatgggaggcgcctcctagacctcctcgaaggcctgacagggcaaaaactgccaaaagaaaaaggatccacaagagttcatgccctgaacaatgtcaacaaggcactgcgggttttgcagaacaataatgttgatttagtgaatattggaagtactgacatcgtagatggaaatcataaactgactcttggtttgatttggaatataatcctccactggcaggtcaaaaatgtaatgaaaaatatcatggctggattgcaacaaaccaacagtgaaaagattctcctgagctgggtccgacaatcaactcgtaattatccacaggttaatgtaatcaacttcaccaccagctggtctgatggcctggctttgaatgctctcatccatagtcataggccagacctatttgactggaatagtgtggtttgccagcagtcagccacacaacgactggaacatgcattcaacatcgccagatatcaattaggcatagagaaactactcgatcctgaagatgttgataccacctatccagataagaagtccatcttaatgtacatcacatcactcttccaagttttgcctcaacaagtgagcattgaagccatccaggaagtggaaatgttgccaaggccacctaaagtgactaaagaagaacattttcagttacatcatcaaatgcactattctcaacagatcacggtcagtctagcacagggatatgagagaacttcttcccctaagcctcgattcaagagctatgcctacacacaggctgcttatgtcaccacctctgaccctacacggagcccatttccttcacagcatttggaagctcctgaagacaagtcatttggcagttcattgatggagagtgaagtaaacctggaccgttatcaaacagctttagaagaagtattatcgtggcttctttctgctgaggacacattgcaagcacaaggagagatttctaatgatgtggaagtggtgaaagaccagtttcatactcatgaggggtacatgatggatttgacagcccatcagggccgggttggtaatattctacaattgggaagtaagctgattggaacaggaaaattatcagaagatgaagaaactgaagtacaagagcagatgaatctcctaaattcaagatgggaatgcctcagggtagctagcatggaaaaacaaagcaatttacatagagttttaatggatctccagaatcagaaactgaaagagttgaatgactggctaacaaaaacagaagaaagaacaaggaaaatggaggaagagcctcttggacctgatcttgaagacctaaaacgccaagtacaacaacataaggtgcttcaagaagatctagaacaagaacaagtcagggtcaattctctcactcacatggtggtggtagttgatgaatctagtggagatcacgcaactgctgctttggaagaacaacttaaggtattgggagatcgatgggcaaacatctgtagatggacagaagaccgctgggttcttttacaagacatccttctcaaatggcaacgtcttactgaagaacagtgcctttttagtgcatggctttcagaaaaagaagatgcagtgaacaagattcacacaactggctttaaagatcaaaatgaaatgttatcaagtcttcaaaaactggccgttttaaaagcggatctagaaaagaaaaagcaatccatgggcaaactgtattcactcaaacaagatcttctttcaacactgaagaataagtcagtgacccagaagacggaagcatggctggataactttgcccggtgttgggataatttagtccaaaaacttgaaaagagtacagcacagatttcacaggctgtcaccaccactcagccatcactaacacagacaactgtaatggaaacagtaactacggtgaccacaagggaacagatcctggtaaagcatgctcaagaggaacttccaccaccacctccccaaaagaagaggcagattactgtggattctgaaattaggaaaaggttggatgttgatataactgaacttcacagctggattactcgctcagaagctgtgttgcagagtcctgaatttgcaatctttcggaaggaaggcaacttctcagacttaaaagaaaaagtcaatgccatagagcgagaaaaagctgagaagttcagaaaactgcaagatgccagcagatcagctcaggccctggtggaacagatggtgaatgagggtgttaatgcagatagcatcaaacaagcctcagaacaactgaacagccggtggatcgaattctgccagttgctaagtgagagacttaactggctggagtatcagaacaacatcatcgctttctataatcagctacaacaattggagcagatgacaactactgctgaaaactggttgaaaatccaacccaccaccccatcagagccaacagcaattaaaagtcagttaaaaatttgtaaggatgaagtcaaccggctatcaggtcttcaacctcaaattgaacgattaaaaattcaaagcatagccctgaaagagaaaggacaaggacccatgttcctggatgcagactttgtggcctttacaaatcattttaagcaagtcttttctgatgtgcaggccagagagaaagagctacagacaatttttgacactttgccaccaatgcgctatcaggagaccatgagtgccatcaggacatgggtccagcagtcagaaaccaaactctccatacctcaacttagtgtcaccgactatgaaatcatggagcagagactcggggaattgcaggctttacaaagttctctgcaagagcaacaaagtggcctatactatctcagcaccactgtgaaagagatgtcgaagaaagcgccctctgaaattagccggaaatatcaatcagaatttgaagaaattgagggacgctggaagaagctctcctcccagctggttgagcattgtcaaaagctagaggagcaaatgaataaactccgaaaaattcagaatcacatacaaaccctgaagaaatggatggctgaagttgatgtttttctgaaggaggaatggcctgcccttggggattcagaaattctaaaaaagcagctgaaacagtgcagacttttagtcagtgatattcagacaattcagcccagtctaaacagtgtcaatgaaggtgggcagaagataaagaatgaagcagagccagagtttgcttcgagacttgagacagaactcaaagaacttaacactcagtgggatcacatgtgccaacaggtctatgccagaaaggaggccttgaagggaggtttggagaaaactgtaagcctccagaaagatctatcagagatgcacgaatggatgacacaagctgaagaagagtatcttgagagagattttgaatataaaactccagatgaattacagaaagcagttgaagagatgaagagagctaaagaagaggcccaacaaaaagaagcgaaagtgaaactccttactgagtctgtaaatagtgtcatagctcaagctccacctgtagcacaagaggccttaaaaaaggaacttgaaactctaaccaccaactaccagtggctctgcactaggctgaatgggaaatgcaagactttggaagaagtttgggcatgttggcatgagttattgtcatacttggagaaagcaaacaagtggctaaatgaagtagaatttaaacttaaaaccactgaaaacattcctggcggagctgaggaaatctctgaggtgctagattcacttgaaaatttgatgcgacattcagaggataacccaaatcagattcgcatattggcacagaccctaacagatggcggagtcatggatgagctaatcaatgaggaacttgagacatttaattctcgttggagggaactacatgaagaggctgtaaggaggcaaaagttgcttgaacagagcatccagtctgcccaggagactgaaaaatccttacacttaatccaggagtccctcacattcattgacaagcagttggcagcttatattgcagacaaggtggacgcagctcaaatgcctcaggaagcccagaaaatccaatctgatttgacaagtcatgagatcagtttagaagaaatgaagaaacataatcaggggaaggaggctgcccaaagagtcctgtctcagattgatgttgcacagaaaaaattacaagatgtctccatgaagtttcgattattccagaaaccagccaattttgagctgcgtctacaagaaagtaagatgattttagatgaagtgaagatgcacttgcctgcattggaaacaaagagtgtggaacaggaagtagtacagtcacagctaaatcattgtgtgaacttgtataaaagtctgagtgaagtgaagtctgaagtggaaatggtgataaagactggacgtcagattgtacagaaaaagcagacggaaaatcccaaagaacttgatgaaagagtaacagctttgaaattgcattataatgagctgggagcaaaggtaacagaaagaaagcaacagttggagaaatgcttgaaattgtcccgtaagatgcgaaaggaaatgaatgtcttgacagaatggctggcagctacagatatggaattgacaaagagatcagcagttgaaggaatgcctagtaatttggattctgaagttgcctggggaaaggctactcaaaaagagattgagaaacagaaggtgcacctgaagagtatcacagaggtaggagaggccttgaaaacagttttgggcaagaaggagacgttggtggaagataaactcagtcttctgaatagtaactggatagctgtcacctcccgagcagaagagtggttaaatcttttgttggaataccagaaacacatggaaacttttgaccagaatgtggaccacatcacaaagtggatcattcaggctgacacacttttggatgaatcagagaaaaagaaaccccagcaaaaagaagacgtgcttaagcgtttaaaggcagaactgaatgacatacgcccaaaggtggactctacacgtgaccaagcagcaaacttgatggcaaaccgcggtgaccactgcaggaaattagtagagccccaaatctcagagctcaaccatcgatttgcagccatttcacacagaattaagactggaaaggcctccattcctttgaaggaattggagcagtttaactcagatatacaaaaattgcttgaaccactggaggctgaaattcagcagggggtgaatctgaaagaggaagacttcaataaagatatgaatgaagacaatgagggtactgtaaaagaattgttgcaaagaggagacaacttacaacaaagaatcacagatgagagaaagagagaggaaataaagataaaacagcagctgttacagacaaaacataatgctctcaaggatttgaggtctcaaagaagaaaaaaggctctagaaatttctcatcagtggtatcagtacaagaggcaggctgatgatctcctgaaatgcttggatgacattgaaaaaaaattagccagcctacctgagcccagagatgaaaggaaaataaaggaaattgatcgggaattgcagaagaagaaagaggagctgaatgcagtgcgtaggcaagctgagggcttgtctgaggatggggccgcaatggcagtggagccaactcagatccagctcagcaagcgctggcgggaaattgagagcaaatttgctcagtttcgaagactcaactttgcacaaattcacactgtccgtgaagaaacgatgatggtgatgactgaagacatgcctttggaaatttcttatgtgccttctacttatttgactgaaatcactcatgtctcacaagccctattagaagtggaacaacttctcaatgctcctgacctctgtgctaaggactttgaagatctctttaagcaagaggagtctctgaagaatataaaagatagtctacaacaaagctcaggtcggattgacattattcatagcaagaagacagcagcattgcaaagtgcaacgcctgtggaaagggtgaagctacaggaagctctctcccagcttgatttccaatgggaaaaagttaacaaaatgtacaaggaccgacaagggcgatttgacagatctgttgagaaatggcggcgttttcattatgatataaagatatttaatcagtggctaacagaagctgaacagtttctcagaaagacacaaattcctgagaattgggaacatgctaaatacaaatggtatcttaaggaactccaggatggcattgggcagcggcaaactgttgtcagaacattgaatgcaactggggaagaaataattcagcaatcctcaaaaacagatgccagtattctacaggaaaaattgggaagcctgaatctgcggtggcaggaggtctgcaaacagctgtcagacagaaaaaagaggctagaagaacaaaagaatatcttgtcagaatttcaaagagatttaaatgaatttgttttatggttggaggaagcagataacattgctagtatcccacttgaacctggaaaagagcagcaactaaaagaaaagcttgagcaagtcaagttactggtggaagagttgcccctgcgccagggaattctcaaacaattaaatgaaactggaggacccgtgcttgtaagtgctcccataagcccagaagagcaagataaacttgaaaataagctcaagcagacaaatctccagtggataaaggtttccagagctttacctgagaaacaaggagaaattgaagctcaaataaaagaccttgggcagcttgaaaaaaagcttgaagaccttgaagagcagttaaatcatctgctgctgtggttatctcctattaggaatcagttggaaatttataaccaaccaaaccaagaaggaccatttgacgttcaggaaactgaaatagcagttcaagctaaacaaccggatgtggaagagattttgtctaaagggcagcatttgtacaaggaaaaaccagccactcagccagtgaagaggaagttagaagatctgagctctgagtggaaggcggtaaaccgtttacttcaagagctgagggcaaagcagcctgacctagctcctggactgaccactattggagcctctcctactcagactgttactctggtgacacaacctgtggttactaaggaaactgccatctccaaactagaaatgccatcttccttgatgttggaggtacctgctctggcagatttcaaccgggcttggacagaacttaccgactggctttctctgcttgatcaagttataaaatcacagagggtgatggtgggtgaccttgaggatatcaacgagatgatcatcaagcagaaggcaacaatgcaggatttggaacagaggcgtccccagttggaagaactcattaccgctgcccaaaatttgaaaaacaagaccagcaatcaagaggctagaacaatcattacggatcgaattgaaagaattcagaatcagtgggatgaagtacaagaacaccttcagaaccggaggcaacagttgaatgaaatgttaaaggattcaacacaatggctggaagctaaggaagaagctgagcaggtcttaggacaggccagagccaagcttgagtcatggaaggagggtccctatacagtagatgcaatccaaaagaaaatcacagaaaccaagcagttggccaaagacctccgccagtggcagacaaatgtagatgtggcaaatgacttggccctgaaacttctccgggattattctgcagatgataccagaaaagtccacatgataacagagaatatcaatgcctcttggagaagcattcataaaagggtgagtgagcgagaggctgctttggaagaaactcatagattactgcaacagttccccctggacctggaaaagtttcttgcctggcttacagaagctgaaacaactgccaatgtcctacaggatgctacccgtaaggaaaggctcctagaagactccaagggagtaaaagagctgatgaaacaatggcaagacctccaaggtgaaattgaagctcacacagatgtttatcacaacctggatgaaaacagccaaaaaatcctgagatccctggaaggttccgatgatgcagtcctgttacaaagacgtttggataacatgaacttcaagtggagtgaacttcggaaaaagtctctcaacattaggtcccatttggaagccagttctgaccagtggaagcgtctgcacctttctctgcaggaacttctggtgtggctacagctgaaagatgatgaattaagccggcaggcacctattggaggcgactttccagcagttcagaagcagaacgatgtacatagggccttcaagagggaattgaaaactaaagaacctgtaatcatgagtactcttgagactgtacgaatatttctgacagagcagcctttggaaggactagagaaactctaccaggagcccagagagctgcctcctgaggagagagcccagaatgtcactcggcttctacgaaagcaggctgaggaggtcaatactgagtgggaaaaattgaacctgcactccgctgactggcagagaaaaatagatgagacccttgaaagactccaggaacttcaagaggccacggatgagctggacctcaagctgcgccaagctgaggtgatcaagggatcctggcagcccgtgggcgatctcctcattgactctctccaagatcacctcgagaaagtcaaggcacttcgaggagaaattgcgcctctgaaagagaacgtgagccacgtcaatgaccttgctcgccagcttaccactttgggcattcagctctcaccgtataacctcagcactctggaagacctgaacaccagatggaagcttctgcaggtggccgtcgaggaccgagtcaggcagctgcatgaagcccacagggactttggtccagcatctcagcactttctttccacgtctgtccagggtccctgggagagagccatctcgccaaacaaagtgccctactatatcaaccacgagactcaaacaacttgctgggaccatcccaaaatgacagagctctaccagtctttagctgacctgaataatgtcagattctcagcttataggactgccatgaaactccgaagactgcagaaggccctttgcttggatctcttgagcctgtcagctgcatgtgatgccttggaccagcacaacctcaagcaaaatgaccagcccatggatatcctgcagattattaattgtttgaccactatttatgaccgcctggagcaagagcacaacaatttggtcaacgtccctctctgcgtggatatgtgtctgaactggctgctgaatgtttatgatacgggacgaacagggaggatccgtgtcctgtcttttaaaactggcatcatttccctgtgtaaagcacatttggaagacaagtacagataccttttcaagcaagtggcaagttcaacaggattttgtgaccagcgcaggctgggcctccttctgcatgattctatccaaattccaagacagttgggtgaagttgcatcctttgggggcagtaacattgagccaagtgtccggagctgcttccaatttgctaataataagccagagatcgaagcggccctcttcctagactggatgagactggaaccccagtccatggtgtggctgcccgtcctgcacagagtggctgctgcagaaactgccaagcatcaggccaaatgtaacatctgcaaagagtgtccaatcattggattcaggtacaggagtctaaagcactttaattatgacatctgccaaagctgctttttttctggtcgagttgcaaaaggccataaaatgcactatcccatggtggaatattgcactccgactacatcaggagaagatgttcgagactttgccaaggtactaaaaaacaaatttcgaaccaaaaggtattttgcgaagcatccccgaatgggctacctgccagtgcagactgtcttagagggggacaacatggaaactcccgttactctgatcaacttctggccagtagattctgcgcctgcctcgtcccctcagctttcacacgatgatactcattcacgcattgaacattatgctagcaggctagcagaaatggaaaacagcaatggatcttatctaaatgatagcatctctcctaatgagagcatagatgatgaacatttgttaatccagcattactgccaaagtttgaaccaggactcccccctgagccagcctcgtagtcctgcccagatcttgatttccttagagagtgaggaaagaggggagctagagagaatcctagcagatcttgaggaagaaaacaggaatctgcaagcagaatatgaccgtctaaagcagcagcacgaacataaaggcctgtccccactgccgtcccctcctgaaatgatgcccacctctccccagagtccccgggatgctgagctcattgctgaggccaagctactgcgtcaacacaaaggccgcctggaagccaggatgcaaatcctggaagaccacaataaacagctggagtcacagttacacaggctaaggcagctgctggagcaaccccaggcagaggccaaagtgaatggcacaacggtgtcctctccttctacctctctacagaggtccgacagcagtcagcctatgctgctccgagtggttggcagtcaaacttcggactccatgggtgaggaagatcttctcagtcctccccaggacacaagcacagggttagaggaggtgatggagcaactcaacaactccttccctagttcaagaggaagaaatacccctggaaagccaatgagagaggacacaatgtag

SEQ ID NO: 3 - DNA, 5953 bp, Artificial Sequence
  Synthetic
atgctttggtgggaagaagtagaggactgttatgaaagagaagatgttcaaaagaaaacattcacaaaatgggtaaatgcacaattttctaagtttgggaagcagcatattgagaacctcttcagtgacctacaggatgggaggcgcctcctagacctcctcgaaggcctgacagggcaaaaactgccaaaagaaaaaggatccacaagagttcatgccctgaacaatgtcaacaaggcactgcgggttttgcagaacaataatgttgatttagtgaatattggaagtactgacatcgtagatggaaatcataaactgactcttggtttgatttggaatataatcctccactggcaggtcaaaaatgtaatgaaaaatatcatggctggattgcaacaaaccaacagtgaaaagattctcctgagctgggtccgacaatcaactcgtaattatccacaggttaatgtaatcaacttcaccaccagctggtctgatggcctggctttgaatgctctcatccatagtcataggccagacctatttgactggaatagtgtggtttggcagcagtcagccacacaacgactggaacatgcattcaacatcgccagatatcaattaggcatagagaaagtactcgatcctgaagatgttgataccacctatccagataagaagtccatcttaatgtacatcacatcactcttccaagttttgcctcaacaagtgagcattgaagccatccaggaagtggaaatgttgccaaggccacctaaagtgactaaagaagaacattttcagtacatcatcaaatgcactattctcaacagatcacggtcagtctagcacagggatatgagagaacttcttcccctaagcctcgattcaagagctatgcctacacacaggctgcttatgtcaccacctctgaccctacacggagcccatttccttcacagcatttggaagctcctgaagacaagtcatttggcagttcattgatggagagtgaagtaaacctggaccgttatcaaacagctttagaagaagtattatcgtggcttctttctgctgaggacacattgcaagcacaaggagagatttctaatgatgtggaagtggtgaaagaccagtttcatactcatgaggggtacatgatggatttgacagcccatcagggccgggttggtaatattctacaattgggaagtaagctgattggaacaggaaaattatcagaagatgaagaaactgaagtacaagagcagatgaatctcctaaattcaagatgggaatgcctcagggtagctagcatggaaaaacaaagcaatttacatagagttttaatggatctccagaatcagaaactgaaagagttgaatgactggctaacaaaaacagaagaaagaacaaggaaaatggaggaagagcctcttggacctgatcttgaagacctaaaacgccaagtacaacaacataaggtgcttcaagaagatctagaacaagaacaagtcagggtcaattctctcactcacatggtggtggtagttgatgaatctagtggagatcacgcaactgctgctttggaagaacaagtttaaggtattgggagatcgatgggcaaacatctgtagatggacagaagaccgctgggttcttttacaagacatccttctcaaatggcaacgtcttactgaagaacagtgcctttttagtgcatggctttcagaaaaagaagatgcagtgaacaagattcacacaactggctttaaagatcaaaatgaaatgttatcaagtcttcaaaaactggccgttttaaaagcggatctagaaaagaaaaagcaatccatgggcaaactgtattcactcaaacaagatcttctttcaacactgaagaataagtcagtgacccagaagacggaagcatggctggataactttgcccggtgttgggataatttagtccaaaaacttgaaaagagtacagcacaggaaactgaaatagcagttcaagctaaacaaccggatgtggaagagattttgtctaaagggcagcatttgtacaaggaaaaaccagccactcagccagtgaagaggaagttagaagatctgagctctgagtggaaggcggtaaaccgtttacttcaagagctgagggcaaagcagcctgacctagctcctggactgaccactattggagcctctcctactcagactgttactctggtgacacaacctgtggttagtaaggaaactgccatctccaaactagaaatgccatcttccttgatgttggaggtacctgctctggcagatttcaacggggcttggacagaacttaccgagtggctttctctgcttgatcaagttataaaatcacagagggtgatggtgggtgaccttgaggatatcaacgagatgatcatcaagcagaaggcaacaatgcaggatttggaacagaggcgtccccagttggaagaactcattaccgctgcccaaaatttgaaaaacaagaccagcaatcaagaggctagaacaatcattacggatcgaattgaaagaattcagaatcagtgggatgaagtacaagaacaccttcagaaccggaggcaacagttgaatgaaatgttaaaggattcaacacaatggctggaagctaaggaagaagctgagcaggtcttaggacagggcagagccaagcttgagtcatggaaggagggtccctatacagtagatgcaatccaaaagaaaatcacagaaaccaagcagttggccaaagacctccgccagtggcagacaaatgtagatgtggcaaatgacttggccctgaaacttctccgggattattctgcagatgataccagaaaagtccacatgataacagagaatatcaatgcctcttggagaagcattcataaaagggtgagtgagcgagaggctgctttggaagaaactcatagattactgcaacagttccccctggacctggaaaagtttcttgcctggcttacagaagctgaaacaactgccaatgtcctacaggatgctacccgtaaggaaaggctcctagaagactccaagggagtaaaagagctgatgaaacaatggcaagacctccaaggtgaaattgaagctcacacagatgtttatcacaacctggatgaaaacagccaaaaaatcctgagatccctggaaggttccgatgatgcagtcctgttacaaagacgtttggataacatgaacttcaagtggagtgaacttcggaaaaagtctctcaacattaggtcccatttggaagccagttctgaccagtggaagcgtctgcacctttctctgcaggaacttctggtgtggctacagctgaaagatgatgaattaagccggcaggcacctattggaggcgactttccagcagttcagaagcagaacgatgtacatagggccttcaagagggaattgaaaactaaagaacctgtaatcatgagtactcttgagactgtacgaatatttctgacagagcagcctttggaaggactagagaaactctaccaggagcccagagagctgcctcctgaggagagagcccagaatgtcactcggcttctacgaaagcaggctgaggaggtcaatactgagtgggaaaaattgaacctgcactccgctgactggcagagaaaaatagatgagacccttgaaagactccaggaacttcaagaggccacggatgagctggacctcaagctgcgccaagctgaggtgatcaagggatcctggcagcccgtgggcgatctcctcattgactctctccaagatcacctcgagaaagtcaaggcacttcgaggagaaattgcgcctctgaaagagaacgtgagccacgtcaatgaccttgctcgccagcttaccactttgggcattcagctctcaccgtataacctcagcactctggaagacctgaacaccagatggaagcttctgcaggtggccgtcgaggaccgagtcaggcagctgcatgaagcccacagggactttggtccagcatctcagcactttctttccacgtctgtccagggtcggtgggagagagccatctcgccaaacaaagtgccctactatatcaaccacgagactcaaacaacttgctgggaccatcccaaaatgacagagctctaccagtctttagctgacctgaataatgtcagattctcagcttataggactgccatgaaactccgaagactgcagaaggccctttgcttggatctcttgagcctgtcagctgcatgtgatgccttggaccagcacaacctcaagcaaaatgaccagcccatggatatcctgcagattattaattgtttgaccactatttatgaccgcctggagcaagagcacaacaatttggtcaacgtccctctctgcgtggatatgtgtctgaactggctgctgaatgtttatgatacgggacgaacagggaggatccgtgtcctgtcttttaaaactggcatcatttccctgtgtaaagcacatttggaagacaagtacagataccttttcaagcaagtggcaagttcaacaggattttgtgaccagcgcaggctgggcctccttctgcatgattctatccaaattccaagacagttgggtgaagttgcatcctttgggggcagtaacattgagccaagtgtccggagctgcttccaatttgctaataataagccagagatcgaagcggccctcttcctagactggatgagactggaaccccagtccatggtgtggctgcccgtcctgcacagagtggctgctgcagaaactgccaagcatcaggccaaatgtaacatctgcaaagagtgtccaatcattggattcaggtacaggagtctaaagcactttaattatgacatctgccaaagctgctttttttctggtcgagttgcaaaaggccataaaatgcactatcccatggtggaatattgcactccgactacatcaggagaagatgttcgagactttgccaaggtactaaaaaacaaatttcgaaccaaaaggtattttgcgaagcatccccgaatgggctacctgccagtgcagactgtcttagagggggacaacatggaaactcccgttactctgatcaacttctggccagtagattctgcgcctgcctcgtcccctcagctttcacacgatgatactcattcacgcattgaacattatgctagcaggctagcagaaatggaaaacagcaatggatcttatctaaatgatagcatctctcctaatgagagcatagatgatgaacatttgttaatccagcattactgccaaagtttgaaccaggactcccccctgagccagcctcgtagtcctgcccagatcttgatttccttagagagtgaggaaagaggggagctagagagaatcctagcagatcttgaggaagaaaacaggaatctgcaagcagaatatgaccgtctaaagcagcagcacgaacataaaggcctgtccccactgccgtcccctcctgaaatgatgcccacctctccccagagtccccgggatgctgagctcattgctgaggccaagctactgcgtcaacacaaaggccgcctggaagccaggatgcaaatcctggaagaccacaataaacagctggagtcacagttacacaggctaaggcaggtgctggagcaaccccaggcagaggccaaagtgaatggcacaacggtgtcctctccttctacctctctacagaggtccgacagcagtcagcctatgctgctccgagtggttggcagtcaaacttcggactccatgggtgaggaagatcttctcagtcgtccccaggacacaagcacagggttagaggaggtgatggagcaactcaacaactcctttccctagttcaagaggaagaaatacccctggaaagccaatgagagaggacacaatgtag

SEQ ID NO: 4 - DNA, 5749 bp, Artificial Sequence
  Synthetic
atgcttggtgggaagaagtagaggactgttatgaaagagaagatgttcaaaagaaaacattcacaaaatgggtaaatgcacaattttctaagtttgggaagcagcatattgagaacctcttcagtgacctacaggatgggaggcgcctcctagacctcctcgaaggcctgacagggcaaaaactgccaaaagaaaaaggatccacaagagttcatgccctgaacaatgtcaacaaggcactgcgggttttgcagaacaataatgttgatttagtgaatattggaagtactgacatcgtagatggaaatcataaactgactcttggtttgatttggaatataatcctccactggcaggtcaaaaatgtaatgaaaaatatcatggctggattgcaacaaaccaacagtgaaaagattctcctgagctgggtgcgacaatcaactcgtaattatccacaggttaatgtaatcaacttcaccaccagctggtctgatggcctggctttgaatgctctcatccatagtcataggccagacctatttgactggaatagtgtggtttgccagcagtcagccacacaacgactggaacatgcattcaacatcgccagatatcaattaggcatagagaaactactcgatcctgaagatgttgataccacctatccagataagaagtccatctttaatgtacatcacatcactcttccaagttttgcctcaacaagtgagcattgaagccatccaggaagtggaaatgttgccaaggccacctaaagtgactaaagaagaacattttcagttacatcatcaaatgcactattctcaacagatcacggtcagtctagcacagggatatgagagaacttcttcccctaagcctcgattcaagagctatgcctacacacaggctgcttatgtcaccacctctgaccctacacggagcccatttccttcacagcatttggaagctcctgaagacaagtcatttggcagttcattgatggagagtgaagtaaacctggaccgttatcaaacagctttagaagaagtattatcgtggcttctttctgctgaggacacattgcaagcacaaggagagatttctaatgatgtggaagtggtgaaagaccagtttcatactcatgaggggtacatgatggatttgacagcccatcagggccgggttggtaatattctacaattgggaagtaagctgattggaacaggaaaattatcagaagatgaagaaactgaagtacaagagcagatgaatctcctaaattcaagatgggaatgcctcagggtagctagcatggaaaaacaaagcaatttacatagagttttaatggatctccagaatcagaaactgaaagagttgaatgactggctaacaaaaacagaagaaagaacaaggaaaatggaggaagagcctcttggacctgatcttgaagacctaaaacgccaagtacaacaacataaggtgcttcaagaagatctagaacaagaacaagtcagggtcaattctctcactcacatggtggtggtagttgatgaatctagtggagatcacgcaactgctgctttggaagaacaacttaaggtattgggagatcgatgggcaaacatctgtagatggacagaagaccgctgggttcttttacaagacatccttctcaaatgggaacgtcttactgaagaacagtgcctttttagtgcatggctttcagaaaaagaagatgcagtgaacaagattcacacaactggctttaaagatcaaaatgaaatgttatcaagtcttcaaaaactggccgttttaaaagcggatctagaaaagaaaaagcaatccatgggcaaactgtattcactcaaacaagatcttctttcaacactgaagaataagtcagtgacccagaagacggaagcatggctggataactttgcccggtgttgggataatttagtccaaaaacttgaaaagagtacagcacagatttcacagcagcctgacctagctcctggactgaccactattggagcctctcctactcagactgttactctggtgacacaacctgtggttactaaggaaactgccatctccaaactagaaatgccatcttccttgatgttggaggtacctgctctggcagatttcaaccgggcttggacagaacttaccgactggctttctctgcttgatcaagttataaaatcacagagggtgatggtgggtgaccttgaggatatcaacgagatgatcatcaagcagaaggcaacaatgcaggatttggaacagaggcgtccccagttggaagaactcattaccgctgcccaaaatttgaaaaacaagaccagcaatcaagaggctagaacaatcattacggatcgaattgaaagaattcagaatcagtgggatgaagtacaagaacaccttcagaaccggaggcaacagttgaatgaaatgttaaaggattcaacacaatggctggaagctaaggaagaagctgagcaggtcttaggacaggccagagccaagcttgagtcatggaaggagggtccctatacagtagatgcaatccaaaagaaaatcacagaaaccaagcagttggccaaagacctccgcgagtggcagacaaatgtagatgtggcaaatgacttggccctgaaacttctgcgggattattctgcagatgataccagaaaagtccacatgataacagagaatatcaatgcctcttggagaagcattcataaaagggtgagtgagcgagaggctgctttggaagaaactcatagattactgcaacagttccccctggacctggaaaagtttcttgcctggcttacagaagctgaaacaactgccaatgtcctacaggatgctacccgtaaggaaaggctcctagaagactccaagggagtaaaagagctgatgaaacaatggcaagacctccaaggtgaaattgaagctcacacagatgtttatgacaacctggatgaaaacagccaaaaaatcctgagatccctggaaggttccgatgatgcagtcctgttacaaagacgtttggataacatgaacttcaagtggagtgaacttcggaaaaagtctctcaacattaggtcccatttggaagccagttctgaccagtggaagcgtctgcacctttctctgcaggaacttctggtgtggctacagctgaaagatgatgaattaagccggcaggcacctattggaggcgactttccagcagttcagaagcagaacgatgtacatagggccttcaagagggaattgaaaactaaagaacctgtaatcatgagtactcttgagactgtacgaatatttctgacagagcagcctttggaaggactagagaaactctaccaggagcccagagagctgcctcctgaggagagagcccagaatgtcactcggcttctacgaaagcaggctgaggaggtcaatactgagtgggaaaaattgaacctgcactccgctgactggcagagaaaaatagatgagacccttgaaagactccaggaacttcaagaggccacggatgagctggacctcaagctgcgccaagctgaggtgatcaagggatcctggcagcccgtgggcgatctcctgattgactctctccaagatcacctcgagaaagtcaaggcacttcgaggagaaattgcgcctctgaaagagaacgtgagcgacgtcaatgaccttgctcgccagcttaccactttgggcattcagctctcaccgtataacctcagcactctggaagacctgaacaccagatggaagcttctgcaggtggccgtcgaggaccgagtcaggcagctgcatgaagcccacagggactttggtccagcatctcagcactttctttccacgtctgtccagggtccctgggagagagccatctcgccaaacaaagtgccctactatatcaaccacgagactcaaacaacttgctgggaccatcccaaaatgacagagctctaccagtctttagctgacctgaataatgtcagattctcagcttataggactgccatgaaactccgaagactgcagaaggccctttgcttggatctcttgagcctgtcagctgcatgtgatgccttggaccagcacaacctcaagcaaaatgaccagcccatggatatcctgcagattattaattgtttgaccactatttatgaccgcctggagcaagagcacaacaatttggtcaacgtccctctctgcgtggatatgtgtctgaactggctgctgaatgtttatgatacgggacgaacagggaggatccgtgtcctgtctttaaaagtggcatcatttccctgtgtaaagcacatttggaagacaagtacagataccttttcaagcaagtggcaagttcaacaggattttgtgaccagcgcaggctgggcctccttctgcatgattctatccaaatccaagacagttgggtgaagttgcatcctttgggggcagtaacattgagccaagtgtccggagctgcttccaatttgctaataataagccagagatcgaagcggccctcttcctagactggatgagactggaaccccagtccatggtgtggctgcccgtcctgcacagagtggctgctggagaaactgccaagcatcaggccaaatgtaacatctgcaaagagtgtccaatcattggattcaggtacaggagtctaaagcactttaattatgacatctgccaaagctgctttttttctggtcgagttgcaaaaggccataaaatgcactatcccatggtggaatattgcactccgactacatcaggagaagatgttcgagactttgccaaggtactaaaaaacaaatttcgaaccaaaaggtattttgcgaagcatccccgaatgggctacctgccagtgcagactgtcttagagggggacaacatggaaacgcctgcctcgtcccctcagctttcacacgatgatactcattcacgcattgaacattatgctagcaggctagcagaaatggaaaacagcaatggatcttatctaaatgatagcatctctcctaatgagagcatagatgatgaacatttgttaatccagcattactgccaaagtttgaaccaggactcccccctgagccagcctcgtagtcctgcccagatcttgatttccttagagagtgaggaaagaggggagctagagagaatcctagcagatcttgaggaagaaaacaggaatctgcaagcagaatatgaccgtctaaagcagcagcacgaacataaaggcctgtccccactgccgtcccctcctgaaatgatgcccacctctccccagagtccccgggatgctgagctcattgctgaggccaagctactgcgtcaacacaaaggccgcctggaagccaggatgcaaatcctggaagaccacaataaacagctggagtcacagttacacaggctaaggcagctgctggagcaaccccaggcagaggccaaagtgaatggcacaacggtgtcctctccttctacctctctacagaggtccgacagcagtcagcctatgctgctccgagtggttggcagtcaaacttcggactccatgggtgaggaagatcttctcagtcctccccaggacacaagcacagggttagaggaggtgatggagcaactcaacaactccttccctagttgaagaggaagaaatacccctggaaagccaatgagagaggacacaatgtag

SEQ ID NO: 5 - DNA, 6397 bp, Artificial Sequence
  Synthetic
atgctttggtgggaagaagtagaggactgttatgaaagagaagatgttcaaaagaaaacattcacaaaatgggtaaatgcacaattttctaagtttgggaagcagcatattgagaacctcttcagtgacctacaggatgggaggcgcctcctagacctcctcgaaggcctgacagggcaaaaactgccaaaagaaaaaggatccacaagagttcatgccctgaacaatgtcaacaaggcactgcgggttttgcagaacaataatgttgatttagtgaatattggaagtactgacatcgtagatggaaatcataaactgactcttggtttgatttggaatataatcctccactggcaggtcaaaaatgtaatgaaaaatatcatggctggattgcaacaaaccaacagtgaaaagattctcctgagctgggtccgacaatcaactcgtaattatccacaggttaatgtaatcaacttcaccaccagctggtctgatggcctggctttgaatgctctcatccatagtcataggccagacctatttgactggaatagtgtggtttgccagcagtcagccacacaacgactggaacatgcattcaacatcgccagatatcaattaggcatagagaaactactcgatcctgaagatgttgataccacctatccagataagaagtccatcttaatgtacatcacatcactcttccaagttttgcctcaacaagtgagcattgaagccatccaggaagtggaaatgttgccaaggccacctaaagtgactaaagaagaacattttcagttacatcatcaaatgcactattctcaacagatcacggtcagtctagcacagggatatgagagaacttcttcccctaagcctcgattcaagagctatgcctacacacaggctgcttatgtcaccacctctgaccctacacggagcccatttccttcacagcatttggaagctcctgaagacaagtcatttggcagttcattgatggagagtgaagtaaacctggaccgttatcaaacagctttagaagaagtattatcgtggcttctttctgctgaggacacattgcaagcacaaggagagatttctaatgatgtggaagtggtgaaagaccagtttcatactcatgaggggtacatgatggatttgacagcccatcagggccgggttggtaatattctacaattgggaagtaagctgattggaacaggaaaattatcagaagatgaagaaactgaagtacaagagcagatgaatctcctaaattcaagatgggaatgcctcagggtagctagcatggaaaaacaaagcaatttacatagagttttaatggatctccagaatcagaaactgaaagagttgaatgactggctaacaaaaacagaagaaagaacaaggaaaatggaggaagagcctcttggacctgatcttgaagacctaaaacgccaagtacaacaacataaggtgcttcaagaagatctagaacaagaacaagtcagggtcaattctctcactcacatggtggtggtagttgatgaatctagtggagatcacgcaactgctgctttggaagaacaacttaaggtattgggagatcgatgggcaaacatctgtagatggacagaagaccgctgggttcttttacaagacatccttctcaaatggcaacgtcttactgaagaacagtgcctttttagtgcatggctttcagaaaaagaagatgcagtgaacaagattcacacaactggctttaaagatcaaaatgaaatgttatcaagtcttcaaaaactggccgttttaaaagcggatctagaaaagaaaaagcaatccatgggcaaactgtattcactcaaacaagatcttctttcaacactgaagaataagtcagtgacccagaagacggaagcatggctggataactttgcccggtgttgggataatttagtccaaaaacttgaaaagagtacagcacagatttcacagcaaaagaatatcttgtcagaatttcaaagagatttaaatgaatttgttttatggttggaggaagcagataacattgctagtatcccacttgaacctggaaaagagcagcaactaaaagaaaagcttgagcaagtcaagttactggtggaagagttgcccctgcgccagggaattctcaaacaattaaatgaaactggaggacccgtgcttgtaagtgctcccataagcccagaagagcaagataaacttgaaaataagctcaagcagacaaatctccagtggataaaggtttccagagctttacctgagaaacaaggagaaattgaagctcaaataaaagaccttgggcagcttgaaaaaaagcttgaagaccttgaagagcagttaaatcatctgctgctgtggttatctcgtattaggaatcagttggaaatttataaccaaccaaaccaagaaggaccatttgacgttcaggaaactgaaatagcagttcaagctaaacaaccggatgtggaagagattttgtctaaagggcagcatttgtacaaggaaaaaccagccactgagccagtgaagaggaagttagaagatctgagctctgagtggaaggcggtaaaccgtttacttcaagagctgagggcaaagcagcctgacctagctcctggactgaccactattggagcctctcctactcagactgttactctggtgacacaacctgtggttactaaggaaactgccatctccaaactagaaatgccatcttccttgatgttggaggtacctgctctggcagatttcaaccgggcttggacagaacttaccgactggctttctctgcttgatcaagttataaaatcacagagggtgatggtgggtgaccttgaggatatcaacgagatgatcatcaagcagaaggcaacaatgcaggatttggaacagaggcgtccccagttggaagaactcattaccgctgcccaaaatttgaaaaacaagaccagcaatcaagaggctagaacaatcattacggatcgaattgaaagaattcagaatcagtgggatgaagtacaagaacaccttcagaaccggaggcaacagttgaatgaaatgttaaaggattcaacacaatggctggaagctaaggaagaagctgagcaggtcttaggacaggccagagccaagcttgagtcatggaaggagggtccctatacagtagatgcaatccaaaagaaaatcacagaaaccaagcagttggccaaagacctccgccagtggcagacaaatgtagatgtggcaaatgacttggccctgaaacttctccgggattattctgcagatgataccagaaaagtccacatgataacagagaatatcaatgcctcttggagaagcattcataaaagggtgagtgagcgagaggctgctttggaagaaactcatagattactgcaacagttccccctggacctggaaaagtttcttgcctggcttacagaagctgaaacaactgccaatgtcctacaggatgctacccgtaaggaaaggctcctagaagactccaagggagtaaaagagctgatgaaacaatggcaagacctccaaggtgaaattgaagctcacacagatgtttatcacaacctggatgaaaacagccaaaaaatcctgagatccctggaaggttccgatgatgcagtcctgttacaaagacgtttggataacatgaacttcaagtggagtgaacttcggaaaaagtctctcaacattaggtcccatttggaagccagttctgaccagtggaagcgtctgcacctttctctgcaggaacttctggtgtggctagagctgaaagatgatgaattaagccggcaggcacctattggaggcgactttccagcagttcagaagcagaacgatgtacatagggccttcaagagggaattgaaaactaaagaacctgtaatcatgagtactcttgagactgtacgaatatttctgacagagcagcctttggaaggactagagaaactctaccaggagcccagagagctgcctcctgaggagagagcccagaatgtcactcggcttctacgaaagcaggctgaggaggtcaatactgagtgggaaaaattgaacctgcactccgctgactggcagagaaaaatagatgagacccttgaaagactccaggaacttcaagaggccacggatgagctggacctcaagctgcgccaagctgaggtgatcaagggatcctggcagccggtgggcgatctcctcattgactctctccaagatcacctcgagaaagtcaaggcacttcgaggagaaattgcgcctctgaaagagaacgtgagccacgtcaatgaccttgctcgccagcttaccactttgggcattcagctctcaccgtataacctcagcactctggaagacctgaacaccagatggaagcttctgcaggtggccgtcgaggaccgagtcaggcagctgcatgaagcccacagggactttggtccagcatctcagcactttctttccacgtctgtccagggtccctgggagagagccatctcgccaaacaaagtgccctactatatcaaccacgagactcaaacaacttgctgggaccatcccaaaatgacagagctctaccagtctttagctgacctgaataatgtcagattctcagcttataggactgccatgaaactccgaagactgcagaaggccctttgcttggatctcttgagcctgtcagctgcatgtgatgccttggaccagcacaacctcaagcaaaatgaccagcccatggatatcctgcagattattaattgtttgaccactatttatgaccgcctggagcaagagcacaacaatttggtcaacgtccctctctgcgtggatatgtgtctgaactggctgctgaatgtttatgatacgggacgaacagggaggatccgtgtcctgtcttttaaaactggcatcatttccctgtgtaaagcacatttggaagacaagtacagataccttttcaagcaagtggcaagttcaacaggattttgtgaccagcgcaggctgggcctccttctgcatgattctatccaaattccaagacagttgggtgaagttgcatcctttgggggcagtaacattgagccaagtgtccggagctgcttccaatttgctaataataagccagagatcgaagcggccctcttcctagactggatgagactggaaccccagtccatggtgtggctgcccgtcctgcacagagtggctgctgcagaaactgccaagcatcaggccaaatgtaacatctgcaaagagtgtccaatcattggattcaggtacaggagtctaaagcactttaattatgacatctgccaaagctgctttttttctggtcgagttgcaaaaggccataaaatgcactatcccatggtggaatattgcactccgactacatcaggagaagatgttcgagactttgccaaggtactaaaaaacaaatttcgaaccaaaaggtattttgcgaagcatccccgaatgggctacctgccagtgcagactgtcttagagggggacaacatggaaacgcctgcctcgtcccctcagctttcacacgatgatactcattcacgcattgaacattatgctagcaggctagcagaaatggaaaacagcaatggatcttatctaaatgatagcatctctcctaatgagagcatagatgatgaacatttgttaatccagcattactgccaaagtttgaaccaggactcccccctgagccagcctcgtagtcctgcccagatcttgatttccttagagagtgaggaaagaggggagctagagagaatcctagcagatcttgaggaagaaaacaggaatctgcaagcagaatatgaccgtctaaagcagcagcacgaacataaaggcctgtccccactgccgtcccctcctgaaatgatgcccacctctccccagagtccccgggatgctgagctcattgctgaggccaagctactgcgtcaacacaaaggccgcctggaagccaggatgcaaatcctggaagaccacaataaacagctggagtcacagttacacaggctaaggcagctgctggagcaaccccaggcagaggccaaagtgaatggcacaacggtgtcctctccttctacctctctacagaggtccgacagcagtcagcctatgctgctccgagtggttggcagtcaaacttcggactccatgggtgaggaagatcttctcagtcctccccaggacacaagcacagggtttagaggaggtgatggagcaactcaacaactccttccctagttcaagaggaagaaatacccctggaaagccaatgagagaggacacaatgtag

SEQ ID NO: 6 - DNA, 6718 bp, Artificial Sequence
  Synthetic
atggtttggtgggaagaagtagaggactgttatgaaagagaagatgttcaaaagaaaacattcacaaaatgggtaaatgcacaattttctaagtttgggaagcagcatattgagaacctcttcagtgacctacaggatgggaggcgcctcctagacctcctcgaaggcctgacagggcaaaaactgccaaaagaaaaaggatccacaagagttcatgccctgaacaatgtcaacaaggcactgcgggttttgcagaacaataatgttgatttagtgaatattggaagtactgacatcgtagatggaaatcataaactgactcttggtttgatttggaatataatcctccactggcaggtcaaaaatgtaatgaaaaatatcatggctggattgcaacaaaccaacagtgaaaagattctcctgagctgggtccgacaatcaactcgtaattatccacaggttaatgtaatcaacttcaccaccagctggtctgatggcctggctttgaatgctctcatccatagtcataggccagacctatttgactggaatagtgtggtttgccagcagtcagccacacaacgactggaacatgcattcaacatcgccagatatcaattaggcatagagaaactactcgatcctgaagatgttgataccacctatccagataagaagtccatcttaatgtacatcacatcactcttccaagttttgcctcaacaagtgagcattgaagccatccaggaagtggaaatgttgccaaggccacctaaagtgactaaagaagaacattttcagttacatcatcaaatgcactattctcaacagatcacggtcagtctagcacagggatatgagagaacttcttcccctaagcctcgattcaagagctatgcctacacacaggctgcttatgtcaccacctctgaccctacacggagcccatttccttcacagcatttggaagctcctgaagacaagtcatttggcagttcattgatggagagtgaagtaaacctggaccgttatcaaacagctttagaagaagtattatcgtggcttctttctgctgaggacacattgcaagcacaaggagagatttctaatgatgtggaagtggtgaaagaccagtttcatactcatgaggggtacatgatggatttgacagcccatcagggccgggttggtaatattctacaattgggaagtaagctgattggaacaggaaaattatcagaagatgaagaaactgaagtacaagagcagatgaatctcctaaattcaagatgggaatgcctcagggtagctagcatggaaaaacaaagcaatttacatagagttttaatggatctccagaatcagaaactgaaagagttgaatgactggctaacaaaaacagaagaaagaacaaggaaaatggaggaagagcctcttggacctgatcttgaagacctaaaacgccaagtacaacaacataaggtgcttcaagaagatctagaacaagaacaagtcagggtcaattctctcactcacatggtggtggtagttgatgaatctagtggagatcacgcaactgctgctttggaagaacaacttaaggtattgggagatcgatgggcaaacatctgtagatggacagaagaccgctgggttcttttacaagacatccttctcaaatggcaacgtcttactgaagaacagtgcctttttagtgcatggctttcagaaaaagaagatgcagtgaacaagattcacacaactggctttaaagatcaaaatgaaatgttatcaagtcttcaaaaactggccgttttaaaagcggatctagaaaagaaaaagcaatccatgggcaaactgtattcactcaaacaagatcttcttcaacactgaagaataagtcagtgacccagaagacggaagcatggctggataactttgcccggtgttgggataatttagtccaaaaacttgaaaagagtacagcacagatttcacagtctgttgagaaatggcggcgttttcattatgatataaagatatttaatcagtggctaacagaagctgaagagtttctcagaaagacacaaattcctgagaattgggaacatgctaaatacaaatggtatcttaaggaactccaggatggcattgggcagcggcaaactgttgtcagaacattgaatgcaactggggaagaaataattcagcaatcctcaaaaacagatgccagtattctacaggaaaaattgggaagcctgaatctgcggtggcaggaggtctgcaaacagctgtcagacagaaaaaagaggctagaagaacaaaagaatatcttgtcagaatttcaaagagatttaaatgaatttgttttatggttggaggaagcagataacattgctagtatcccacttgaacctggaaaagagcagcaactaaaagaaaagcttgagcaagtcaagttactggtggaagagttgcccctgcgccagggaattctcaaacaattaaatgaaactggaggacccgtgcttgtaagtgctcccataagcccagaagagcaagataaacttgaaaataagctcaagcagacaaatctccagtggataaaggtttccagagctttacctgagaaacaaggagaaattgaagctcaaataaaagaccttgggcagcttgaaaaaaagcttgaagaccttgaagagcagttaaatcatctgctgctgtggttatctcctattaggaatcagttggaaatttataaccaaccaaaccaagaaggaccatttgacgttcaggaaactgaaatagcagttcaagctaaacaaccggatgtggaagagattttgtctaaagggcagcatttgtacaaggaaaaaccagccactcagccagtgaagaggaagttagaagatctgagctctgagtggaaggcggtaaaccgtttacttcaagagctgagggcaaagcagcctgacctagctcctggactgaccactattggagcctctcctactcagactgttactctggtgacacaacctgtggttactaaggaaactgccatctccaaactagaaatgccatcttccttgatgttggaggtacctgctctggcagatttcaaccgggcttggacagaacttaccgactggctttctctgcttgatcaagttataaaatcacagagggtgatggtgggtgaccttgaggatatcaacgagatgatcatcaagcagaaggcaacaatgcaggatttggaacagaggcgtccccagttggaagaactcattaccgctgcccaaaatttgaaaaacaagaccagcaatcaagaggctagaacaatcattacggatcgaattgaaagaattcagaatcagtgggatgaagtacaagaacaccttcagaaccggaggcaacagttgaatgaaatgttaaaggattcaacacaatggctggaagctaaggaagaagctgagcaggtcttaggacaggccagagccaagcttgagtcatggaaggagggtccctatacagtagatgcaatccaaaagaaaatcacagaaaccaagcagttggccaaagacctccgccagtggcagacaaatgtagatgtggcaaatgacttggccctgaaacttctccgggattattctgcagatgataccagaaaagtccacatgataacagagaatatcaatgcctcttggagaagcattcataaaagggtgagtgagcgagaggctgctttggaagaaactcatagattactgcaacagtccccctggacctggaaaagtttcttgcctggcttacagaagctgaaacaactgccaatgtcctacaggatgctacccgtaaggaaaggctcctagaagactccaagggagtaaaagagctgatgaaacaatggcaagacctccaaggtgaaattgaagctcacacagatgtttatcacaacctggatgaaaacagccaaaaaatcctgagatccgtggaaggttccgatgatgcagtcctgttacaaagacgtttggataacatgaacttcaagtggagtgaacttcggaaaaagtctctcaacattaggtcccatttggaagccagttctgaccagtggaagcgtctgcacctttctctgcaggaacttctggtgtggctacagctgaaagatgatgaattaagccggcaggcacctattggaggcgactttccagcagttcagaagcagaacgatgtacatagggccttcaagagggaattgaaaactaaagaacctgtaatcatgagtactcttgagactgtacgaatatttctgacagagcagcctttggaaggactagagaaactctaccaggagcccagagagctgcctcctgaggagagagcccagaatgtcactcggcttctacgaaagcaggctgaggaggtcaatactgagtgggaaaaattgaacctgcactccgctgactggcagagaaaaatagatgagacccttgaaagactccaggaacttcaagaggccacggatgagctggacctcaagctgcgccaagctgaggtgatcaagggatcctggcagcccgtgggcgatctcctcattgactctctccaagatcacctcgagaaagtcaaggcacttcgaggagaaatttgcgcctctgaaagagaacgtgagccacgtcaatgaccttgctcgccagcttaccactttgggcattcagctctcaccgtataacctcagcactctggaagacctgaacaccagatggaagcttctgcaggtggccgtcgaggaccgagtcaggcagctgcatgaagcccacagggactttggtccagcatctcagcactttctttccacgtctgtccagggtccctgggagagagccatctcgccaaacaaagtgccctactatatcaaccacgagactcaaacaacttgctgggaccatcccaaaatgacagagctctaccagtctttagctgacctgaataatgtcagattctcagcttataggactgccatgaaactccgaagactgcagaaggccctttgcttggatctcttgagcctgtcagctgcatgtgatgccttggaccagcacaacctcaagcaaaatgaccagcccatggatatcctgcagattattaattgtttgaccactatttatgaccgcctggagcaagagcacaacaatttggtcaacgtccctctctgcgtggatatgtgtctgaactggctgctgaatgtttatgatacgggacgaacagggaggatccgtgtcctgtcttttaaaactggcatcatttccctgtgtaaagcacatttggaagacaagtacagataccttttcaagcaagtggcaagttcaacaggattttgtgaccagcgcaggctgggcctccttctgcatgattctatccaaattccaagacagttgggtgaagttgcatcctttgggggcagtaacattgagccaagtgtccggagctgcttccaatttgctaataataagccagagatcgaagcggccctcttcctagactggatgagactggaaccccagtccatggtgtggctgcccgtcctgcacagagtggctgctgcagaaactgccaagcatcaggccaaatgtaacatctgcaaagagtgtccaatcattggatttcaggtacaggagtctaaagcactttaattatgacatctgccaaagctgctttttttctggtcgagttgcaaaaggccataaaatgcactatcccatggtggaatattgcactccgactacatcaggagaagatgttcgagactttgccaaggtactaaaaaacaaatttcgaaccaaaaggtattttgcgaagcatccccgaatgggctacctgccagtgcagactgtcttagagggggacaacatggaaacgcctgcctcgtcccctgagctttcacacgatgatactcattcacgcattgaacatatgctagcaggctagcagaaatggaaaacagcaatggatcttatctaaatgatagcatctctcctaatgagagcatagatgatgaacattttgttaatccagcattactgccaaagtttgaaccaggactcccccctgagccagcctcgtagtcctgcccagatcttgatttccttagagagtgaggaaagaggggagctagagagaatcctagcagatcttgaggaagaaaacaggaatctgcaagcagaatatgaccgtctaaagcagcagcacgaacataaaggcctgtccccactgccgtcccctcctgaaatgatgcccacgtctccccagagtccccgggatgctgagctcattgctgaggccaagctactgcgtcaacacaaaggccgcctggaagccaggatgcaaatcctggaagaccacaataaacagctggagtcacagttacacaggctaaggcagctgctggagcaaccccaggcagaggccaaagtgaatggcacaacggtgtcctctcctttctacctctctacagaggtccgacagcagtcagcctatgctgctccgagtggttggcagtcaaacttcggactccatgggtgaggaagatcttctcagtcctccccaggacacaagcacagggttagaggaggtgatggagcaactcaacaactccttccctagttcaagaggaagaaatacccctggaaagccaatgagagaggacacaatgtag

SEQ ID NO: 7 - DNA, 7049 bp, Artificial Sequence
  Synthetic
atgctttggtgggaagaagtagaggactgttatgaaagagaagatgttcaaaagaaaacattcacaaaatgggtaaatgcacaattttctaagtttgggaagcagcatattgagaacctcttcagtgacctacaggatgggaggcgcctcctagacctcctcgaaggcctgacagggcaaaaactgccaaaagaaaaaggatccacaagagttcatgccctgaacaatgtcaacaaggcactgcgggttttgcagaacaataatgttgatttagtgaatattggaagtactgacatcgtagatggaaatcataaactgactgttggtttgatttggaatataatcctccactggcaggtcaaaaatgtaatgaaaaatatcatggctggattgcaacaaaccaacagtgaaaagattctcctgagctgggtccgacaatcaactcgtaattatccacaggttaatgtaatcaacttcaccaccagctggtctgatggcctggctttgaatgctctcatccatagtcataggccagacctatttgactggaatagtgtggtttgccagcagtcagccacacaacgactggaacatgcattcaacatcgccagatatcaattaggcatagagaaactactcgatcctgaagatgttgataccacctatccagataagaagtccatcttaatgtacatcacatcactcttccaagttttgcctcaacaagtgagcattgaagccatccaggaagtggaaatgttgccaaggccacctaaagtgactaaagaagaacattttcagttacatcatcaaatgcactattctcaacagatcacggtcagtctagcacagggatatgagagaacttcttcccctaagcctcgattcaagagctatgcctacacacaggctgcttatgtcaccacctctgaccctacacggagcccatttccttcacagcatttggaagctcctgaagacaagtcatttggcagttcattgatggagagtgaagtaaacctggaccgttatcaaacagctttagaagaagtattatcgtggcttctttctgctgaggacacattgcaagcacaaggagagatttctaatgatgtggaagtggtgaaagaccagtttcatactcatgaggggtacatgatggatttgacagcccatcagggccgggttggtaatattctacaattgggaagtaagctgattggaacaggaaaattatcagaagatgaagaaactgaagtacaagagcagatgaatctcctaaattcaagatgggaatgcctcagggtagctagcatggaaaaacaaagcaatttacatagagttttaatggatctccagaatcagaaactgaaagagttgaatgactggctaacaaaaacagaagaaagaacaaggaaaatggaggaagagcctcttggacctgatcttgaagacctaaaacgccaagtacaacaacataaggtgcttcaagaagatctagaacaagaacaagtcagggtcaattctctcactcacatggtggtggtagttgatgaatctagtggagatcacgcaactgctgctttggaagaacaacttaaggtatttgggagatcgatgggcaaacatctgtagatggacagaagaccgctgggttcttttacaagacatccttctcaaatggcaacgtcttactgaagaacagtgcctttttagtgcatggctttcagaaaaagaagatgcagtgaacaagattcacacaactggctttaaagatcaaaatgkaatgttatcaagtcttcaaaaagtggccgttttaaaagcggatctagaaaagaaaaagcaatccatgggcaaactgtattcactcaaacaagatcttctttcaacactgaagaataagtcagtgacccagaagacggaagcatggctggataactttgcccggtgttgggataatttagtccaaaaacttgaaaagagtacagcacagatttcacaggaaatttcttatgtgccttctacttatttgactgaaatcactcatgtctcacaagccctattagaagtggaacaacttctcaatgctcctgacctctgtgctaaggactttgaagatctctttaagcaagaggagtctctgaagaatataaaagatagtctacaacaaagctcaggtcggattgacattattcatagcaagaagacagcagcattgcaaagtgcaacgcctgtggaaagggtgaagctacaggaagctctctcccagcttgatttccaatgggaaaaagttaacaaaatgtacaaggaccgacaagggcgatttgacagatctgttgagaaatggcggcgttttcattatgatataaagatatttaatcagtggctaacagaagctgaacagtttctcagaaagacacaaattcctgagaattgggaacatgctaaatacaaatggtatcttaaggaactccaggatggcattgggcagcggcaaactgttgtcagaacattgaatgcaactggggaagaaataattcagcaatcctcaaaaacagatgccagtattctacaggaaaaattgggaagcctgaatctgcggtggcaggaggtctgcaaacagctgtcagacagaaaaaagaggctagaagaacaaaagaatatcttgtcagaatttcaaagagatttaaatgaatttgttttatggttggaggaagcagataacattgctagtatcccacttgaacctggaaaagagcagcaactaaaagaaaagcttgagcaagtcaagttactggtggaagagttgcccctgcgccagggaattctcaaacaattaaatgaaactggaggacccgtgcttgtaagtgctcccataagcccagaagagcaagataaacttgaaaataagctcaagcagacaaatctccagtggataaaggtttccagagctttacctgagaaacaaggagaaattgaagctcaaataaaagaccttgggcagcttgaaaaaaagcttgaagaccttgaagagcagttaaatcatctgctgctgtggttatctcctattaggaatcagttggaaatttataaccaaccaaaccaagaaggaccatttgacgttcaggaaactgaaatagcagttcaagctaaacaaccggatgtggaagagattttgtctaaagggcagcatttgtacaaggaaaaaccagccactcagccagtgaagaggaagttagaagatctgagctctgagtggaaggcggtaaaccgtttacttcaagagctgagggcaaagcagcctgacctagctcctggactgaccactattggagcctctcctactcagactgttactctggtgacacaacctgtggttactaaggaaactgccatctccaaactagaaatgccatcttccttgatgttggaggtacctgctctggcagatttcaaccgggcttggacagaacttaccgactggctttctctgcttgatcaagttataaaatcacagagggtgatggtgggtgaccttgaggatatcaacgagatgatcatcaagcagaaggcaacaatgcaggatttggaacagaggcgtccccagttggaagaactcattaccgctggccaaaatttgaaaaacaagaccagcaatcaagaggctagaacaatcattacggatcgaattgaaagaattcagaatcagtgggatgaagtacaagaacaccttcagaaccggaggcaacagttgaatgaaatgttaaaggattcaacacaatggctggaagctaaggaagaagctgagcaggtcttaggacaggccagagccaagcttgagtcatggaaggagggtccctatacagtagatgcaatccaaaagaaaatcacagaaaccaagcagttggccaaagacctccgccagtggcagacaaatgtagatgtggcaaatgacttggccctgaaacttctccgggattattctgcagatgataccagaaaagtccacatgataacagagaatatcaatgcctcttggagaagcattcataaaagggtgagtgagcgagaggctgctttggaagaaactcatagattactgcaacagttccccctggacctggaaaagtttcttgcctggcttacagaagctgaaacaactgccaatgtcctacaggatgctacccgtaaggaaaggctcctagaagactccaagggagtaaaagagctgatgaaacaatggcaagacctccaaggtgaaattgaagctcacacagatgtttatcacaacctggatgaaaacagccaaaaaatcctgagatccctggaaggttccgatgatgcagtcctgttacaaagacgtttggataacatgaacttcaagtggagtgaacttcggaaaaagtctctcaacattaggtcccatttggaagccagttctgaccagtggaagcgtctgcacctttctctgcaggaacttctggtgtggctacagctgaaagatgatgaattaagccggcaggcacctattggaggcgactttccagcagttcagaagcagaacgatgtacatagggccttcaagagggaattgaaaactaaagaacctgtaatcatgagtactcttgagactgtacgaatatttctgacagagcagcctttggaaggactagagaaactctaccaggagcccagagagctgcctcctgaggagagagcccagaatgtcactcggcttctacgaaagcaggctgaggaggtcaatactgagtgggaaaaattgaacctgcactccgctgactggcagagaaaaatagatgagacccttgaaagactccaggaacttcaagaggccacggatgagctggacctcaagctgcgcgaagctgaggtgatcaagggatcctggcagcccgtgggcgatctcctcattgactctctccaagatcacctcgagaaagtcaaggcacttcgaggagaaattgcgcctctgaaagagaacgtgagccacgtcaatgaccttgctcgccagcttaccactttgggcattcagctctcaccgtataacctcagcactctggaagacctgaacaccagatggaagcttctgcaggtggccgtcgaggaccgagtcaggcagctgcatgaagcccacagggactttggtccagcatctcagcactttctttccacgtctgtccagggtccctgggagagagccatctcgccaaacaaagtgccctactatatcaaccacgagactcaaacaacttgctgggaccatcccaaaatgacagagctctaccagtctttagctgacctgaataatgtcagattctcagcttataggactgccatgaaactccgaagactgcagaaggccctttgcttggatctcttgagcctgtcagctgcatgtgatgccttggaccagcacaacctcaagcaaaatgaccagcccatggatatcctgcagattattaattgtttgaccactatttatgaccgcctggagcaagagcacaacaatttggtgaacgtgcctctctgcgtggatatgtgtctgaactggctggtgaatgtttatgatacgggacgaacagggaggatccgtgtcctgtcttttaaaactggcatcatttccctgtgtaaagcacatttggaagacaagtacagataccttttcaagcaagtgggaagttcaacaggattttgtgaccagcgcaggctgggcctccttctgcatgattctatccaaattccaagacagttgggtgaagttgcatcctttgggggcagtaacattgagccaagtgtccggagctgcttccaatttgctaataataagccagagatcgaagcggccctcttcctagactggatgagactggaaccccagtccatggtgtggctgcccgtcctgcacagagtggctgctgcagaaactgccaagcatcaggccaaatgtaacatctgcaaagagtgtccaatcattggattcaggtacaggagtctaaagcactttaattatgacatctgccaaagctgctttttttctggtcgagttgcaaaaggccataaaatgcactatcccatggtggaatattgcactccgactacatcaggagaagatgttcgagactttgccaaggtactaaaaaacaaatttcgaaccaaaaggtattttgcgaagcatccccgaatgggctacctgccagtgcagactgtcttagagggggacaacatggaaacgcctgcctcgtcccctcagctttcacaggatgatactcattcacgcattgaacattatgctagcaggctagcagaaatggaaaacagcaatggatctttatctaaatgatagcatctctcctaatgagagcatagatgatgaacatttgttaatccagcattactgccaaagtttgaaccaggactcccccctgagccagcctcgtagtcctgcccagatcttgatttccttagagagtgaggaaagaggggagctagagagaatcctagcagatcttgaggaagaaaacaggaatctgcaagcagaatatgaccgtctaaagcagcagcacgaacataaaggcctgtccccactgccgtcccctcctgaaatgatgcccacctctccccagagtccccgggatgctgagctcattgctgaggccaagctactgcgtcaacacaaaggccgcctggaagccaggatgcaaatcctggaagaccacaataaacagctggagtcacagttacacaggctaaggcagctggtggagcaaccccaggcagaggccaaagtgaatggcacaacggtgtcctctccttctacctctctacagaggtccgacagcagtcagcctatgctgctccgagtggttggcagtcaaacttcggactccatgggtgaggaagatcttctcagtcctccccaggacacaagcacagggttagaggaggtgatggagcaactcaacaactccttccctagttcaagaggaagaaatacccctggaaagccaatgagagaggacacaatgtag

SEQ ID NO: 8 - DNA, 6398 bp, Artificial Sequence
  Synthetic
atgctttggtgggaagaagtagaggactgttatgaaagagaagatgttcaaaagaaaacattcacaaaatgggtaaatgcacaattttctaagtttgggaagcagcatattgagaacctcttcagtgacctacaggatgggaggcgcctcctagacctcctcgaaggcctgacagggcaaaaactgccaaaagaaaaaggatccacaagagttcatgccctgaacaatgtcaacaaggcactgcgggttttgcagaacaataatgttgatttagtgaatattggaagtactgacatcgtagatggaaatcataaactgactcttggtttgatttggaatataatcctccactggcaggtcaaaaatgtaatgaaaaatatcatggctggattgcaacaaaccaacagtgaaaagattctcctgagctgggtccgacaatcaactcgtaattatccacaggttaatgtaatcaacttcaccaccagctggtctgatggcctggcttgaatgctctcatccatagtcataggccagacctatttgactggaatagtgtggtttgccagcagtcagccacacaacgactggaacatgcattcaacatcgccagatatcaattaggcatagagaaactactcgatcctgaagatgttgataccacctatccagataagaagtccatcttaatgtacatcacatcactcttccaagttttgcctcaacaagtgagcattgaagccatccaggaagtggaaatgttgccaaggccacctaaagtgactaaagaagaacattttcagttacatcatcaaatgcactattctcaacagatcacggtcagtctagcacagggatatgagagaacttcttcccctaaggctcgattcaagagctatgcctacacacaggctgcttatgtcaccacctctgaccctacacggagcccatttccttcacagcatttggaagctcctgaagacaagtcatttggcagttcattgatggagagtgaagtaaacctggaccgttatcaaacagctttagaagaagtattatcgtggcttctttctgctgaggacacattgcaagcacaaggagagatttctaatgatgtggaagtggtgaaagaccagtttcatactcatgaggggtacatgatggatttgacagcccatcagggccgggttggtaatattctacaattgggaagtaagctgattggaacaggaaaattatcagaagatgaagaaactgaagtacaagagcagatgaatctcctaaattcaagatgggaatgcctcagggtagctagcatggaaaaacaaagcaatttacatagagttttaatggatctccagaatcagaaactgaaagagttgaatgactggctaacaaaaacagaagaaagaacaaggaaaatggaggaagagcctcttggacctgatcttgaagacctaaaacgccaagtacaacaacataaggtgcttcaagaagatctagaacaagaacaagtcagggtcaattctctcactcacatggtggtggtagttgatgaatctagtggagatcacgcaactgctgctttggaagaacaacttaaggtattgggagatcgatgggcaaacatctgtagatggacagaagaccgctgggttcttttacaagacatccttctcaaatggcaacgtcttactgaagaacagtgcctttttagtgcatggctttcagaaaaagaagatgcagtgaacaagattcacacaactggctttaaagatcaaaatgaaatgttatcaagtcttcaaaaactggccgttttaaaagcggatctagaaaagaaaaagcaatccatgggcaaactgtattcactcaaacaagatcttctttcaacactgaagaataagtcagtgacccagaagacggaagcatggctggataactttgcccggtgttgggataatttagtccaaaaacttgaaaagagtacagcacagatttcacaggaaatttcttatgtgccttctacttatttgactgaaatcactcatgtctcacaagccctattagaagtggaacaacttctcaatgctcctgacctctgtgctaaggactttgaagatctctttaagcaagaggagtctctgaagaatataaaagatagtctacaacaaagctcaggtcggattgacattattcatagcaagaagacagcagcattgcaaagtgcaacgcctgtggaaagggtgaagctacaggaagctctctcccagcttgatttccaatgggaaaaagttaacaaaatgtacaaggaccgacaagggcgatttgacagatctgttgagaaatggcggcgttttcattatgatataaagatatttaatcagtggctaacagaagctgaacagtttctcagaaagacacaaattcctgagaattgggaacatgctaaatacaaatggtatcttaaggaactccaggatggcattgggcagcggcaaactgttgtcagaacattgaatgcaactggggaagaaataattcagcaatcctcaaaaacagatgccagtattctacaggaaaaattgggaagcctgaatctgcggtggcaggaggtctgcaaacagctgtcagacagaaaaaagaggctagaagaacagcctgacctagctcctggactgacgactattggagcctctcctactcagactgttactctggtgacacaacctgtggttactaaggaaactgccatctccaaactagaaatgccatcttccttgatgttggaggtacctgctctggcagatttcaaccgggcttggacagaacttaccgactggctttctgtgcttgatcaagttataaaatcacagagggtgatggtgggtgaccttgaggatatcaacgagatgatcatcaagcagaaggcaacaatgcaggatttggaacagaggcgtccccagttggaagaactcattaccgctgcccaaaatttgaaaaacaagaccagcaatcaagaggctagaacaatcattacggatcgaattgaaagaattcagaatcagtgggatgaagtacaagaacaccttcagaaccggaggcaacagttgaatgaaatgttaaaggattcaacacaatggctggaagctaaggaagaagctgagcaggtcttaggacaggccagagccaagcttgagtcatggaaggagggtccctatacagtagatgcaatccaaaagaaaatcacagaaaccaaggagttggccaaagacctccgccagtggcagacaaatgtagatgtggcaaatgacttggccctgaaacttgtccgggattattctgcagatgataccagaaaagtccacatgataacagagaatatcaatgcctcttggagaagcattcataaaagggtgagtgagcgagaggctgctttggaagaaactcatagattactgcaacagttccccctggacctggaaaagtttcttgcctggcttacagaagctgaaacaactgccaatgtcctacaggatgctacccgtaaggaaaggctcctagaagactccaagggagtaaaagagctgatgaaacaatggcaagacctccaaggtgaaatgaagctcacacagatgtttatcacaacctggatgaaaacagccaaaaaatcctgagatccctggaaggttccgatgatgcagtcctgttacaagacgthtggataacatgaacttcaagtggagtgaacttcggaaaaagtctctcaacattaggtcccatttggaagccagttctgaccagtggaagcgtctgcacctttctctgcaggaacttctggtgtggctacagctgaaagatgatgaattaagccggcaggcacctattggaggcgactttccagcagttcagaagcagaacgatgtacatagggccttcaagagggaattgaaaactaaagaacctgtaatcatgagtactcttgagactgtacgaatatttctgacagagcagcctttggaaggactagagaaactctaccaggagcccagagagctgcctcctgaggagagagcccagaatgtcactcggcttctacgaaagcaggctgaggaggtcaatactgagtgggaaaaattgaacctgcactccgctgactggcagagaaaaatagatgagacccttgaaagactccaggaacttcaagaggccacggatgagctggacctcaagctgcgccaagctgaggtgatcaagggatcctggcagcccgtgggcgatctcctcatgactctctccaagatcacctcgagaaagtcaaggcacttcgaggagaaattgcgcctctgaaagagaacgtgagccacgtcaatgaccttgctcgccagcttaccactttgggcattcagctctcaccgtataacctcagcactctggaagacctgaacaccagatggaagcttctgcaggtggccgtcgaggaccgagtcaggcagctgcatgaagcccacagggactttggtccagcatctcagcactttctttccacgtctgtccagggtccctgggagagagccatctcgccaaacaaagtgccctactatatcaaccacgagactcaaacaacttgctgggaccatcccaaaatgacagagctctaccagtctttagctgacctgaataatgtcagattctcagcttataggactgccatgaaactccgaagactgcagaaggccctttgcttggatctcttgagcctgtcagctgcatgtgatgccttggaccagcacaacctcaagcaaaatgaccagcccatggatatcctgcagattattaattgtttgaccactatttatgaccgcctggagcaagagcacaacaatttggtcaacgtccctctctgcgtggatatgtgtctgaactggctgctgaatgtttatgatacgggacgaacagggaggatccgtgtcctgtcttttaaaactggcatcatttccctgtgtaaagcacatttggaagacaagtacagataccttttcaagcaagtggcaagttcaacaggattttgtgaccagcgcaggctgggcctccttctgcatgattctatccaaattccaagacagttgggtgaagttgcatcctttgggggcagtaacattgagccaagtgtccggagctgcttccaatttgctaataataagccagagatcgaagcggccctcttcctagactggatgagactggaaccccagtccatggtgtggctgcccgtcctgcacagagtggctgctgcagaaactgccaagcatcaggccaaatgtaacatctgcaaagagtgtccaatcattggattcaggtacaggagtctaaagcactttaattatgacatctgccaaagctgctttttttctggtcgagttgcaaaaggccataaaatgcactatcccatggtggaatattgcactccgactacatcaggagaagatgttcgagactttgccaaggtactaaaaaacaaatttcgaaccaaaaggtattttgcgaagcatccccgaatgggctacctgccagtgcagactgtcttagagggggacaacatggaaacgcctgcctcgtcccctcagctttcacacgatgatactcattcacgcattgaacattatgctagcaggctagcagaaatggaaaacagcaatggatcttatctaaatgatagcatctctcctaatgagagcatagatgatgaacatttgttaatccagcattactgccaaagtttgaaccaggactcccccctgagccagcctcgtagtcctgcccagatcttgatttccttagagagtgaggaaagaggggagctagagagaatcctagcagatcttgaggaagaaaacaggaatctgcaagcagaatatgaccgtctaaagcagcagcacgaacataaaggcctgtccccactgccgtcccctcctgaaatgatgcccacctctccccagagtccccgggatgctgagctcattgctgaggccaagctactgcgtcaacacaaaggccgcgtggaagccaggatgcaaatcctggaagaccacaataaacagctggagtcacagttacacaggctaaggcagctgctggagcaaccccaggcagaggccaaagtgaatggcacaacggtgtcctctccttctacctctctacagaggtccgacagcagtcagcctatgctgctccgagtggttggcagtcaaacttcggactccatgggtgaggaagatcttctcagtcctccccaggacacaagcacagggttagaggaggtgatggagcaactcaacaactccttccctagttcaagaggaagaaatacccctggaaagccaatgagagaggacacaatgtag

SEQ ID NO: 9 - DNA, 6078 bp, Artificial Sequence
  Synthetic
atgctttggtgggaagaagtagaggactgttatgaaagagaagatgttcaaaagaaaacattcacaaaatgggtaaatgcacaattttctaagtttgggaagcagcatattgagaacctcttcagtgacctacaggatgggaggcgcctcctagacctcctcgaaggcctgacagggcaaaaactgccaaaagaaaaaggatccacaagagttcatgccctgaagaatgtcaacaaggcactgcgggttttgcagaacaataatgttgatttagtgaatattggaagtactgagatcgtagatggaaatcataaactgactcttggtttgatttggaatataatcctccactggcaggtcaaaaatgtaatgaaaaatatcatggctggattgcaacaaaccaacagtgaaaagattctcctgagctgggtccgacaatcaactcgtaattatccacaggttaatgtaatcaacttcaccaccagctggtctgatggcctggctttgaatgctctcatccatagtcataggccagacctatttgactggaatagtgtggtttgccagcagtcagccacacaacgactggaacatgcattcaacatcgccagatatcaattaggcatagagaaactactcgatcctgaagatgttgataccacctatccagataagaagtccatcttaatgtacatcacatcactcttccaagttttgcctcaacaagtgagcattgaagccatccaggaagtggaaatgttgccaaggccacctaaagtgactaaagaagaacattttcagttacatcatcaaatgcactattctcaacagatcacggtcagtctagcacagggatatgagagaacttcttcccctaagcctcgattcaagagctatgcctacacacaggctgcttatgtcaccacctctgaccctacacggagcccatttccttcacagcatttggaagctcctgaagacaagtcatttggcagttcattgatggagagtgaagtaaacctggaccgttatcaaacagctttagaagaagtattatcgtggcttctttctgctgaggacacattgcaagcacaaggagagatttctaatgatgtggaagtggtgaaagaccagtttcatactcatgaggggtacatgatggatttgacagcccatcagggccgggttggtaatattctacaattgggaagtaagctgattggaacaggaaaattatcagaagatgaagaaactgaagtacaagagcagatgaatctcctaaattcaagatgggaatgcctcagggtagctagcatggaaaaacaaagcaatttacatagagttttaatggatctccagaatcagaaactgaaagagttgaatgactggctaacaaaaacagaagaaagaacaaggaaaatggaggaagagcctcttggacctgatcttgaagacctaaaacgccaagtacaacaacataaggtgcttcaagaagatctagaacaagaacaagtcagggtcaattctctcactcacatggtggtggtagttgatgaatctagtggagatcacgcaactgctgctttggaagaacaacttaaggtattgggagatcgatgggcaaacatctgtagatggacagaagaccgctgggttcttttacaagacatccttctcaaatggcaacgtcttactgaagaacagtgcctttttagtgcatggctttcagaaaaagaagatgcagtgaacaagattcacacaactggctttaaagatcaaaatgaaatgttatcaagtcttcaaaaactggccgttttaaaagcggatctagaaaagaaaaagcaatccatgggcaaactgtattcactcaaacaagatcttctttcaacactgaagaataagtcagtgacccagaagacggaagcatggctggataactttgcccggtgtgggataatttagtccaaaaacttgaaaagagtacagcacagatttcacaggaaattcttatgtgccttctacttatttgactgaaatcactcatgtctcacaagccctattagaagtggaacaacttctcaatgctcctgacctctgtgctaaggactttgaagatctctttaagcaagaggagtctctgaagaatataaaagatagtctacaacaaagctcaggtcggattgacattattcatagcaagaagacagcagcattgcaaagtgcaacgcctgtggaaagggtgaagctacaggaagctctctcccagcttgatttccaatgggaaaaagttaacaaaatgtacaaggaccgacaagggcgatttgacagacagcctgacctagctcctggactgaccactattggagcctctcctactcagactgttactctggtgacacaacctgtggttactaaggaaactgccatctccaaactagaaatgccatcttccttgatgttggaggtacctgctctggcagatttcaaccgggcttggacagaacttaccgactggctttctctgcttgatcaagttataaaatcacagagggtgatggtgggtgaccttgaggatatcaacgagatgatcatcaagcagaaggcaacaatgcaggatttggaacagaggcgtccccagttggaagaactcattaccgctgcccaaaatttgaaaaacaagaccagcaatcaagaggctagaacaatcattacggatcgaattgaaagaattcagaatcagtgggatgaagtacaagaacaccttcagaaccggaggcaacagttgaatgaaatgttaaaggattcaacacaatggctggaagctaaggaagaagctgagcaggtcttaggacaggccagagccaagcttgagtcatggaaggagggtccctatacagtagatgcaatccaaaagaaaatcacagaaaccaagcagttggccaaagacctccgccagtggcagacaaatgtagatgtggcaaatgacttggccctgaaacttctccgggattattctgcagatgataccagaaaagtccacatgataacagagaatatcaatgcctcttggagaagcattcataaaagggtgagtgagcgagaggctgctttggaagaaactcatagattactgcaacagttccccctggacctggaaaagtttcttgcctggcttacagaagctgaaacaactgccaatgtcctacaggatgctacccgtaaggaaaggctcctagaagactccaagggagtaaaagagctgatgaaacaatggcaagacctccaaggtgaaattgaagctcacacagatgtttatcacaacctggatgaaaacagccaaaaaatcctgagatccctggaaggttccgatgatgcagtcctgttacaaagacgtttggataacatgaacttcaagtggagtgaacttcggaaaaagtctctcaacattaggtcccatttggaagccagttctgaccagtggaagcgtctgcacctttctctgcaggaacttctggtgtggctacagctgaaagatgatgaattaagccggcaggcacctattggaggcgactttccagcagttcagaagcagaacgatgtacatagggccttcaagagggaattgaaaactaaagaacctgtaatcatgagtactctgagactgtacgaatatttctgacagagcagcctttggaaggactagagaaactctaccaggagcccagagagctgcctcctgaggagagagcccagaatgtcactcggcttctacgaaagcaggctgaggaggtcaatactgagtgggaaaaattgaacctgcactccgctgactggcagagaaaaatagatgagacccttgaaagactccaggaacttcaagaggccacggatgagctggacctcaagctgcgccaagctgaggtgatcaagggatcctggcagcccgtgggcgatctcctcattgactctctccaagatcacctcgagaaagtcaaggcacttcgaggagaaattgcgcctctgaaagagaacgtgagccacgtcaatgaccttgctcgccagcttaccactttggggattcagctctcaccgtataacctcagcactctggaagacctgaacaccagatggaagcttctgcaggtggccgtcgaggacggagtcaggcaggtgcatgaagcccacagggactttggtccagcatgtcagcactttctttccacgtctgtccagggtccctgggagagagccatctcgccaaacaaagtgccctactatatcaaccacgagactcaaacaacttgctgggaccatcccaaaatgacagagctctaccagtctttagctgacctgaataatgtcagattctcagcttataggactgccatgaaactccgaagactgcagaaggccctttgcttggatctcttgagcctgtcagctgcatgtgatgccttggaccagcacaacctcaagcaaaatgaccagcccatggatatcctgcagattattaattgtttgaccactatttatgaccgcctggagcaagagcacaacaatttggtcaacgtccctctctgcgtggatatgtgtctgaactggctgctgaatgtttatgatacgggacgaacagggaggatccgtgtcctgtcttttaaaactggcatcatttccctgtgtaaagcacatttggaagacaagtacagataccttttcaagcaagtggcaagttcaacaggattttgtgaccagcgcaggctgggcctccttctgcatgattctatccaaattccaagacagttgggtgaagttgcatcctttgggggcagtaacattgagccaagtgtccggagctgcttccaatttgctaataataagccagagatcgaagcggccctcttcctagactggatgagactggaaccccagtccatggtgtggctgcccgtcctgcacagagtggctgctgcagaaactgccaagcatcaggccaaatgtaacatctgcaaagagtgtccaatcattggattcaggtacaggagtctaaagcactttaattatgacatctgccaaagctgctttttttctggtcgagttgcaaaaggccataaaatgcactatcccatggtggaatattgcactccgactacatcaggagaagatgttcgagactttgccaaggtactaaaaaacaaatttcgaagcaaaaggtattttgcgaagcatccccgaatgggctacctgccagtgcagactgtcttagagggggacaacatggaaacgcctgcctcgtcccctcagctttcacacgatgatactcattcacgcattgaacattatgctagcaggctagcagaaatggaaaacagcaatggatcttatctaaatgatagcatctctcctaatgagagcatagatgatgaacatttgttaatccagcattactgccaaagtttgaaccaggactcccccctgagccagcctcgtagtcctgcccagatcttgatttccttagagagtgaggaaagaggggagctagagagaatcctagcagatcttgaggaagaaaacaggaatctgcaagcagaatatgaccgtctaaagcagcagcacgaacataaaggcctgtccccactgccgtcccctcctgaaatgatgcccacctctccccagagtccccgggatgctgagctcattgctgaggccaagctactgcgtcaacacaaaggccgcctggaagccaggatgcaaatcctggaagaccacaataaacagctggagtcacagttacacaggctaaggcagctgctggagcaaccccaggcagaggccaaagtgaatggcacaacggtgtcctctccttctacctctctacagaggtccgacagcagtcagcctatgctgctccgagtggttggcagtcaaacttcggactccatgggtgaggaagatcttctcagtcctccccaggacacaagcacagggttagaggaggtgatggagcaactcaacaactccttccctagttgaagaggaagaaatacccctggaaagccaatgagagaggacacaatgtag

SEQ ID NO: 10 - DNA, 6264 bp, Artificial Sequence
  Synthetic
atgctttggtgggaagaagtagaggactgttatgaaagagaagatgttcaaaagaaaacattcacaaaatgggtaaatgcacaattttctaagtttgggaagcagcatattgagaacctcttcagtgacctacaggatgggaggcgcctcctagacctcctcgaaggcctgacagggcaaaaactgccaaaagaaaaaggatccacaagagttcatgccctgaacaatgtcaacaaggcactgcgggttttgcagaacaataatgttgatttagtgaatattggaagtactgacatcgtagatggaaatcataaactgactcttggtttgatttggaatataatcctccactggcaggtcaaaaatgtaatgaaaaatatgatggctggattgcaacaaaccaacagtgaaaagattctcctgagctgggtccgacaatcaactcgtaattatccacaggttaatgtaatcaacttcaccaccagctggtctgatggcctggctttgaatgctctcatccatagtcataggccagacctatttgactggaatagtgtggtttgccagcagtcagccacacaacgactggaacatgcattcaacatcgccagatatcaattaggcatagagaaactactcgatcctgaagatgttgataccacctatccagataagaagtccatcttaatgtacatcacatcactcttccaagttttgcctcaacaagtgagcattgaagccatccaggaagtggaaatgttgccaaggccacctaaagtgactaaagaagaacattttcagttacatcatcaaatgcactattctcaacagatcacggtcagtctagcacagggatatgagagaacttcttcccctaagcctcgattcaagagctatgcctacacacaggctgcttatgtcaccacctctgaccctacacggagcccatttccttcacagcatttggaagctcctgaagacaagtcatttggcagttcattgatggagagtgaagtaaacctggaccgttatcaaacagctttagaagaagtattatcgtggcttctttctgctgaggacacattgcaagcacaaggagagatttctaatgatgtggaagtggtgaaagaccagtttcatactcatgaggggtacatgatggatttgacagcccatcagggccgggttggtaatattctacaattgggaagtaagctgattggaacaggaaaatttatcagaagatgaagaaactgaagtacaagagcagatgaatctcctaaattcaagatgggaatgcctcagggtagctagcatggaaaaacaaagcaatttacatagagttttaatggatctccagaatcagaaactgaaagagttgaatgactggctaacaaaaacagaagaaagaacaaggaaaatggaggaagagcctcttggacctgatcttgaagacctaaaacgccaagtacaacaacataaggtgcttcaagaagatctagaacaagaacaagtcagggtcaattctctcactcacatggtggtggtagttgatgaatctagtggagatcacgcaactgctgctttggaagaacaacttaaggtattgggagatcgatgggcaaacatctgtagatggacagaagaccgctgggttcttttacaagacatccttctcaaatggcaacgtcttactgaagaacagtgcctttttagtgcatggctttcagaaaaagaagatgcagtgaacaagattcacacaactggctttaaagatcaaaatgaaatgttatcaagtcttcaaaaactggccgttttaaaagcggatctagaaaagaaaaagcaatccatgggcaaactgtattcactcaaacaagatcttctttcaacactgaagaataagtcagtgacccagaagacggaagcatggctggataactttgcccggtgttgggataatttagtccaaaaacttgaaaagagtacagcacagatttcacaggaaatttcttatgtgccttctacttatttgactgaaatcactcatgtctcacaagccctattagaagtggaacaacttctcaatgctcctgacctctgtgctaaggactttgaagatctctttaagcaagaggagtctctgaagaatataaaagatagtctacaacaaagctcaggtcggattgacattattcatagcaagaagacagcagcattgcaaagtgcaacgcctgtggaaagggtgaagctacaggaagctctctcccagcttgatttccaatgggaaaaagttaacaaaatgtacaaggacggacaagggcgatttgacagatctgttgagaaatggcggcgttttcattatgatataaagatatttaatcagtggctaacagaagctgaacagtttctcagaaagacacaaattcctgagaattgggaacatgctaaatacaaatggtatcttaaggaactccaggatggcattgggcagcggcaaactgttgtcagaacattgaatgcaactggggaagaaataattcagcaatcctcaaaaacagatgccagtattctacaggaaaaattgggaagcctgaatctgcggtggcaggaggtctgcaaacagctgtcagacagaaaaaagaggctagaagaacaaaagaatatcttgtcagaatttcaaagagatttaaatgaatttgttttatggttggaggaagcagataacattgctagtatcccacttgaacctggaaaagagcagcaactaaaagaaaagcttgagcaagtcaagttactggtggaagagttgcccctgcgccagggaattctcaaacaattaaatgaaactggaggacccgtgcttgtaagtgctcccataagcccagaagagcaagataaacttgaaaataagctcaagcagacaaatctccagtggataaaggtttccagagctttacctgagaaacaaggagaaattgaagctcaaataaaagaccttgggcagcttgaaaaaaagcttgaagaccttgaagagcagttaaatcatctgctgctgtggttatctcctattaggaatcagttggaaatttataaccaaccaaaccaagaaggaccatttgacgttcaggaaactgaaatagcagttcaagctaaacaaccggatgtggaagagattttgtctaaagggcagcatttgtacaaggaaaaaccagccactcagccagtgaagaggaagttagaagatctgagctctgagtggaaggcggtaaaccgtttacttcaagagctgagggcaaagcagcctgacctagctcctggactgaccactattggagcctctcctactcagactgttactctggtgacacaacctgtggttactaaggaaactgccatctccaaactagaaatgccatcttccttgatgttggaggtacctgctctggcagatttcaaccgggcttggacagaacttaccgactggctttctctgcttgatcaagttataaaatcacagagggtgatggtgggtgaccttgaggatatcaacgagatgatcatcaagcagaaggcaacaatgcaggatttggaacagaggcgtccccagttggaagaactcattaccgctgcccaaaatttgaaaaacaagaccagcaatcaagaggctagaacaatcattacggatcgaattgaaagaattcagaatcagtgggatgaagtacaagaacaccttcagaaccggaggcaacagttgaatgaaatgttaaaggattcaacacaatggctggaagctaaggaagaagctgagcaggtcttaggacaggccagagccaagcttgagtcatggaaggagggtccctatacagtagatgcaatccaaaagaaaatcacagaaaccaagcagttggccaaagacctccgccagtggcagacaaatgtagatgtggcaaatgacttggccctgaaacttctccgggattattctgcagatgataccagaaaagtccacatgataacagagaatatcaatgcctcttggagaagcattcataaaagggtgagtgagcgagaggctgctttggaagaaactcatagattactgcaacagttccccctggacctggaaaagtttcttgcctggcttacagaagctgaaacaactgccaatgtcctacaggatgctacccgtaaggaaaggctcctagaagactccaagggagtaaaagagctgatgaaacaatggcaagacctccaaggtgaaattgaagctcacacagatgtttatcacaacctggatgaaaacagccaaaaaatcctgagatccctggaaggttccgatgatgcagtcctgttacaaagacgtttggataacatgaacttcaagtggagtgaacttcggaaaaagtctctcaacattaggtcccatttggaagccagttctgaccagtggaagcgtctgcacctttctctgcaggaacttctggtgtggctacagctgaaagatgatgaattaagccggcaggcacctattggaggcgactttccagcagttcagaagcagaacgatgtacatagggccttcaagagggaattgaaaactaaagaacctgtaatcatgagtactctgagactgtacgaatatttctgacagagcagcctttggaaggactagagaaactctaccaggagcccagagagctgcctcctgaggagagagcccagaatgtcactcggcttctacgaaagcaggctgaggaggtcaatactgagtgggaaaaattgaacctgcactccgctgactggcagagaaaaatagatgagacccttgaaagactccaggaacttcaagaggccacggatgagctggacctcaagctgcgccaagctgaggtgatcaagggatcctggcagcccgtgggcgatctcctcattgactctctccaagatcacctcgagaaagtcaaggcacttcgaggagaaattgcgcctctgaaagagaacgtgagccacgtcaatgaccttgctcgccagcttaccactttgggcattcagctctcaccgtataacctcagcactctggaagacctgaacaccagatggaagcttctgcaggtggccgtcgaggaccgagtcaggcagctgcatgaagcccacagggactttggtccagcatctcagcactttctttccacgtctgtccagggtccctgggagagagccatctcgccaaacaaagtgccctactatatcaaccacgagactcaaacaacttgctgggaccatcccaaaatgacagagctctaccagtctttagctgacctgaataatgtcagattctcagcttataggactgccatgaaactccgaagactgcagaaggccctttgcttggatctcttgagcctgtcagctgcatgtgatgccttggaccagcacaacctcaagcaaaatgaccagcccatggatatcctgcagattattaattgtttgaccactatttatgaccgcctggagcaagagcacaacaatttggtcaacgtccctctctgcgtggatatgtgtctgaactggctgctgaatgtttatgatacgggacgaacagggaggatccgtgtcctgtcttttaaaactggcatcatttccctgtgtaaagcacatttggaagacaagtacagataccttttcaagcaagtggcaagttcaacaggattttgtgaccagcgcaggctgggcctccttctgcatgattctatccaaattccaagacagttgggtgaagttgcatcctttgggggcagtaacattgagccaagtgtccggagctgcttccaatttgctaataataagccagagatcgaagcggccctcttcctagactggatgagactggaaccccagtccatggtgtggctgcccgtcctgcacagagtggctgctgcagaaactgccaagcatcaggccaaatgtaacatctgcaaagagtgtccaatcattggattcaggtacaggagtctaaagcactttaattatgacatctgccaaagctgctttttttctggtcgagttgcaaaaggccataaaatgcactatcccatggtggaatattgcactccgactacatcaggagaagatgttcgagactttgccaaggtactaaaaaacaaatttcgaaccaaaaggtattttgcgaagcatccccgaatgggctacctgccagtgcagactgtcttagagggggacaacatggaaactgacacaatgtag

SEQ ID NO: 11 - DNA, 4078 bp, Artificial Sequence
  Synthetic
atgctttggtgggaagaagtagaggactgttatgaaagagaagatgttcaaaagaaaacattcacaaaatgggtaaatgcacaattttctaagtttgggaagcagcatattgagaacctcttcagtgacctacaggatgggaggcgcctcctagacctcctcgaaggcctgacagggcaaaaactgccaaaagaaaaaggatccacaagagttcatgccctgaacaatgtcaacaaggcactgcgggttttgcagaacaataatgttgatttagtgaatattggaagtactgacatcgtagatggaaatcataaactgactcttggtttgatttggaatataatcctccactggcaggtcaaaaatgtaatgaaaaatatcatggctggattgcaacaaaccaacagtgaaaagattctcctgagctgggtccgacaatcaactcgtaattatccagaggttaatgtaatcaacttcaccaccagctggtctgatggcctggctttgaatgctctcatccatagtcataggccagacctatttgactggaatagtgtggtttgccagcagtcagccacacaacgactggaacatgcattcaacatcgccagatatcaattaggcatagagaaactactcgatcctgaagatgttgataccacctatccagataagaagtccatcttaatgtacatcacatcactcttccaagttttgcctcaacaagtgagcattgaagccatccaggaagtggaaatgttgccaaggccacctaaagtgactaaagaagaacattttcagttacatcatcaaatgcactattctcaacagatcacggtcagtctagcacagggatatgagagaacttcttcccctaagcctcgattcaagagctatgcctacacacaggctgcttatgtcaccacctctgaccctacacggagcccatttccttcacagcatttggaagctcctgaagacaagtcatttggcagttcattgatggagagtgaagtaaacctggaccgttatcaaacagctttagaagaagtattatcgtggcttctttctgctgaggacacattgcaagcacaaggagagatttctaatgatgtggaagtggtgaaagaccagtttcatactcatgaggggtacatgatggatttgacagcccatcagggccgggttggtaatattctacaattgggaagtaagctgattggaacaggaaaattatcagaagatgaagaaactgaagtacaagagcagatgaatctcctaaattcaagatgggaatgcctcagggtagctagcatggaaaaacaaagcaatttacatagagaaatttcttatgtgccttctacttatttgactgaaatcactcatgtctcacaagccctattagaagtggaacaacttctcaatgctcctgacctctgtgctaaggactttgaagatctctttaagcaagaggagtctctgaagaatataaaagatagtctacaacaaagctcaggtcggattgacattattcatagcaagaagacagcagcattgcaaagtgcaacgcctgtggaaagggtgaagctacaggaagctctctcccagcttgatttcgaatgggaaaaagttaacaaaatgtacaaggaccgacaagggcgatttgacagatctgttgagaaatggcggcgttttcattatgatataaagatatttaatcagtggctaacagaagctgaacagtttctcagaaagacacaaattcctgagaattgggaacatgctaaatacaaatggtatcttaaggaactccaggatggcattgggcagcggcaaactgttgtcagaacattgaatgcaactggggaagaaataattcagcaatcctcaaaaacagatgccagtattctacaggaaaaattgggaagcctgaatctgcggtggcaggaggtctgcaaacagctgtcagacagaaaaaagaggctagaagaacaaaagaatatcttgtcagaatttcaaagagatttaaatgaatttgttttatggttggaggaagcagataacattgctagtatcccacttgaacctggaaaagagcagcaactaaaagaaaagcttgagcaagtcaagttactggtggaagagttgcccctgcgccagggaattctcaaacaattaaatgaaactggaggacccgtgcttgtaagtgctcccataagcccagaagagcaagataaacttgaaaataagctcaagcagacaaatctccagtggataaaggtttccagagctttacgtgagaaagaaggagaaattgaagctcaaataaaagaccttgggcagcttgaaaaaaagcttgaagaccttgaagagcagttaaatcatctgctgctgtggttatctcctattaggaatcagttggaaatttataaccaaccaaaccaagaaggaccatttgacgttcaggaaactgaaatagcagtcaagctaaacaaccggatgtggaagagattttgtctaaagggcagcatttgtacaaggaaaaaccagccactcagccagtgaagaggaagttagaagatctgagctctgagtggaaggcggtaaaccgtttacttcaagagctgagggcaaagacccttgaaagactccaggaacttcaagaggccacggatgagctggacctcaagctgcgccaagctgaggtgatcaagggatcctggcagcccgtgggcgatctcctcattgactctctccaagatcacctcgagaaagtcaaggcacttcgaggagaaattgcgcctctgaaagagaacgtgagccacgtcaatgaccttgctcgccagctaccactttgggcattcagctctcaccgtataacctcagcactctggaagacctgaacaccagatggaagcttctgcaggtggccgtcgaggaccgagtcaggcagctgcatgaagcccacagggactttggtccagcatctcagcactttctttccacgtctgtccagggtccctgggagagagccatctcgccaaacaaagtgccctactatatcaaccacgagactcaaacaacttgctgggaccatcccaaaatgacagagctctaccagtctttagctgacctgaataatgtcagattctcagcttataggactgccatgaaactccgaagactgcagaaggccctttgcttggatctcttgagcctgtcagctgcatgtgatgccttggaccagcacaacctcaagcaaaatgaccagcccatggatatcctgcagattattaattgtttgagcactatttatgaccgcctggagcaagagcacaacaatttggtcaacgtccctctctgcgtggatatgtgtctgaactggctgctgaatgtttatgatacgggacgaacagggaggatccgtgtcctgtcttttaaaactggcatcatttccctgtgtaaagcacatttggaagacaagtacagataccttttcaagcaagtggcaagttcaacaggattttgtgaccagcgcaggctgggcctccttctgcatgattctatccaaattccaagacagttgggtgaagttgcatcctttgggggcagtaacattgagccaagtgtccggagctgcttccaatttgctaataataagccagagatcgaagcggccctcttcctagactggatgagactggaaccccagtccatggtgtggctgcccgtcctgcacagagtggctgctgcagaaactgccaagcatcaggccaaatgtaacatctgcaaagagtgtccaatcattggattcaggtacaggagtctaaagcactttaattatgacatctgccaaagctgctttttttctggtcgagttgcaaaaggccataaaatgcactatcccatggtggaatattgcactccgactacatcaggagaagatgttcgagactttgccaaggtactaaaaaacaaatttcgaaccaaaaggtattttgcgaagcatccccgaatgggctacctgccagtgcagactgtcttagagggggacaacatggaaactgacacaatgtag

SEQ ID NO: 12 - DNA, 3761 bp, Artificial Sequence
  Synthetic
atgctttggtgggaagaagtagaggactgttatgaaagagaagatgttcaaaagaaaacattcacaaaatgggtaaatgcacaattttctaagtttgggaagcagcatattgagaacctcttcagtgacctacaggatgggaggcgcctcctagacctcctcgaaggcctgacagggcaaaaactgccaaaagaaaaaggatccacaagagttcatgccctgaacaatgtcaacaaggcactgcgggttttgcagaacaataatgttgatttagtgaatattggaagtactgacatcgtagatggaaatcataaactgactcttggtttgatttggaatataatcctccactggcaggtcaaaaatgtaatgaaaaatatcatggctggattgcaacaaaccaacagtgaaaagattctcctgagctgggtccgacaatcaactcgtaattatccacaggtaatgtaatcaacttcaccaccagctggtctgatggcctggctttgaatgctctcatccatagtcataggccagacctatttgactggaatagtgtggtttgccagcagtcagccacacaacgactggaacatgcattcaacatcgccagatatcaattaggcatagagaaactactcgatcctgaagatgttgataccacctatccagataagaagtccatcttaatgtacatcacatcactcttccaagttttgcctcaacaagtgagcattgaagccatccaggaagtggaaatgttgccaaggccacctaaagtgactaaagaagaacattttcagttacatcatcaaatgcactattctcaacagatcacggtcagtctagcacagggatatgagagaacttcttcccctaagcctcgattcaagagctatgcctacacacaggctgcttatgtcaccacctctgaccctacacggagcccatttccttcacagcatttggaagctcctgaagacaagtcatttggcagttcattgatggagagtgaagtaaacctggaccgttatcaaacagctttagaagaagtattatcgtggcttctttctgctgaggacacattgcaagcacaaggagagatttctaatgatgtggaagtggtgaaagaccagtttcatactcatgaggggtacatgatggatttgacagcccatcagggccgggttggtaatattctacaattgggaagtaagctgattggaacaggaaaattatcagaagatgaagaaactgaagtacaagagcagatgaatctcctaaattcaagatgggaatgcctcagggtagctagcatggaaaaacaaagcaatttacatagagttttaatggatctccagaatcagaaactgaaagagttgaatgactggctaacaaaaacagaagaaagaacaaggaaaatggaggaagagcctcttggacctgatcttgaagacctaaaacgccaagtacaacaacataaggtgcttcaagaagatctagaacaagaacaagtcagggtcaattctctcactcacatggtggtggtagttgatgaatctagtggagatcacgcaactgctgctttggaagaacaacttaaggtattgggagatcgatgggcaaacatctgtagatggacagaagaccgctgggttcttttacaagacgaaatttcttatgtgccttctacttatttgactgaaatcactcatgtctcacaagccctattagaagtggaacaacttctcaatgctcctgacctctgtgctaaggactttgaagatctctttaagcaagaggagtctctgaagaatataaaagatagtctacaacaaagctcaggtcggattgacattattcatagcaagaagacagcagcattgcaaagtgcaacgcctgtggaaagggtgaagctacaggaagctctctcccagcttgatttccaatgggaaaaagttaacaaaatgtacaaggaccgacaagggcgatttgacagatctgttgagaaatggcggcgttttcattatgatataaagatatttaatcagtggctaacagaagctgaacagtttctcagaaagacacaaattcctgagaattgggaacatgctaaatacaaatggtatcttaaggaactccaggatggcattgggcagcggcaaactgttgtcagaacattgaatgcaactggggaagaaataattcagcaatcctcaaaaacagatgccagtattctacaggaaaaattgggaagcctgaatctgcggtggcaggaggtctgcaaacagctgtcagacagaaaaaagaggctagaagaaacccttgaaagactccaggaacttcaagaggccacggatgagctggacctcaagctgcgccaagctgaggtgatcaagggatcctggcagcccgtgggcgatctcctcattgactctctccaagatcacctcgagaaagtcaaggcacttcgaggagaaattgcgcctctgaaagagaacgtgagccacgtcaatgaccttgctcgccagcttaccactttgggcattcagctctcaccgtataacctcagcactctggaagacctgaacaccagatggaagcttctgcaggtggccgtcgaggaccgagtcaggcagctgcatgaagcccacagggactttggtccagcatctcagcactttctttccacgtctgtccagggtccctgggagagagccatctcgccaaacaaagtgccctactatatcaaccacgagactcaaacaacttgctgggaccatcccaaaatgacagagctctaccagtctttagctgacctgaataatgtcagattctcagcttataggactgccatgaaactccgaagactgcagaaggccctttgcttggatctcttgagcctgtcagctgcatgtgatgccttggaccagcacaacctcaagcaaaatgaccagcccatggatatcctgcagattattaattgtttgaccactatttatgaccgcctggagcaagagcacaacaatttggtcaacgtccctctctgcgtggatatgtgtctgaactggctgctgaatgtttatgatacgggacgaacagggaggatccgtgtcctgtcttttaaaactggcatcatttccctgtgtaaagcacatttggaagacaagtacagataccttttcaagcaagtggcaagttcaacaggattttgtgaccagcgcaggctgggcctccttctgcatgattctatccaaattccaagacagttgggtgaagttgcatcctttgggggcagtaacattgagccaagtgtccggagctgcttccaatttgctaataataagccagagatcgaagcggccctcttcctagactggatgagactggaaccccagtccatggtgtggctgcccgtcctgcacagagtggctgctgcagaaactgccaagcatcaggccaaatgtaacatctgcaaagagtgtccaatcattggattcaggtacaggagtctaaagcactttaattatgacatctgccaaagctgctttttttctggtcgagttgcaaaaggccataaaatgcactatcccatggtggaatattgcactccgactacatcaggagaagatgttcgagactttgccaaggtactaaaaaacaaatttcgaaccaaaaggtattttgcgaagcatccccgaatgggctacctgccagtgcagactgtcttagagggggacaacatggaaactgacacaatgtag

SEQ ID NO: 13 - DNA, 3434 bp, Artificial Sequence
  Synthetic
atgctttggtgggaagaagtagaggactgttatgaaagagaagatgttcaaaagaaaacattcacaaaatgggtaaatgcacaattttctaagtttgggaagcagcatattgagaacctcttcagtgacctacaggatgggaggcgcctcctagacctcctcgaaggcctgacagggcaaaaactgccaaaagaaaaaggatccacaagagttcatgccctgaacaatgtcaacaaggcactgcgggttttgcagaacaataatgttgatttagtgaatattggaagtactgacatcgtagatggaaatcataaactgactcttggtttgatttggaatataatcctccactggcaggtcaaaaatgtaatgaaaaatatcatggctggattgcaacaaaccaacagtgaaaagattctcctgagctgggtccgacaatcaactcgtaattatccacaggttaatgtaatcaacttcaccaccagctggtctgatggcctggctttgaatgctctcatccatagtcataggccagacctatttgactggaatagtgtggtttgccagcagtcagccacacaacgactggaacatgcattcaacatcgccagatatcaattaggcatagagaaactactcgatcctgaagatgttgataccacctatccagataagaagtccatcttaatgtacatcacatcactcttccaagttttgcctcaacaagtgagcattgaagccatccaggaagtggaaatgttgccaaggccacctaaagtgactaaagaagaacattttcagttacatcatcaaatgcactattctcaacagatcacggtcagtctagcacagggatatgagagaacttcttcccctaagcctcgattcaagagctatgcctacacacaggctgcttatgtcaccacctctgaccctacacggagcccatttccttcacagcatttggaagctcctgaagacaagtcatttggcagttcattgatggagagtgaagtaaacctggaccgttatcaaacagctttagaagaagtattatcgtggcttctttctgctgaggacacattgcaagcacaaggagagatttctaatgatgtggaagtggtgaaagaccagtttcatactcatgaggggtacatgatggatttgacagcccatcagggccgggttggtaatattctacaattgggaagtaagctgattggaacaggaaaattatcagaagatgaagaaactgaagtacaagagcagatgaatctcctaaattcaagatgggaatgcctcagggtagctagcatggaaaaacaaagcaattacatagagaaatttcttatgtgccttctacttatttgactgaaatcactcatgtctcacaagccctattagaagtggaacaacttctcaatgctcctgacctctgtgctaaggactttgaagatctctttaagcaagaggagtctctgaagaatataaaagatagtctacaacaaagctcaggtcggattgacattattcatagcaagaagacagcagcattgcaaagtgcaacgcctgtggaaagggtgaagctacaggaagctctctcccagcttgatttccaatgggaaaaagttaacaaaatgtacaaggaccgacaagggcgatttgacagatctgttgagaaatggcggcgttttcattatgatataaagatatttaatcagtggctaacagaagctgaacagtttctcagaaagacacaaattcctgagaattgggaacatgctaaatacaaatggtatcttaaggaactccaggatggcattgggcagcggcaaactgttgtcagaacattgaatgcaactggggaagaaataattcagcaatcctcaaaaacagatgccagtattctacaggaaaaattgggaagcctgaatctgcggtggcaggaggtctgcaaacagctgtcagacagaaaaaagaggctagaagaaacccttgaaagactccaggaacttcaagaggccacggatgagctggacctcaagctgcgccaagctgaggtgatcaagggatcctggcagcccgtgggcgatctcctcattgactctctccaagatcacctcgagaaagtcaaggcacttcgaggagaaattgcgcctctgaaagagaacgtgagccacgtcaatgaccttgctcgccagcttaccactttgggcattcagctctcaccgtataacctcagcactctggaagacctgaacaccagatggaagcttctgcaggtggccgtcgaggaccgagtcaggcagctgcatgaagcccacagggactttggtccagcatctcagcactttctttccacgtctgtccagggtccctgggagagagccatctcgccaaacaaagtgccctactatatcaaccacgagactcaaacaacttgctgggacgatcccaaaatgacagagctctaccagtctttagctgacctgaataatgtcagattctcagcttataggactgccatgaaactccgaagactgcagaaggccctttgcttggatctcttgagcctgtcagctgcatgtgatgccttggaccagcacaacctcaagcaaaatgaccagcccatggatatcctgcagattattaattgtttgaccactatttatgaccgcctggagcaagagcacaacaatttggtcaacgtccctctctgcgtggatatgtgtctgaactggctgctgaatgtttatgatacgggacgaacagggaggatccgtgtcctgtcttttaaaactggcatcatttccctgtgtaaagcacatttggaagacaagtacagataccttttcaagcaagtggcaagttcaacaggattttgtgaccagcgcaggctgggcctccttctgcatgattctatccaaattccaagacagttgggtgaagttgcatcctttgggggcagtaacattgagccaagtgtccggagctgcttccaatttgctaataataagccagagatcgaagcggccctcttcctagactggatgagactggaaccccagtccatggtgtggctgcccgtcctgcacagagtggctgctgcagaaactgccaagcatcaggccaaatgtaacatctgcaaagagtgtccaatcattggattcaggtacaggagtctaaagcactttaattatgacatctgccaaagctgctttttttctggtcgagttgcaaaaggccataaaatgcactatcccatggtggaatattgcactccgactacatcaggagaagatgttcgagactttgccaaggtactaaaaaacaaatttcgaaccaaaaggtattttgcgaagcatccccgaatgggctacctgccagtgcagactgtcttagagggggacaacatggaaactgacacaatgtag

SEQ ID NO: 14 - DNA, 3439 bp, Artificial Sequence
  Synthetic
atgctttggtgggaagaagtagaggactgttatgaaagagaagatgttcaaaagaaaacattcacaaaatgggtaaatgcacaattttctaagtttgggaagcagcatattgagaacctcttcagtgacctacaggatgggaggcgcctcctagacctcctcgaaggcctgacagggcaaaaactgccaaaagaaaaaggatccacaagagttcatgccctgaacaatgtcaacaaggcactgcgggttttgcagaacaataatgttgatttagtgaatattggaagtactgacatcgtagatggaaatcataaactgactcttggtttgatttggaatataatcctccactggcaggtcaaaaatgtaatgaaaaatatcatggctggattgcaacaaaccaacagtgaaaagattctcctgagctgggtccgacaatcaactcgtaattatccacaggttaatgtaatcaacttcaccaccagctggtctgatggcctggctttgaatgctctcatccatagtcataggccagacctatttgactggaatagtgtggtttggcagcagtcagccacacaacgactggaacatgcattcaacatcgccagatatcaattaggcatagagaaactactcgatcctgaagatgttgataccacctatccagataagaagtccatcttaatgtacatcacatcactcttccaagttttgcctcaacaagtgagcatgaagccatccaggaagtggaaatgttgccaaggccacctaaagtgactaaagaagaacattttcagttacatcatcaaatgcactattctcaacagatcacggtcagtctagcacagggatatgagagaacttcttcccctaagcctcgattcaagagctatgcctacacacaggctgcttatgtcaccacctctgaccctacacggagcgcatttccttcacagcatttggaagctcctgaagacaagtcatttggcagttcattgatggagagtgaagtaaacctggaccgttatcaaacagctttagaagaagtattatcgtggcttctttctgctgaggacacattgcaagcacaaggagagatttctaatgatgtggaagtggtgaaagaccagtttcatactcatgaggggtacatgatggatttgacagcccatcagggccgggttggtaatattctacaattgggaagtaagctgattggaacaggaaaattatcagaagatgaagaaactgaagtacaagagcagatgaatctcctaaattcaagatgggaatgcctcagggtagctagcatggaaaaacaaagcaatttacatagagttttaatggatctccagaatcagaaactgaaagagttgaatgactggctaacaaaaacagaagaaagaacaaggaaaatggaggaagagcctcttggacctgatcttgaagacctaaaacgccaagtacaacaacataaggtgcttcaagaagatctagaacaagaacaagtcagggtcaattctctcactcacatggtggtggtagttgatgaatctagtggagatcacgcaactgctgctttggaagaacaacttaaggtattgggagatcgatgggcaaacatctgtagatggacagaagaccgctgggttcttttacaagacgaaatttcttatgtgccttctacttatttgactgaaatcactcatgtctcacaagccctattagaagtggaacaacttctcaatgctcctgacctctgtgctaaggactttgaagatctctttaagcaagaggagtctctgaagaatataaaagatagtctacaacaaagctcaggtcggattgacattattcatagcaagaagacagcagcattgcaaagtgcaacgcctgtggaaagggtgaagctacaggaagctctctcccagcttgatttccaatgggaaaaagttaacaaaatgtacaaggaccgacaagggcgatttgacagaacccttgaaagactccaggaacttcaagaggccacggatgagctggacctcaagctgcgccaagctgaggtgatcaagggatcctggcagcccgtgggcgatctcctcattgactctctccaagatcacctcgagaaagtcaaggcacttcgaggagaaattgcgcctctgaaagagaacgtgagccacgtcaatgaccttgctcgccagcttaccactttgggcattcagctctcaccgtataacctcagcactctggaagacctgaacaccagatggaagcttctgcaggtggccgtcgaggaccgagtcaggcagctgcatgaagcccacagggactttggtccagcatctcagcactttctttccacgtctgtccagggtccctgggagagagccatctcgccaaacaaagtgccctactatatcaaccacgagactcaaacaacttgctgggaccatcccaaaatgacagagctctaccagtctttagctgacctgaataatgtcagattctcagcttataggactgccatgaaactccgaagactgcagaaggccctttgcttggatctcttgagcctgtcagctgcatgtgatgccttggaccagcacaacctcaagcaaaatgaccagcccatggatatcctgcagattattaattgtttgaccactatttatgaccgcctggagcaagagcacaacaatttggtcaacgtccctctctgcgtggatatgtgtctgaactggctgctgaatgtttatgatacgggacgaacagggaggatccgtgtcctgtcttttaaaactggcatcatttccctgtgtaaagcacatttggaagacaagtacagataccttttcaagcaagtggcaagtcaacaggattttgtgaccagcgcaggctgggcctccttctgcatgattctatccaaattccaagacagttgggtgaagttgcatcctttgggggcagtaacattgaggcaagtgtccggagctgcttccaatttgctaataataagccagagatcgaagcggccctcttcctagactggatgagactggaaccccagtccatggtgtggctgcccgtcctgcacagagtggctgctgcagaaactgccaagcatcaggccaaatgtaacatctgcaaagagtgtccaatcattggattcaggtacaggagtctaaagcactttaattatgacatctgccaaagctgctttttttctggtcgagttgcaaaaggccataaaatgcactatcccatggtggaatattgcactccgactacatcaggagaagatgttcgagactttgccaaggtactaaaaaacaaatttcgaaccaaaaggtattttgcgaagcatccccgaatgggctacctgccagtgcagactgtcttagagggggacaacatggaaactgacacaatgtag

SEQ ID NO: 15 - DNA, 8312 bp, Artificial Sequence
  Synthetic
cattaatgaatcggccaacgcgcggggagaggcggtttgcgtattgggcgctcttccgcttcctcgctcactgactcgctgcgctcggtcgttcggctgcggcgagcggtatcagctcactcaaaggcggtaatacggttatccacagaatcaggggataacgcaggaaagaacatgtgagcaaaaggccagcaaaaggccaggaaccgtaaaaaggccgcgttgctggcgttttccataggctccgcccccctgacgagcatcacaaaaatcgacgctcaagtcagaggtggcgaaacccgacaggactataaagataccaggcgtttccccctggaagctccctcgtgcgctctcctgttccgaccctgccgcttaccggatacctgtccgcctttctcccttcgggaagcgtggcgctttctcatagctcacgctgtaggtatctcagttcggtgtaggtcgttcgctccaagctgggctgtgtgcacgaaccccccgttcagcccgaccgctgcgccttatccggtaactatcgtcttgagtccaacccggtaagacacgacttatcgccactggcagcagccactggtaacaggattagcagagcgaggtatgtaggcggtgctacagagttcttgaagtggtggcctaactacggctacactagaaggacagtatttggtatctgcgctctgctgaagccagttaccttcggaaaaagagttggtagctcttgatccggcaaacaaaccaccgctggtagcggtggtttttttgtttgcaagcagcagattacgcgcagaaaaaaaggatctcaagaagatcctttgatcttttctacggggtctgacgctcagtggaacgaaaactcacgttaagggattttggtcatgagattatcaaaaaggatcttcacctagatccttttaaattaaaaatgaagttttaaatcaatctaaagtatatatgagtaaacttggtctgacagttaccaatgcttaatcagtgaggcacctatctcagcgatctgtctatttcgttcatccatagttgcctgactccccgtcgtgtagataactacgatacgggagggcttaccatctggccccagtgctgcaatgataccgcgagacccacgctgaccggctccagatttatcagcaataaaccagccagccggaagggccgagcgcagaagtggtcctgcaagtttatccgcctccatccagtgtattaattgttgccgggaagctagagtaagtagttcgccagttaatagtttgcgcaacgttgttgccattgctacaggcatcgtggtgtcaggctcgtcgtttggtatggcttcattcagctccggttcccaacgatcaaggcgagttacatgatcccccatgttgtgcaaaaaagcggttagctccttcggtcctccgatcgttgtcagaagtaagttggccgcagtgttatcactcatggttatggcagcactgcataattctcttactgtcatgccatccgtaagatgcttttctgtgactggtgagtactcaaccaagtcattctgagaatagtgtatgcggcgaccgagttgctcttgcccggcgtcaatacgggataataccgcgccacatagcagaactttaaaagtgctcatcattggaaaacgttcttcggggcgaaaactctcaaggatcttaccgctgttgagatccagtcgatgtaacccactcgtgcacccaactgatcttcagcatcttttactttcaccagcgtttctgggtgagcaaaaacaggaaggcaaaatgccgcaaaaaagggaataagggcgacacggaaatgttgatactcatactcttcctttttcaatattattgaagcatttatcagggttattgtctcatgagcggatacatatttgaatgtatttagaaaaataaacaaataggggttccgcgcacatttccccgaaaagtgccacctgacgtctaagaaaccattattatcatgacattaacctataaaaataggcgtatcacgaggccctttcgtctcgcgcgtttcggtgatgacggtgaaaagctctgacacatgcagctcccggagacggtcacagcttgtctgtaagcggatgccgggagcagacaagcccgtcagggcgcgtcagcgggtgttggcgggtgtcggggctggcttaactatgcggcatcagagcagattgtactgagagtgcaccatatgcggtgtgaaataccgcacagatgcgtaaggagaaaataccgcatcaggaattccaacatccaataaatcatacaggcaaggcaaagaattagcaaaattaagcaataaagcctcagagcataaagctaaatcggttgtaccaaaaacattatgaccctgtaatacttttgcgggagaagcctttatttcaacgcaaggataaaaatttttagaaccctcatatattttaaatgcaatgcctgagtaatgtgtaggtaaagattcaaacgggtgagaaaggccggagacagtcaaatcaccatcaatatgatattcaaccgttctagctgataaattcatgccggagagggtagctatttttgagaggtctctacaaaggctatcaggtcattgcctgagagtctggagcaaacaagagaatcgatgaacggtaatcgtaaaactagcatgtcaatcatatgtaccccggttgataatcagaaaagccccaaaaacaggaagattgtataagcaaatatttaaattgtaaacgttaatattttgttaaaattcgcgttaaatttttgtaaatcagctcattttttaaccaataggccgaaatcggcaaaatcccttataaatcaaaagaatagaccgagatagggttgagtgttgttccagtttggaacaagagtccactattaaagaacgtggactccaacgtcaaagggcgaaaaaccgtctatcagggcgatggcccactacgtgaaccatcaccctaatcaagttttttggggtcgaggtgccgtaaagcactaaatcggaaccctaaagggagcccccgatttagagcttgacggggaaagccggcgaacgtggcgagaaaggaagggaagaaagcgaaaggagcgggcgctagggcgctggcaagtgtagcggtcacgctgcgcgtaaccaccacacccgccgcgcttaatgcgccgctacagggcgcgtactatggttgctttgacgagcaggtataacgtgctttcctcgttagaatcagagcgggagctaaacaggaggccgattaaagggattttagacaggaacggtacgccagaatcctgagaagtgtttttataatcagtgaggccaccgagtaaaagagtctgtcgatcacgcaaattaaccgttgtcgcaatacttctttgattagtaataacatcacttgcctgagtagaagaactcaaactatcggccttgctggtaatatccagaacaatattaccgccagccattgcaagaggaaaaacgctcatggaaatacctacattttgacgctcaatcgtctggaattccattcgccattcaggctgcgcaactgttgggaagggcgatcggtgcgggcctcttcgctattacgccagctggcgcgctcgctcgctcactgaggccgcccgggcaaagcccgggcgtcgggcgacctttggtcgcccggcctcagtgagcgagcgagcgcgcagagagggagtggccaactccatcactaggggttccttgtagttaatgattaacccgccatgctacttatctacggccgcggtaccgcgttacataacttacggtaaatggcccgcctggctgaccgcccaacgacccccgcccattgacgtcaataatgacgtatgttcgcatagtaacgccaatagggactttccattgacgtcaatgggtggagtatttacggtaaactgcccacttggcagtacatcaagtgtatcatatgccaagtacgccccctattgacgtcaatgacggtaaatggcccgcctggcattatgcccagtacatgaccttatgggactttcctacttggcagtacatctacgtattagtcatcgctattaccatggtgatgcggttttggcagtacatcaatgggcgtggatagcggtttgactcacggggatttccaagtctccaccccattgacgtcaatgggagtttgttttggcaccaaaatcaacgggactttccaaaatgtcgtaacaactccgccccattgacgcaaatgggcggtaggcgtgtacggtgggaggtctatataagcagagctcgtttagtgaaccgtctagacggccgcggttttttttatcgctgccttgatatacactttccaccatgctttggtgggaagaagtagaggactgttatgaaagagaagatgttcaaaagaaaacattcacaaaatgggtaaatgcacaattttctaagtttgggaagcagcatattgagaacctcttcagtgacctacaggatgggaggggcctcctagacctcctcgaaggcctgacagggcaaaaactgccaaaagaaaaaggatccacaagagttcatgccctgaacaatgtcaacaaggcactgcgggttttgcagaacaataatgttgatttagtgaatattggaagtactgacatcgtagatggaaatcataaactgactcttggtttgatttggaatataatcctccactggcaggtcaaaaatgtaatgaaaaatatcatggctggattgcaacaaaccaacagtgaaaagattctcctgagctgggtccgacaatcaactcgtaattatccacaggttaatgtaatcaacttcaccaccagctggtctgatggcctggctttgaatgctctcatccatagtcataggccagacctatttgactggaatagtgtggtttgccagcagtcagccacacaacgactggaacatgcattcaacatcgccagatatcaattaggcatagagaaactactcgatcctgaagatgttgataccacctatccagataagaagtccatcttaatgtacatcacatcactcttccaagttttgcctcaacaagtgagcattgaagccatccaggaagtggaaatgttgccaaggccacctaaagtgactaaagaagaacattttcagttacatcatcaaatgcactattctcaacagatcacggtcagtctagcacagggatatgagagaacttcttcccctaagcctcgattcaagagctatgcctacacacaggctgcttatgtcaccacctctgaccctacacggagcccatttccttcacagcatttggaagctcctgaagacaagtcatttggcagttcattgatggagagtgaagtaaacctggaccgttatcaaacagctttagaagaagtattatcgtggcttctttctgctgaggacacattgcaagcacaaggagagatttctaatgatgtggaagtggtgaaagaccagtttcatactcatgaggggtacatgatggatttgacagcgcatcagggccgggttggtaatattctacaattgggaagtaagctgattggaacaggaaaattatcagaagatgaagaaactgaagtacaagagcagatgaatctcctaaattcaagatgggaatgcctcagggtagctagcatggaaaaacaaagcaatttacatagagaaatttcttatgtgccttctacttatttgactgaaatcactcatgtctcacaagccctattagaagtggaacaacttctcaatgctcctgacctctgtgctaaggactttgaagatctctttaagcaagaggagtctctgaagaatataaaagatagtctacaacaaagctcaggtcggattgacattattcatagcaagaagacagcagcattgcaaagtgcaacgcctgtggaaagggtgaagctacaggaagctctctccgagcttgatttccaatgggaaaaagttaacaaaatgtacaaggaccgacaagggcgatttgacagatctgttgagaaatggcggcgttttcattatgatataaagatatttaatcagtggctaacagaagctgaacagtttctcagaaagagacaaattcctgagaattgggaacatgctaaatacaaatggtatcttaaggaactccaggatggcattgggcagcggcaaactgttgtcagaacattgaatgcaactggggaagaaataattcagcaatcctcaaaaacagatgccagtattctacaggaaaaattgggaagcctgaatctgcggtggcaggaggtctgcaaacagctgtcagacagaaaaaagaggctagaagaaacccttgaaagactccaggaacttcaagaggccacggatgaggtggacctcaagctgcgccaagctgaggtgatcaagggatcctggcagcccgtgggcgatctcctcattgactctctccaagatcacctcgagaaagtcaaggcacttcgaggagaaattgcgcctctgaaagagaacgtgagccacgtcaatgaccttgctcgccagcttaccactttgggcattcagctctcaccgtataacctcagcactctggaagacctgaacaccagatggaagcttctgcaggtggccgtcgaggaccgagtcaggcagctgcatgaagcccacagggactttggtccagcatctcagcactttctttccacgtctgtccagggtccctgggagagagccatctcgccaaacaaagtgccctactatatcaaccacgagactcaaacaacttgctgggaccatcccaaaatgacagagctctaccagtctttagctgacctgaataatgtcagattctcagcttataggactgccatgaaactccgaagactgcagaaggccctttgcttggatctcttgagcctgtcagctgcatgtgatgccttggaccagcacaacctcaagcaaaatgaccagcccatggatatcctgcagattattaattgtttgaccactatttatgaccgcctggagcaagagcacaacaatttggtcaacgtccctctctgcgtggatatgtgtctgaactggctgctgaatgtttatgatacgggacgaacagggaggatccgtgtcctgtcttttaaaactggcatcatttccctgtgtaaagcacatttggaagacaagtacagataccttttcaagcaagtggcaagttcaacaggattttgtgaccagcgcaggctgggcctccttctgcatgattctatccaaattccaagacagttgggtgaagttgcatcctttgggggcagtaacattgagccaagtgtccggagctgcttccaatttgctaataataagccagagatcgaagcggccctcttcctagactggatgagactggaaccccagtccatggtgtggctgcccgtcctgcacagagtggctgctgcagaaactgccaagcatcaggccaaatgtaacatctgcaaagagtgtccaatcattggattcaggtacaggagtctaaagcactttaattatgacatctgccaaagctgctttttttctggtcgagttgcaaaaggccataaaatgcactatcccatggtggaatattgcactccgactacatcaggagaagatgttcgagactttgccaaggtactaaaaaacaaatttcgaaccaaaaggtattttgcgaagcatccccgaatgggctacctgccagtgcagactgtcttagagggggacaacatggaaactgacacaatgtaggaagtcttttccacatggcagatgatttgggcagagcgatggagtccttagtatcagtcatgacagatgaagaaggagcagaataaatgttttacaactcctgattcccgcatgcggccgatccagacatgataagatacattgatgagtttggacaaaccacaactagaatgcagtgaaaaaaatgctttatttgtgaaatttgtgatgctattgctttatttgtaaccattataagctgcaataaacaagttaacaacaacaattgcattcattttatgtttcaggttcagggggaggtgtgggaggttttttgcggccgtagataagtagcatggcgggttaatcattaactacaaggaacccctagtgatggagttggccactccctctctgcgcgctcgctcgctcactgaggccgggcgaccaaaggtcgcccgacgcccgggctttgcccgggcggcctcagtgagcgagcgagcgcgcagctgctg

SEQ ID NO: 16 - DNA, 8293 bp, Artificial Sequence
  Synthetic
cattaatgaatcggccaacgcgcggggagaggcggtttgcgtattgggcgctcttccgcttcctcgctcactgactcgctgcgctcggtcgttcggctgcggcgagcggtatcagctcactcaaaggcggtaatacggttatccacagaatcaggggataacgcaggaaagaacatgtgagcaaaaggccagcaaaaggccaggaaccgtaaaaaggccgcgttgctggcgtttttccataggctccgcccccctgacgagcatcacaaaaatcgacgctcaagtcagaggtggcgaaacccgacaggactataaagataccaggcgtttccccctggaagctccctcgtgcgctctcctgttccgaccctgccgcttaccggatacctgtccgcctttctcccttcgggaagcgtggcgctttctcatagctcacgctgtaggtatctcagttcggtgtaggtcgttcgctccaagctgggctgtgtgcacgaaccccccgttcagcccgaccgctgcgccttatccggtaactatcgtcttgagtccaacccggtaagacacgacttatcgccactggcagcagccactggtaacaggattagcagagcgaggtatgtaggcggtgctacagagttcttgaagtggtggcctaactacggctacactagaaggacagtatttggtatctgcgctctgctgaagccagttaccttcggaaaaagagttggtagctcttgatccggcaaacaaaccaccgctggtagcggtggtttttttgtttgcaagcagcagattacgcgcagaaaaaaaggatctcaagaagatcctttgatcttttctacggggtctgacgctcagtggaacgaaaactcacgttaagggattttggtcatgagattatcaaaaaggatcttcacctagatccttttaaattaaaaatgaagttttaaatcaatctaaagtatatatgagtaaacttggtctgacagttaccaatgcttaatcagtgaggcacctatctgagcgatctgtctatttcgttcatccatagttgcctgactccccgtcgtgtagataactacgatacgggagggcttaccatctggccccagtgctgcaatgataccgcgagacccacgctgaccggctccagatttatcagcaataaaccagccagccggaagggccgagcgcagaagtggtcctgcaactttatccgcctccatccagtctattaattgttgccgggaagctagagtaagtagttcgccagttaatagtttgcgcaacgttgttgccattgctacaggcatcgtggtgtcacgctcgtcgtttggtatggcttcattcagctccggttcccaacgatcaaggcgagttacatgatcccccatgttgtgcaaaaaagcggttagctccttcggtcctccgatcgttgtcagaagtaagttggccgcagtgttatcactcatggttatggcagcactgcataattctcttactgtcatgccatccgtaagatgcttttctgtgactggtgagtactcaaccaagtcattctgagaatagtgtatgcggcgaccgagttgctcttgcccggcgtcaataggggataataccgcgccacatagcagaactttaaaagtgctcatcattggaaaacgttcttcggggcgaaaactctcaaggatcttaccgctgttgagatccagttcgatgtaacccactcgtgcacccaactgatcttcagcatcttttactttcaccagcgtttctgggtgagcaaaaacaggaaggcaaaatgccgcaaaaaagggaataagggcgacacggaaatgttgaatactcatactcttcctttttcaatattattgaagcatttatcagggttattgtctcatgagcggatacatatttgaatgtatttagaaaaataaacaaataggggttccgcgcacatttccccgaaaagtgccacctgacgtctaagaaaccattattatcatgacattaacctataaaaataggcgtatcacgaggccctttcgtctcgcgcgtttcggtgatgacggtgaaaacctctgacacatgcagctcccggagacggtcacagcttgtctgtaagcggatgccgggagcagacaagcccgtcagggcgcgtcagcgggtgttggcgggtgtcggggctggcttaactatgcggcatcagagcagattgtactgagagtgcaccatatgcggtgtgaaataccgcacagatgcgtaaggagaaaataccgcatcaggaattccaacatccaataaatcatacaggcaaggcaaagaattagcaaaattaagcaataaagcctcagagcataaagctaaatcggttgtaccaaaaacattatgaccctgtaatacttttgcgggagaagcctttatttcaacgcaaggataaaaatttttagaaccctcatatattttaaatgcaatgcctgagtaatgtgtaggtaaagattcaaacgggtgagaaaggccggagacagtcaaatcaccatcaatatgatattcaaccgttctagctgataaattcatgccggagagggtagctatttttgagaggtctctacaaaggctatcaggtcattgcctgagagtctggagcaaacaagagaatcgatgaacggtaatcgtaaaactagcatgtcaatcatatgtaccccggttgataatcagaaaagccccaaaaacaggaagattgtataagcaaatatttaaattgtaaacgttaatattttgttaaaattcgcgttaaatttttgttaaatcagctcattttttaaccaataggccgaaatcggcaaaatcccttataaatcaaaagaatagaccgagatagggttgagtgttgttccagtttggaacaagagtccactattaaagaacgtggactccaacgtcaaagggcgaaaaaccgtctatcagggcgatggcccactacgtgaaccatcaccctaatcaagttttttggggtcgaggtgccgtaaagcactaaatcggaaccctaaagggagcccccgatttagagcttgacggggaaagccggcgaacgtggcgagaaaggaagggaagaaagcgaaaggagcgggcgctagggcgctggcaagtgtagcggtcacgctgcgcgtaaccaccacacccgccgcgcttaatgcgccgctacagggcgcgtactatggttgctttgacgagcacgtataacgtgctttcctcgttagaatcagagcgggagctaaacaggaggccgattaaagggattttagacaggaacggtacgccagaatcctgagaagtgtttttataatcagtgaggccaccgagtaaaagagtctgtccatcacgcaaattaaccgttgtcgcaatacttcttgattagtaataacatcacttgcctgagtagaagaactcaaactatcggccttgctggtaatatccagaacaatattaccgccagccattgcaacaggaaaaacgctcatggaaatacctacattttgacgctcaatcgtctggaattccattcgccattcaggctgcgcaactgttgggaagggcgatcggtgcgggcctcttcgctattacgccagctggcgcgctcgctcgctcactgaggccgccggggcaaagcccgggcgtcgggcgacctttggtcgcccggcctcagtgagcgagcgagcgcgcagagagggagtggccaactccatcactaggggttccttgtagttaatgattaacccgccatgctacttatctacggccgcggtaccactcacggggatttccaagtctccaccccattgacgtcaatgggagtttgttttggcaccaaaatcaacgggactttccaaaatgtcgtaataaccccgccccgttgacgcaaatgggcggtaggcgtgtacggtgggaggtctatataagcagagctcgtttagtgaaccgtctctagacggccgcggttttttttatcgctgccttgatatacactttccaccatgctttggtgggaagaagtagaggactgttatgaaagagaagatgttcaaaagaaaacattcacaaaatgggtaaatgcacaattttctaagtttgggaagcagcatattgagaacctcttcagtgacctacaggatgggaggcgcctcctagacctcctcgaaggcctgacagggcaaaaactgccaaaagaaaaaggatccacaagagttcatgccctgaacaatgtcaacaaggcactgcgggttttgcagaacaataatgttgatttagtgaatattggaagtactgacatcgtagatggaaatcataaactgactcttggtttgatttggaatataatcctccactggcaggtcaaaaatgtaatgaaaaatatcatggctggattgcaacaaaccaacagtgaaaagattctcctgagctgggtccgacaatcaactcgtaattatccacaggttaatgtaatcaacttcaccaccagctggtctgatggcctggctttgaatgctctcatccatagtcataggccagacctatttgactggaatagtgtggtttgccagcagtcagccacacaacgactggaacatgcattcaacatcgccagatatcaattaggcatagagaaactactcgatcctgaagatgttgataccacctatccagataagaagtccatcttaatgtacatcacatcactcttccaagttttgcctcaacaagtgagcattgaagccatccaggaagtggaaatgttgccaaggccacctaaagtgactaaagaagaacattttcagttacatcatcaaatgcactattctcaacagatcacggtcagtctagcacagggatatgagagaagttcttcccctaagcctcgattcaagagctatgcctacacacaggctgcttatgtcaccacctctgaccctacacggagcccatttccttcacagcatttggaagctcctgaagacaagtcatttggcagttcattgatggagagtgaagtaaacctggaccgttatcaaacagctttagaagaagtattatcgtggcttctttctgctgaggacacattgcaagcacaaggagagatttctaatgatgtggaagtggtgaaagaccagtttcatactcatgaggggtacatgatggatttgacagcccatcagggccgggttggtaatattctacaattgggaagtaagctgattggaacaggaaaattatcagaagatgaagaaactgaagtacaagagcagatgaatctcctaaattcaagatgggaatgcctcagggtagctagcatggaaaaacaaagcaatttacatagagttttaatggatctccagaatcagaaactgaaagagttgaatgactggctaacaaaaacagaagaaagaacaaggaaaatggaggaagagcctcttggacctgatcttgaagacctaaaacggcaagtacaacaacataaggtgcttcaagaagatctagaacaagaacaagtcagggtcaattctctcactcacatggtggtggtagttgatgaatctagtggagatcacgcaactgctgctttggaagaacaacttaaggtattgggagatcgatgggcaaacatctgtagatggacagaagaccgctgggttcttttacaagacgaaatttcttatgtgccttctacttatttgactgaaatcactcatgtctcacaagccctattagaagtggaacaacttctcaatgctcctgacctctgtgctaaggactttgaagatctctttaagcaagaggagtctctgaagaatataaaagatagtctacaacaaagctcaggtcggattgacattattcatagcaagaagacagcagcattgcaaagtgcaacgcctgtggaaagggtgaagctacaggaagctctctcccagcttgatttccaatgggaaaaagttaacaaaatgtacaaggaccgacaagggcgatttgacagatctgttgagaaatggcggcgttttcattatgatataaagatatttaatcagtggctaacagaagctgaacagtttctcagaaagacacaaattcctgagaattgggaacatgctaaatacaaatggtatcttaaggaactccaggatggcattgggcagcggcaaactgttgtcagaacattgaatgcaactggggaagaaataattcagcaatcgtcaaaaacagatgccagtattctacaggaaaaattgggaagcctgaatctgcggtggcaggaggtctgcaaacagctgtcagacagaaaaaagaggctagaagaaacccttgaaagactccaggaacttcaagaggccacggatgagctggacctcaagctgcgccaagctgaggtgatcaagggatcctggcagcccgtgggcgatctcctcattgactctctccaagatcacctcgagaaagtcaaggcacttcgaggagaaattgcgcctctgaaagagaacgtgagccacgtcaatgaccttgctcgccagcttaccactttgggcattcaggtctcacggtataacctcagcactctggaagacctgaacaccagatggaagcttctgcaggtggccgtcgaggaccgagtcaggcagctgcatgaagcccacagggactttggtccagcatctcagcactttctttccacgtctgtccagggtccctgggagagagccatctcgccaaacaaagtgccctactatatcaaccacgagactcaaacaacttgctgggaccatcccaaaatgacagagctctaccagtctttagctgacctgaataatgtcagattctcagcttataggactgccatgaaactccgaagactgcagaaggccctttgcttggatctcttgagcctgtcagctgcatgtgatgccttggaccagcacaacctcaagcaaaatgaccagcccatggatatcctgcagattattaattgtttgaccactatttatgaccgcctggagcaagagcacaacaatttggtcaacgtccctctctgcgtggatatgtgtctgaactggctgctgaatgtttatgatacgggacgaacagggaggatccgtgtcctgtcttttaaaactggcatcatttccctgtgtaaagcacatttggaagacaagtacagataccttttcaagcaagtggcaagttcaacaggattttgtgaccagcgcaggctgggcctccttctgcatgattctatccaaattccaagacagttgggtgaagttgcatcctttgggggcagtaacattgagccaagtgtccggagctgcttccaatttgctaataataagccagagatcgaagcggccctcttcctagactggatgagactggaaccgcagtccatggtgtggctgcccgtcctgcacagagtggctgctgcagaaactgccaagcatcaggccaaatgtaacatctgcaaagagtgtccaatcattggattcaggtacaggagtctaaagcactttaattatgacatctgccaaagctgctttttttctggtcgagttgcaaaaggccataaaatgcactatcccatggtggaatattgcactccgactacatcaggagaagatgttcgagactttgccaaggtactaaaaaacaaatttcgaaccaaaaggtattttgcgaagcatccccgaatgggctacctgccagtgcagactgtcttagagggggacaacatggaaactgacacaatgtaggaagtcttttccacatggcagatgatttgggcagagcgatggagtccttagtatcagtcatgacagatgaagaaggagcagaataaatgttttacaactcctgattcccgcatgcggccgatccagacatgataagatacattgatgagtttggacaaaccacaactagaatgcagtgaaaaaaatgctttatttgtgaaatttgtgatgctattgctttatttgtaaccattataagctgcaataaacaagttaacaacaacaattgcattcattttatgtttcaggttcagggggaggtgtgggaggttttttgcggccgtagataagtagcatggcgggttaatcattaactacaaggaacccctagtgatggagttggccactccctctctgcgcgctcggtcgctcactgaggccgggcgaccaaaggtcgcccgacgcccgggctttgcccgggcggcctcagtgagcgagcgagcgcgcagctgctg

SEQ ID NO: 17 - DNA, 756 bp, Homo sapiens
atgctttggtgggaagaagtagaggactgttatgaaagagaagatgttcaaaagaaaacattcacaaaatgggtaaatgcacaattttctaagtttgggaagcagcatattgagaacctcttcagtgacctacaggatgggaggcgcctcctagacctcctcgaaggcctgacagggcaaaaactgccaaaagaaaaaggatccacaagagttcatggcctgaacaatgtcaacaaggcactgcgggttttgcagaacaataatgttgatttagtgaatattggaagtactgacatcgtagatggaaatcataaactgactcttggtttgatttggaatataatcctccactggcaggtcaaaaatgtaatgaaaaatatcatggctggattgcaacaaaccaacagtgaaaagattctcctgagctgggtccgacaatcaactcgtaattatccacaggttaatgtaatcaacttcaccaccagctggtctgatggcctggctttgaatgctctcatccatagtcataggccagacctatttgactggaatagtgtggtttgccagcagtcagccacacaacgactggaacatgcattcaacatcgccagatatcaattaggcatagagaaactactcgatcctgaagatgttgataccacctatccagataagaagtccatcttaatgtacatcacatcactcttccaagttttgcctcaacaagtgagcattgaagccatccaggaagtggaa

SEQ ID NO: 18 - DNA, 252 bp, Homo sapiens
atgttgccaaggccacctaaagtgactaaagaagaacattttcagttacatcatcaaatgcactattctcaacagatcacggtcagtctagcacagggatatgagagaacttcttcccctaagcctcgattcaagagctatgcctacacacaggctgcttatgtcaccacctctgaccctacacggagcccatttccttcacagcatttggaagctcctgaagacaagtcatttggcagttcattgatggag

SEQ ID NO: 19 - DNA, 333 bp, Homo sapiens
agtgaagtaaacctggaccgttatcaaacagctttagaagaagtattatcgtggcttctttctgctgaggacacattgcaagcacaaggagagatttctaatgatgtggaagtggtgaaagaccagtttcatactcatgaggggtacatgatggatttgacagcccatcagggccgggttggtaatattctacaattgggaagtaagctgattggaacaggaaaattatcagaagatgaagaaactgaagtacaagagcagatgaatctcctaaattcaagatgggaatgcctcagggtagctagcatggaaaaacaaagcaatttacataga

SEQ ID NO: 20 - DNA, 327 bp, Homo sapiens
gttttaatggatctccagaatcagaaactgaaagagttgaatgactggctaacaaaaacagaagaaagaacaaggaaaatggaggaagagcctcttggacctgatcttgaagacctaaaacgccaagtacaacaacataaggtgcttcaagaagatctagaacaagaacaagtcagggtcaattctctcactcacatggtggtggtagttgatgaatctagtggagatcacgcaactgctgctttggaagaacaacttaaggtattgggagatcgatgggcaaacatctgtagatggacagaagaccgctgggttcttttacaagac

SEQ ID NO: 21 - DNA, 333 bp, Homo sapiens
atccttctcaaatggcaacgtcttactgaagaacagtgcctttttagtgcatggctttcagaaaaagaagatgcagtgaacaagattcacacaactggctttaaagatcaaaatgaaatgttatcaagtcttcaaaaactggccgttttaaaagcggatctagaaaagaaaaagcaatccatgggcaaactgtattcactcaaacaagatcttctttcaacactgaagaataagtcagtgacccagaagacggaagcatggctggataactttgcccggtgttgggataatttagtccaaaaacttgaaaagagtacagcacagatttcacag

SEQ ID NO: 22 - DNA, 150 bp, Homo sapiens
gctgtcaccaccactcagccatcactaacacagacaactgtaatggaaacagtaactacggtgaccacaagggaacagatcctggtaaagcatgctcaagaggaacttccaccaccacctccccaaaagaagaggcagattactgtggat

SEQ ID NO: 23 - DNA, 262 bp, Homo sapiens
tctgaaattaggaaaaggttggatgttgatataactgaacttcacagctggattactcgctcagaagctgtgttgcagagtcctgaatttgcaatctttcggaaggaaggcaacttctcagacttaaaagaaaaagtcaatgccatagagcgagaaaaagctgagaagttcagaaaactgcaagatgccagcagatcagctcaggccctggtggaacagatggtgaatgagggtgttaatgcagatagcatcaaacaagcct

SEQ ID NO: 24 - DNA, 389 bp, Homo sapiens
cagaacaactgaacagccggtggatcgaattctgccagttgctaagtgagagacttaactggctggagtatcagaacaacatcatcgctttctataatcagctacaacaattggagcagatgacaactactgctgaaaactggttgaaaatccaacccaccaccccatcagagccaacagcaattaaaagtcagttaaaaatttgtaaggatgaagtcaaccggctatcaggtcttcaacctcaaattgaacgattaaaaattcaaagcatagccctgaaagagaaaggacaaggacccatgttcctggatgcagactttgtggcctttacaaatcattttaagcaagtcttttctgatgtgcaggccagagagaaagagctacagaca

SEQ ID NO: 25 - DNA, 333 bp, Homo sapiens
atttttgacactttgccaccaatgcgctatcaggagaccatgagtgccatcaggacatgggtccagcagtcagaaaccaaactctccatacctcaacttagtgtcaccgactatgaaatcatggagcagagactcggggaattgcaggctttacaaagttctctgcaagagcaacaaagtggcctatactatctcagcaccactgtgaaagagatgtcgaagaaagcgccctctgaaattagccggaaatatcaatcagaatttgaagaaattgagggacgctggaagaagctctcctcccagctggttgagcattgtcaaaagctagaggag

SEQ ID NO: 26 - DNA, 327 bp, Homo sapiens
caaatgaataaactccgaaaaattcagaatcacatacaaaccctgaagaaatggatggctgaagttgatgtttttctgaaggaggaatggcctgcccttggggattcagaaattctaaaaaagcagctgaaacagtgcagacttttagtcagtgatattcagacaattcagcccagtctaaacagtgtcaatgaaggtgggcagaagataaagaatgaagcagagccagagtttgcttcgagacttgagacagaactcaaagaacttaacactcagtgggatcacatgtgccaacaggtctatgccagaaaggaggccttgaaggga

SEQ ID NO: 27 - DNA, 327 bp, Homo sapiens
ggtttggagaaaactgtaagcctccagaaagatctatcagagatgcacgaatggatgacacaagctgaagaagagtatcttgagagagattttgaatataaaactccagatgaattacagaaagcagttgaagagatgaagagagctaaagaagaggcccaacaaaaagaagcgaaagtgaaactccttactgagtctgtaaatagtgtcatagctcaagctccacctgtagcacaagaggccttaaaaaaggaacttgaaactctaaccaccaactaccagtggctctgcactaggctgaatgggaaatgcaagactttggaagaa

SEQ ID NO: 28 - DNA, 312 bp, Homo sapiens
gtttgggcatgttggcatgagttattgtcatacttggagaaagcaaacaagtggctaaatgaagtagaatttaaacttaaaaccactgaaaacattcctggcggagctgaggaaatctctgaggtgctagattcacttgaaaatttgatgcgacattcagaggataacccaaatcagattcgcatattggcacagaccctaacagatggcggagtcatggatgagctaatcaatgaggaacttgagacatttaattctcgttggagggaactacatgaagaggctgtaaggaggcaaaagttgcttgaacag

SEQ ID NO: 29 - DNA, 288 bp, Homo sapiens
agcatccagtctgcccaggagactgaaaaatccttacacttaatccaggagtccctcacattcattgacaagcagttggcagcttatattgcagacaaggtggacgcagctcaaatgcctcaggaagcccagaaaatccaatctgatttgacaagtcatgagatcagtttagaagaaatgaagaaacataatcaggggaaggaggctgcccaaagagtcctgtctcagattgatgttgcacagaaaaaattacaagatgtctccatgaagtttcgattattccagaaa

SEQ ID NO: 30 - DNA, 315 bp, Homo sapiens
ccagccaattttgagctgcgtctacaagaaagtaagatgattttagatgaagtgaagatgcacttgcctgcattggaaacaaagagtgtggaacaggaagtagtacagtcacagctaaatcattgtgtgaacttgtataaaagtctgagtgaagtgaagtctgaagtggaaatggtgataaagactggacgtcagattgtacagaaaaagcagacggaaaatcccaaagaacttgatgaaagagtaacagctttgaaattgcattataatgagctgggagcaaaggtaacagaaagaaagcaacagttggagaaa

SEQ ID NO: 31 - DNA, 324 bp, Homo sapiens
tgcttgaaattgtcccgtaagatgcgaaaggaaatgaatgtcttgacagaatggctggcagctacagatatggaattgacaaagagatcagcagttgaaggaatgcctagtaatttggattctgaagttgcctggggaaaggctactcaaaaagagattgagaaacagaaggtgcacctgaagagtatcacagaggtaggagaggccttgaaaacagttttgggcaagaaggagacgttggtggaagataaactcagtcttctgaatagtaactggatagctgtcacctcccgagcagaagagtggttaaatcttttgttggaa

SEQ ID NO: 32 - DNA, 306 bp, Homo sapiens
taccagaaacacatggaaacttttgaccagaatgtggaccacatcacaaagtggatcattcaggctgacacacttttggatgaatcagagaaaaagaaaccccagcaaaaagaagacgtgcttaagcgtttaaaggcagaactgaatgacatacgcccaaaggtggactctacacgtgaccaagcagcaaacttgatggcaaaccgcggtgaccactgcaggaaattagtagagccccaaatctcagagctcaaccatcgatttgcagccatttcacacagaattaagactggaaaggcctccatt

SEQ ID NO: 33 - DNA, 288 bp, Homo sapiens
cctttgaaggaattggagcagtttaactcagatatacaaaaattgcttgaaccactggaggctgaaattcagcagggggtgaatctgaaagaggaagacttcaataaagatatgaatgaagacaatgagggtactgtaaaagaattgttgcaaagaggagacaacttacaacaaagaatcacagatgagagaaagagagaggaaataaagataaaacagcagctgttacagacaaaacataatgctctcaaggatttgaggtctcaaagaagaaaaaaggctctagaa

SEQ ID NO: 34 - DNA, 297 bp, Homo sapiens
atttctcatcagtggtatcagtacaagaggcaggctgatgatctcctgaaatgcttggatgacattgaaaaaaaattagccagcctacctgagcccagagatgaaaggaaaataaaggaaattgatcgggaattgcagaagaagaaagaggagctgaatgcagtgcgtaggcaagctgagggcttgtctgaggatggggccgcaatggcagtggagccaactcagatccagctcagcaagcgctggcgggaaattgagagcaaatttgctcagtttcgaagactcaactttgcacaa

SEQ ID NO: 35 - DNA, 384 bp, Homo sapiens
attcacactgtccgtgaagaaacgatgatggtgatgactgaagacatgcctttggaaatttcttatgtgccttctacttatttgactgaaatcactcatgtctcacaagccctattagaagtggaacaacttctcaatgctcctgacctctgtgctaaggactttgaagatctctttaagcaagaggagtctctgaagaatataaaagatagtctacaacaaagctcaggtcggattgacattattcatagcaagaagacagcagcattgcaaagtgcaacgcctgtggaaagggtgaagctacaggaagctctctcccagcttgatttccaatgggaaaaagttaacaaaatgtacaaggaccgacaagggcgatttgacaga

SEQ ID NO: 36 - DNA, 321 bp, Homo sapiens
tctgttgagaaatggcggcgttttcattatgatataaagatatttaatcagtggctaacagaagctgaacagtttctcagaaagacacaaattcctgagaattgggaacatgctaaatacaaatggtatcttaaggaactccaggatggcattgggcagcggcaaactgttgtcagaacattgaatgcaactggggaagaaataattcagcaatcctcaaaaacagatgccagtattctacaggaaaaattgggaagcctgaatctgcggtggcaggaggtctgcaaacagctgtcagacagaaaaaagaggctagaagaa

SEQ ID NO: 37 - DNA, 330 bp, Homo sapiens
caaaagaatatcttgtcagaatttcaaagagatttaaatgaatttgttttatggttggaggaagcagataacattgctagtatcccacttgaacctggaaaagagcagcaactaaaagaaaagcttgagcaagtcaagttactggtggaagagttgcccctgcgccagggaattctcaaacaattaaatgaaactggaggacccgtgcttgtaagtgctcccataagcccagaagagcaagataaacttgaaaataagctcaagcagacaaatctccagtggataaaggtttccagagctttacctgagaaacaaggagaaattgaagct

SEQ ID NO: 38 - DNA, 315 bp, Homo sapiens
caaataaaagaccttgggcagcttgaaaaaaagcttgaagaccttgaagagcagttaaatcatctgctgctgtggttatctcctattaggaatcagttggaaatttataaccaaccaaaccaagaaggaccatttgacgttcaggaaactgaaatagcagttcaagctaaacaaccggatgtggaagagattttgtctaaagggcagcatttgtacaaggaaaaaccagccactcagccagtgaagaggaagttagaagatctgagctctgagtggaaggcggtaaaccgtttacttcaagagctgagggcaaag

SEQ ID NO: 39 - DNA, 141 bp, Homo sapiens
cagcctgacctagctcctggactgaccactattggagcctctcctactcagactgttactctggtgacacaacctgtggttactaaggaaactgccatctccaaactagaaatgccatcttccttgatgttggaggtacct

SEQ ID NO: 40 - DNA, 321 bp, Homo sapiens
gctctggcagatttcaaccgggcttggacagaacttaccgactggctttctctgcttgatcaagttataaaatcacagagggtgatggtgggtgaccttgaggatatcaacgagatgatcatcaagcagaaggcaacaatgcaggatttggaacagaggcgtccccagttggaagaactcattaccgctgcccaaaatttgaaaaacaagaccagcaatcaagaggctagaacaatcattacggatcgaattgaaagaattcagaatcagtgggatgaagtacaagaacaccttcagaaccggaggcaacagttgaatgaa

SEQ ID NO: 41 - DNA, 327 bp, Homo sapiens
atgttaaaggattcaacacaatggctggaagctaaggaagaagctgagcaggtcttaggacaggccagagccaagcttgagtcatggaaggagggtccctatacagtagatgcaatccaaaagaaaatcacagaaaccaagcagttggccaaagacctccgccagtggcagacaaatgtagatgtggcaaatgacttggccctgaaacttctccgggattattctgcagatgataccagaaaagtccacatgataacagagaatatcaatgcctcttggagaagcattcataaaagggtgagtgagcgagaggctgctttggaagaa

SEQ ID NO: 42 - DNA, 348 bp, Homo sapiens
actcatagattactgcaacagttccccctggacctggaaaagtttcttgcctggcttacagaagctgaaacaactgccaatgtcctacaggatgctacccgtaaggaaaggctcctagaagactccaagggagtaaaagagctgatgaaacaatggcaagacctccaaggtgaaattgaagctcacacagatgtttatcacaacctggatgaaaacagccaaaaaatcctgagatccctggaaggttccgatgatgcagtcctgttacaaagacgtttggataacatgaacttcaagtggagtgaacttcggaaaaagtctctcaacattaggtcccatttggaagcc

SEQ ID NO: 43 - DNA, 387 bp, Homo sapiens
agttctgaccagtggaagcgtctgcacctttctctgcaggaacttctggtgtggctacagctgaaagatgatgaattaagccggcaggcacctattggaggcgactttccagcagttcagaagcagaacgatgtacatagggccttcaagagggaattgaaaactaaagaacctgtaatcatgagtactcttgagactgtacgaatatttctgacagagcagcctttggaaggactagagaaactctaccaggagcccagagagctgcctcctgaggagagagcccagaatgtcactcggcttctacgaaagcaggctgaggaggtcaatactgagtgggaaaaattgaacctgcactccgctgactggcagagaaaaatagatgag

SEQ ID NO: 44 - DNA, 327 bp, Homo sapiens
acccttgaaagactccaggaacttcaagaggccacggatgagctggacctcaagctgcgccaagctgaggtgatcaagggatcctggcagcccgtgggcgatctcctcattgactctctccaagatcacctcgagaaagtcaaggcacttcgaggagaaattgcgcctctgaaagagaacgtgagccacgtcaatgaccttgctcgccagcttaccactttgggcattcagctctcaccgtataacctcagcactctggaagacctgaacaccagatggaagcttctgcaggtggccgtcgaggaccgagtcaggcagctgcatgaa

SEQ ID NO: 45 - DNA, 216 bp, Homo sapiens
gcccacagggactttggtccagcatctcagcactttctttccacgtctgtccagggtccctgggagagagccatctcgccaaacaaagtgccctactatatcaaccacgagactcaaacaacttgctgggaccatcccaaaatgacagagctctaccagtctttagctgacctgaataatgtcagattctcagcttataggactgccatgaaactc

SEQ ID NO: 46 - DNA, 888 bp, Homo sapiens
cgaagactgcagaaggccctttgcttggatctcttgagcctgtcagctgcatgtgatgccttggaccagcacaacctcaagcaaaatgaccagcccatggatatcctgcagattattaattgtttgaccactatttatgaccgcctggagcaagagcacaacaatttggtcaacgtccctctctgcgtggatatgtgtctgaactggctgctgaatgtttatgatacgggacgaacagggaggatccgtgtcctgtcttttaaaactggcatcatttccctgtgtaaagcacatttggaagacaagtacagataccttttcaagcaagtggcaagttcaacaggattttgtgaccagcgcaggctgggcctccttctgcatgattctatccaaattccaagacagttgggtgaagttgcatcctttgggggcagtaacattgagccaagtgtccggagctgcttccaatttgctaataataagccagagatcgaagcggccctcttcctagactggatgagactggaaccccagtccatggtgtggctgcccgtcctgcacagagtggctgctgcagaaactgccaagcatcaggccaaatgtaacatctgcaaagagtgtccaatcattggattcaggtacaggagtctaaagcactttaattatgacatctgccaaagctgctttttttctggtcgagttgcaaaaggccataaaatgcactatcccatggtggaatattgcactccgactacatcaggagaagatgttcgagactttgccaaggtactaaaaaacaaatttcgaaccaaaaggtattttgcgaagcatccccgaatgggctacctgccagtgcagactgtcttagagggggacaacatggaaact

SEQ ID NO: 47 - DNA, 834 bp, Homo sapiens
cccgttactctgatcaacttctggccagtagattctgcgcctgcctcgtcccctcagctttcacacgatgatactcattcacgcattgaacattatgctagcaggctagcagaaatggaaaacagcaatggatcttatctaaatgatagcatctctcctaatgagagcatagatgatgaacatttgttaatccagcattactgccaaagtttgaaccaggactcccccctgagccagcctcgtagtcctgcccagatcttgatttccttagagagtgaggaaagaggggagctagagagaatcctagcagatcttgaggaagaaaacaggaatctgcaagcagaatatgaccgtctaaagcagcagcacgaacataaaggcctgtccccactgccgtcccctcctgaaatgatgcccacctctccccagagtccccgggatgctgagctcattgctgaggccaagctactgcgtcaacacaaaggccgcctggaagccaggatgcaaatcctggaagaccacaataaacagctggagtcacagttacacaggctaaggcagctgctggagcaacccgaggcagaggccaaagtgaatggcacaacggtgtcctctccttctacctctctacagaggtccgacagcagtcagcctatgctgctccgagtggttggcagtcaaacttcggactccatgggtgaggaagatcttctcagtcctccccaggacacaagcacagggttagaggaggtgatggagcaactcaacaactccttccctagttcaagaggaagaaatacccctggaaagccaatgagagaggacacaatgtag

SEQ ID NO: 48 - DNA, 11044 bp, Canis familiaris
atgctttggtgggaagaagtagaggactgttatgaaagagaagatgttcaaaagaaaacattcacaaaatgggtaaatgcacagttttctaagtttgggaagcagcacatagagaacctcttcagtgacctacaggatgggagacgcctcctagaccttttggaaggcctgacagggcaaaaactgccaaaagaaaaaggatccacaagagttcatgccctgaacaatgtcaacaaggcactgcgcgtcttgcagaaaaataatgttgatttagtgaacattggaagtactgacatagtagatggaaatcacaaactgactcttggtttgatttggaatataatcctccactggcaggtcaaaaatgtaatgaaaaatatcatggctggattgcaacaaaccaacagtgaaaagattctcctgagctgggtccgacaatcaactcgtaattatccacaggttaatgtcattaacttcaccaccagctggtctgatggcctggctttgaacgctctcatccacagtcataggccagacctgtttgattggaatagtgtggtttgccagcagtcagccacacaacgcctggaacatgcattcaacattgccaaatatcaattaggcatagagaaactgcttgatcctgaagatgttgccaccacttatccagataagaagtccatcttaatgtatatcacatcactcttccaagttttgcctcaacaagtgagcattgaagccatccaggaagtggaaatgttgccaaggccatctcaagttactagagaagaacattttcagatacatcatcaaatgcactattctcaacagatcacagtcagtctagcacagggatatgaacgagccccttcctttcctaagcctcggttcaagagctatgcctacacacaggctgcttatgtcaccacttctgaccccacacggagcccacttccttcacagcatttggaaactcctgaagacaagtcatttggccggtcattgacagagaccgaagcaaacctggacagttatcaaacagctttggaagaagtactctcgtggcttctttcagctgaggatgcactgcaagcccaaggagagatttctaatgatgtcgaagaagtgaaagaacaatttcatactcatgagggatatatgatggacttgacatcccatcagggacgggtcggtaatgttctccaactgggaagtcaactgattggaacagggaaattatcagaagatgaagaaaccgaagtgcaggaacaaatgaatctcctcaattcaagatgggaatgcctcagggtagctagcatggaaaaacaaagcaatttacataaagttctaatggatctccagaatcagcaactgaaagagttaaatgactggctaaccaaaacagaagagagaacaaggaaaatggagaaggagccccttggacctgatattgaagacctaaaacgccaagtacaacaacataaggtgcttcaagaagacttagaacaggaacaagtcagggtcaattccctcactcatatggtggtggtagtcgatgaatctagtggagaccatgcaactgctgctttggaagaacaacttaaggtactgggagatcgatgggcaaacatctgtaggtggacagaagatcgctgggttcttttacaagacatcctcctaaaatggcagcgttttactgaagaacagtgcctttttagtgcatggctttcggagaaggaagatgcagtgaacaagattcacacaactggctttaaggatcaaagtgaagtgttatcaaatcttcagaaactggctgtcttaaaaacagatctggaaaagaagaagcaaaccatggacaaactctgctcactcaaccaagaccttctttcagcgctgaaaaacacagtggtagcccacaagatggaagcatggctggacaactttgcccagcgctgggataatttagtccagaaacttgaaaaaagttcagcacagatttcacaggctgtcaccaccactcagccatcactaacacagacaactgtaatggaaacagtaactatggtgaccacgagggaacacatcttggtaaagcatgcccaagaggaactgccaccaccaccccctcagaagaagaggcagattatcgtggattctgaaattaggaaaaggttggatgtcgatataactgaacttcacagttggattactcgttcagaagctgtgttgcagagtcctgaatttgcaatctatcggaaggaaggcaacttctcagaccttaaagaaaaagtcaatgccatagagcgagaaaaagccgagaagttcagaaaactgcaagatgccagcagatcagctcaggccctggtggaacagatggtgaatgagggtgttaatgctgacagcatcaaacaagcctccgaacaactgaacagccggtggatagagttctgccaattgctaagcgagagacttaactggctggagtatcagaacaacatcatcactttctataatcagctacaacaattggagcagatgacaactactgctgaaaactggttgaaaacccagcctaccaccacatcagagccaacagcaattaaaagccagttaaaaatttgtaaggatgaaatcaaccgactgtcagctcttcagcctcaaatcgagcgattaaaaattcaaagcatagccctgaaagagaaaggacaagggccaatgttcctggatgcagactttgtggcctttacaaatcattttaaccaagtctttgctgatgtgcaggcaagagaaaaagagctacaaacaatttttgacagtttgccacccatgcgctatcaggagactatgagtaccatcctgacatggatccagcagtcagaaaccaaactctctatacctcaggttactgtcactgaatatgacatcatggaacagagactcggagagctacaggctttacaaagctctctgcaagagcaacaaaatggcctaaactatctcagcaccactgtgaaagagatgtcaaagaaagcaccactgtctgatattagtcggaaatatcaatcagaatttgaagagattgagggacgttggaagaagctgtcttcccagctggttgaacattgtcaaaagttggaggagcaaatggctaaacttcgaaaaattcagaatcacataaaaactctgaagaaatggatcactgaagtcgatgttttcctgaaggaggaatggcctgcccttggggattcagaaattctgaaaagacagctgaaacagtgcaggcttttagtcaatgacattcagaccatccagcctagtctcaacagtgtcaatgaaggggctcagaagatgaagaatgaagcagaaccagagtttgctggcagacttgagacagagctccgagaacttaacacccagtgggattacatgtgccgccaggtctatgccaggaaggaagccttaaaaggaggttttggataaaactgtaagtcttcagaaagatctgtcagagatgcatgagtggatgacacaagctgaagaagaatacctagagagagatttcgaatacaagacccctgatgaattacagacagcagttgaagagatgaagagagctaaagaagaggcccagcaaaaagaagcaaaagtgaaactcctaaccgagtccgtcaatagtgtcatagctcaggctccacctgcagcacaagaggccttaaaaaaggaacttgacactctcaccaccaactaccagtggctctgcaccaggctcaatggcaaatgcaagaccttggaagaagtttgggcgtgctggcatgagttattgtcctacttggagaaggcaaacaagtggctaagtgaagtagaagtcaagcttaaaaccactgaaaatatttctgggggagctgaggaaatcgccgaggtgcttgattcgcttgaaaatttgatgcaacattcagaggataacccgaatcagattcgcatattggcacagaccttgacagatggtggagtcatggatgaactgatcaatgaggagcttgagacatttaattctcgttggagagaactccatgaagaggctgtgaggaggcaaaagttgcttgagcagagtatccagtcggcccaggagatagaaaaatccttgcacttaattcaggagtccctctcttccattgacaagcagttggcagcttatattgctgacaaagtggatgcagctcagatgcctcaggaagcccagaaaatccaatcagatttgacaagtcatgagatcagtttagaagaaatgaagaaacataaccagggaaaggagactgcccaaagggtactatcccaaattgatgtggcacagaaaaaattgcaggatgtttccatgaagtttcgattattccagaagccagccaattttgagcagcgcctacaagaaagtaaaatgattttagatgaagtgaagatgcatttacctgcgttggaaacaaagagtgtggaacaggaagtagtacagtcacagttaaatcattgtgtgaacttgtataaaagtctgagtgaagtgaagtctgaagtggaaatggtaataaaaactggacgtcagattgtacagaagaagcagacggaaaacccgaaagagcttgatgaaagagttacagctttgaaattgcattataatgagctgggagcaaaggtgacagaaagaaagcaacagttggaaaaatgcttgaaattgtcccgtaagatgcgaaaggaaatgaatgccctgacagaatggctggcagctacagatatggaactgacaaagagatcggcagttgaaggaatgcctagtaatttggattctgaagttgcctggggaaaggctactcagaaagagattgagaaacagaaggttcacctaaagagtgtcacagaggtaggagaggccttgaaaacggttttgggcaagaaggaaatgttggtggaagataaactgagtcttctgaatagtaactggatagccgtcacttcccgagcagaagagtggttaaaccttttattggaataccagaaacacatggaaacttttgaccagaatgtggattacatcacaaactggatcattcaggctgatgcacttttggatgaatctgagaaaaagaaacctcagcaaaaagaagacatacttaagcgtttaaaggctgaaatgaatgacatacgtccaaaggtggattctacacgtgaccaagcagcaaacctgatggcaaaccgcggcgaccactgcaggaaagtagtagagcccaaaatctcagagctcaaccatcgatttgcagccatttctcacagaattaagactggaaaggcctccattcctttgaaggaattggagcagtttaactcagatatacaaaaattgcttgaaccactggaggctgaaattcagcagggggtgaatctgaaagaggaagacttcaataaagatatgagtgaagacaatgagggtactgtaaaagaattgttgcaaagaggagacaacttacaacaaagaatcacagatgagagaaagcgagaggaaataaagataaaacaacagctgttacagacaaaacataatgctctcaaggatttgaggtctcaaagaagaaaaaaggctctagaaatttctcaccagtggtatcagtacaagaggcaggctgatgatctcctgaaatgcttggatgacattgaaaaaaaattagccagcctacctgaacccagagatgaaaggaaaataaaggaaattgatcgtgaattgcagaagaagaaagaggagctgaatgcagtgcgtaggcaagctgagggcttgtctgaggatggggccgcaatggcagtggagccaactcagatccagctcagcaagcgctggcgggaaattgagagcaaatttgctcagtttcgaagactcaactttgcacaaattcacactgtccatgaagagtcagtggtggcgatgactgaagacatgcctttggaaatttcttatgtgccttctacttacctgactgagatcactcatgtctcacaagccctatcagaagtggaagagcttcttaatgctcccgacctttgtgctcaagattttgaagatctctttaaacaagaggaatccttgaagaacataaaagacagcctgcaacaaatctcaggtcggattgacatcattcacaataaaaagacagcagcattgcacagtgccactcctgcagaaagggcaaagctccaggaagctctctcacggcttgatttccaatgggaaagagttaacaatatgtacaaggaccgacaagggagatttgacagatctgtggaaaaatggcggcggtttcattatgatatgaagatacttaatcaatggctaacagaagctgaacagtttctcaaaaagacacaaattcctgagaattgggaacatgccaaatacaaatggtatcttaaggaactccaggatggcattggacagcggcaaagtgttgtcagggtattgaatgcaactggggaagaaataattcaacagtcctcaaaaacagatgccagtattctccaagaaaaactgggaagcctgaatctgcggtggcaggaggtctgcaaacagctggcagaaagaaaaaagaggctagaggaacagaagaatatcttgtcagaatttcaaagagatgtaaatgaatttgttttatggttggaagaagcggataacgttgctaatattccacttgaacctggaaatgagcagcagctaaaagaaaaacttgaacaagtcaagttactggcagaagagttgcccctgcgccagggaattctaaaacaattaaatgaaactggaggaacagtgcttgtaagtgctcccctaagcccagaagagcaagataaacttgaaaataagctcaagcagacaaatcttcagtggataaaggtttctagaaatctgcctgagaagcaagaagaaattgaggcacacgtaaaagaccttggacagctggaagagcagttaaatcatctgcttctatggctgtctcctattaggaatcagttggaaatttacaatcagccaaatcaaacaggaccatttgacatcaaggaaattgaagtagcagttcaagctaaacagccggatgtggaagggattttgtctaaagggcagcatttgtacaaggaaaaaccagccactcagccagcgaagagaaagctggaagatctcagctctgattggaaggtggtaactcagttgcttcaagagctgcgggcaaagcaacctggcccagctcctggactgaccactgtcagagcccctcccagtcagactgttactctggtgacacaacccgcggttaccaaggaaactgccatctccaaactagaaatgccatcttcattgctgttggaggtacctgcactggcagatttcaaccgagcttggacagaacttaccgactggctgtctctgcttgatcgagttataaaatcacagagggtgatggtgggtgatcttgaagacattaacgagatgatcatcaagcagaaggcaacgctgcaggatttggaacagaggcgcccccagttggaagaactcattaccgctgcccagaatttgaaaaacaagaccagcaatcaagaggctagaacaatcattactgatcgaattgaaagaattcagagtcagtgggatgaagtacaggaacatcttcagaaccggaggctacagttgactgaaatgttaaaggattccacacaatggctggaagctaaagaggaggctgagcaggtgttggggcaggccagagccaagcttgagtcatggaaggaggctccctacacagtagatgcaatccaaaagaaaatcacagaaaccaagcagttggccaaagacctccgccagtggcagataaatgtagatgttgcaaatgatttggcactgaaacttctccgagattattctgcagatgataccagaaaagtacacatgataacagagaacatcaatgcctcttgggcaagcatccataaaagattgagtgagcgagaggctgctctggaagaaacccacagattactgcaacagttccccttggacctggagaagttccttgcctggcttacagaagccgaaacaactgccaacgtcctgcaggatgccacccataaggaaaggcttctagaagattccaagggagtaagagagctgatgaaacaatggcaagacctccaaggagaaatcgaagctcacacagatatctatcacaacctggacgaaaatggccaaaaagtcctgagatccctggaaggttctgacgatgcagccttgttgcaaagacgtttggataacatgaacttcaagtggagcgaacttcggaaaaagtctctcaacattaggtctcacttggaagccagttctgaccagtggaagcgtctgcacctttctcttcaggaacttctggtatggctccagctgaaagatgatgagttaagccggcaggcacccattggaggagactttccagcggtgcagaagcagaatgatgtacacagggccttcaagagggaattgaaaacgaaagaacctgtaatcatgagtactcttgagactgtacgaatatttctgacagagcagcctttagaaggactagagaaactctaccaggagcccagagagctgcctcctgaagagagagcccagaatgtcacacggctcctacgaaagcaagctgaggaggtcaacactcagtgggaaaaactgaacgtgcactctgcagactggcagagaaaaatagacgaggccctcgaaagactccaggagcttcaggaagcaacagatgagctggatctcaaactacgtcaggcagaggtgatcaaaggatcctggcagcctgtgggtgacctcctcattgactctctccaagatcacctcgaaaaagtcaaggcgcttcgaggagaaattacacctctgaaagagaatgtcagctacgtcaatgaccttgctcgccaactcactacgttgggcattcagctgtcaccatataacctcaacactctggaagacctgaacaccagatggaagcttctgcaggtggccattgaggaccgcatcaggcagctgcatgaagcgcacagggactttggaccagcctcccagcacttcctttccacttctgtccagggtccctgggagagagccatctcaccaaacaaagtgccctactatatcaaccacgagacccaaacaacttgctgggaccatcccaaaatgacagagctctaccagtctttagctgacctgaataatgtcaggttctcagcttacaggactgccatgaaactccgaagactgcagaaggccctttgcttggatctcttgagcctatcggctgcatgcgatgccttggaccagcacaacctcaagcaaaatgaccagcccatggatatcctgcaggtcattaactgtctgaccactatttatgatcgcctagagcaagagcacaacaatctggtcaacgtccctctctgcgtggatatgtgtctcaattggctgctgaatgtttatgacacgggacgaacggggaggatccgggtcctgtcttttaaaactggcatcatttctctgtgtaaagcccatttggaagacaagtacagatacctcttcaagcaagtggcaagttcgacaggattttgtgaccagcgcaggctgggcctcctcctgcatgactctatccagatcccaagacagttgggtgaagtcgcatcgttcgggggcagtaacattgagccgagtgtcaggagctgcttccagtttgctaataataagcctgagatcgaagcggccctcttcctagactggatgcgcctggagccccagtccatggtgtggctgcctgtcctgcaccgagtggctgccgcggaaactgccaagcaccaggccaagtgcaacatctgcaaggagtgtcccatcatcggattcaggtacaggagtctaaagcactttaattatgacatctggcaaagttgctttttttctggtcgagttgcaaaaggccataaaatgcactatcccatggtggaatactgcactccgactacatcgggagaagatgtccgtgactttgccaaggtactaaaaaacaaatttcgaaccaaaaggtattttgcgaagcatccccgaatgggctacctgccagtgcagactgtcttagagggggacaacatggaaactcctgtcactctgatcaacttctggccggtagattctgcgcctgcctcgtcccctcagctttcacacgatgatactcattcacgcattgagcattatgctagcaggctaaaaaaaatggaaaacagcaatggatcttatctaaatgatagcatctctcctaatgagagcatagatgatgaacatttgttaatccagcattactggcgaagtttgaaccaggaatcccccctgagccagcctcgtagtcctgcccagatcttgatttccttagagagtgaggaaagaggggagctagagagaatcctagcagatcttgaggggagaaacagaaatctgcaagcagagtatgatcgtctaaagcagcagcatgaacacaaaggcctgtccccactgccatcccctcctgaaatgatgcctacttctccccaaagtccccgggatgctgagctcatcgctgaggccaagctgctgcgtcaacacaaaggccgcctggaagccaggatgcaaatccttgaagaccataacaaacaactggaatcccagttacacaggctcaggcagctgctggagcaaccccaggcagaggccaaggtgaatggtacaacggtgtcttctccttctacctctcttcagaggtcagatagcagtcagcctatgctgctccgggtggtcggcagtcagacttcagaatccatgggcgaggaagacctgctcagccctccccaggacacaagcacagggttagaggaagtgatggagcagctcaaccactccttccctagttccagaggaagaaatacccctgggaagccaatgagagaggacacaatgtag

SEQ ID NO: 49 - protein, 3680 aa, Canis familiaris
MLWWEEVEDCYEREDVQKKTFTKWVNAQFSKFGKQHIENLFSDLQDGRRLLDLLEGLTGQKLPKEKGSTRVHALNNVNKALRVLQKNNVDLVNIGSTDIVDGNHKLTLGLIWNIILHWQVKNVMKNIMAGLQQTNSEKILLSWVRQSTRNYPQVNVINFTTSWSDGLALNALIHSHRPDLFDWNSVVCQQSATQRLEHAFNIAKYQLGIEKLLDPEDVATTYPDKKSILMYITSLFQVLPQQVSIEAIQEVEMLPRPSQVTREEHFQIHHQMHYSQQITVSLAQGYERAPSFPKPRFKSYAYTQAAYVTTSDPTRSPLPSQHLETPEDKSFGRSLTETEANLDSYQTALEEVLSWLLSAEDALQAQGEISNDVEEVKEQFHTHEGYMMDLTSHQGRVGNVLQLGSQLIGTGKLSEDEETEVQEQMNLLNSRWECLRVASMEKQSNLHKVLMDLQNQQLKELNDWLTKTEERTRKMEKEPLGPDIEDLKRQVQQHKVLQEDLEQEQVRVNSLTHMVVVVDESSGDHATAALEEQLKVLGDRWANICRWTEDRWVLLQDILLKWQRFTEEQCLFSAWLSEKEDAVNKIHTTGFKDQSEVLSNLQKLAVLKTDLEKKKQTMDKLCSLNQDLLSALKNTVVAHKMEAWLDNFAQRWDNLVQKLEKSSAQISQAVTTTQPSLTQTTVMETVTMVTTREHILVKHAQEELPPPPPQKKRQIIVDSEIRKRLDVDITELHSWITRSEAVLQSPEFAIYRKEGNFSDLKEKVNAIEREKAEKFRKLQDASRSAQALVEQMVNEGVNADSIKQASEQLNSRWIEFCQLLSERLNWLEYQNNIITFYNQLQQLEQMTTTAENWLKTQPTTTSEPTAIKSQLKICKDEINRLSALQPQIERLKIQSIALKEKGQGPMFLDADFVAFTNHFNQVFADVQAREKELQTIFDSLPPMRYQETMSTILTWIQQSETKLSIPQVTVTEYDIMEQRLGELQALQSSLQEQQNGLNYLSTTVKEMSKKAPLSDISRKYQSEFEEIEGRWKKLSSQLVEHCQKLEEQMAKLRKIQNHIKTLKKWITEVDVFLKEEWPALGDSEILKRQLKQCRLLVNDIQTIQPSLNSVNEGAQKMKNEAEPEFAGRLETELRELNTQWDYMCRQVYARKEALKGGLDKTVSLQKDLSEMHEWMTQAEEEYLERDFEYKTPDELQTAVEEMKRAKEEAQQKEAKVKLLTESVNSVIAQAPPAAQEALKKELDTLTTNYQWLCTRLNGKCKTLEEVWACWHELLSYLEKANKWLSEVEVKLKTTENISGGAEEIAEVLDSLENLMQHSEDNPNQIRILAQTLTDGGVMDELINEELETFNSRWRELHEEAVRRQKLLEQSIQSAQEIEKSLHLIQESLSSIDKQLAAYIADKVDAAQMPQEAQKIQSDLTSHEISLEEMKKHNQGKETAQRVLSQIDVAQKKLQDVSMKFRLFQKPANFEQRLQESKMILDEVKMHLPALETKSVEQEVVQSQLNHCVNLYKSLSEVKSEVEMVIKTGRQIVQKKQTENPKELDERVTALKLHYNELGAKVTERKQQLEKCLKLSRKMRKEMNALTEWLAATDMELTKRSAVEGMPSNLDSEVAWGKATQKEIEKQKVHLKSVTEVGEALKTVLGKKEMLVEDKLSLLNSNWIAVTSRAEEWLNLLLEYQKHMETFDQNVDYITNWIIQADALLDESEKKKPQQKEDILKRLKAEMNDIRPKVDSTRDQAANLMANRGDHCRKVVEPKISELNHRFAAISHRIKTGKASIPLKELEQFNSDIQKLLEPLEAEIQQGVNLKEEDFNKDMSEDNEGTVKELLQRGDNLQQRITDERKREEIKIKQQLLQTKHNALKDLRSQRRKKALEISHQWYQYKRQADDLLKCLDDIEKKLASLPEPRDERKIKEIDRELQKKKEELNAVRRQAEGLSEDGAAMAVEPTQIQLSKRWREIESKFAQFRRLNFAQIHTVHEESVVAMTEDMPLEISYVPSTYLTEITHVSQALSEVEELLNAPDLCAQDFEDLFKQEESLKNIKDSLQQISGRIDIIHNKKTAALHSATPAERAKLQEALSRLDFQWERVNNMYKDRQGRFDRSVEKWRRFHYDMKILNQWLTEAEQFLKKTQIPENWEHAKYKWYLKELQDGIGQRQSVVRVLNATGEEIIQQSSKTDASILQEKLGSLNLRWQEVCKQLAERKKRLEEQKNILSEFQRDVNEFVLWLEEADNVANIPLEPGNEQQLKEKLEQVKLLAEELPLRQGILKQLNETGGTVLVSAPLSPEEQDKLENKLKQTNLQWIKVSRNLPEKQEEIEAHVKDLGQLEEQLNHLLLWLSPIRNQLEIYNQPNQTGPFDIKEIEVAVQAKQPDVEGILSKGQHLYKEKPATQPAKRKLEDLSSDWKVVTQLLQELRAKQPGPAPGLTTVRAPPSQTVTLVTQPAVTKETAISKLEMPSSLLLEVPALADFNRAWTELTDWLSLLDRVIKSQRVMVGDLEDINEMIIKQKATLQDLEQRRPQLEELITAAQNLKNKTSNQEARTIITDRIERIQSQWDEVQEHLQNRRLQLTEMLKDSTQWLEAKEEAEQVLGQARAKLESWKEAPYTVDAIQKKITETKQLAKDLRQWQINVDVANDLALKLLRDYSADDTRKVHMITENINASWASIHKRLSEREAALEETHRLLQQFPLDLEKFLAWLTEAETTANVLQDATHKERLLEDSKGVRELMKQWQDLQGEIEAHTDIYHNLDENGQKVLRSLEGSDDAALLQRRLDNMNFKWSELRKKSLNIRSHLEASSDQWKRLHLSLQELLVWLQLKDDELSRQAPIGGDFPAVQKQNDVHRAFKRELKTKEPVIMSTLETVRIFLTEQPLEGLEKLYQEPRELPPEERAQNVTRLLRKQAEEVNTQWEKLNVHSADWQRKIDEALERLQELQEATDELDLKLRQAEVIKGSWQPVGDLLIDSLQDHLEKVKALRGEITPLKENVSYVNDLARQLTTLGIQLSPYNLNTLEDLNTRWKLLQVAIEDRIRQLHEAHRDFGPASQHFLSTSVQGPWERAISPNKVPYYINHETQTTCWDHPKMTELYQSLADLNNVRFSAYRTAMKLRRLQKAICLDLLSLSAACDALDQHNLKQNDQPNDILQVINCLTTIYDRLEQEHNNLVNVPLCVDMCLNWLLNVYDTGRTGRIRVLSFKTGIISLCKAHLEDKYRYLFKQVASSTGFCDQRRLGLLLHDSIQIPRQLGEVASFGGSNIEPSVRSCFQFANNKPEIEAALFLDWMRLEPQSMVWLPVLHRVAAAETAKHQAKCNICKECPIIGFRYRSLKHFNYDICQSCFFSGRVAKGHKMHYPMVEYCTPTTSGEDVRDFAKVLKNKFRTKRYFAKHPRMGYLPVQTVLEGDNMETPVTLINFWPVDSAPASSPQLSHDDTHSRIEHYASRLKKMENSNGSYLNDSISPNESIDDEHLLIQHYWRSLNQESPLSQPRSPAQILISLESEERGELERILADLEGRNRNLQAEYDRLKQQHEHKGLSPLPSPPEMMPTSPQSPRDAELIAEAKLLRQHKGRLEARMQILEDHNKQLESQLHRLRQLLEQPQAEAKVNGTTVSSPSTSLQRSDSSQPMLLRVVGSQTSESMGEEDLLSPPQDTSTGLEEVMEQLNHSFPSSRGRNTPGKPMREDTM

SEQ ID NO: 50 - protein, 251 aa, Homo sapiens
MLWWEEVEDCYEREDVQKKTFTKWVNAQFSKFGKQHIENLFSDLQDGRRLLDLLEGLTGQKLPKEKGSTRVHALNNVNKALRVLQNNNVDLVNIGSTDIVDGNHKLTLGLIWNIILHWQVKVMKNIMAGLQQTNSEKILLSWVRQSTRNYPQVNVINFTTSWSDGLALNALIHSHRPDLFDWNSVVCQQSATQRLEHAFNIARYQLGIEKLLDPEDVDTTYPDKKSILMYITSLFQVLPQQVSIEAIQEVE

SEQ ID NO: 51 - protein, 2860 aa, Homo sapiens
MLPRPPKVTKEEHFQLHHQMHYSQQITVSLAQGYERTSSPKPRFKSYAYTQAAYVTTSDPTRSPFPSQHLEAPEDKSFGSSLMESEVNLDRYQTALEEVLSWLLSAEDTLQAQGEISNDVEVVKDQFHTHEGYMMDLTAHQGRVGNILQLGSKLIGTGKLSEDEETEVQEQMNLLNSRWECLRVASMEKQSNLHRVLMDLQNQKLKELNDWLTKTEERTRKMEEEPLGPDLEDLKRQVQQHKVLQEDLEQEQVRVNSLTHMVVVVDESSGDHATAALEEQLKVLGDRWANICRWTEDRWVLLQDILLKWQRLTEEQCLFSAWLSEKEDAVNKIHTTGFKDQNEMLSSLQKLAVLKADLEKKKQSMGKLYSLKQDLLSTLKNKSVTQKTEAWLDNFARCWDNLVQKLEKSTAQISQAVTTTQPSLTQTTVMETVTTVTTREQILVKHAQEELPPPPPQKKRQITVDSEIRKRLDVDITELHSWITRSEAVLQSPEFAIFRKEGNFSDLKEKVNAIEREKAEKFRKLQDASRSAQALVEQMVNEGVNADSIKQASEQLNSRWIEFCQLLSERLNWLEYQNNIIAFYNQLQQLEQMTTTAENWLKIQPTTPSEPTAIKSQLKICKDEVNRLSGLQPQIERLKIQSIALKEKGQGPMFLDADFVAFTNHFKQVFSDVQAREKELQTIFDTLPPMRYQETMSAIRTWVQQSETKLSIPQLSVTDYEIMEQRLGELQALQSSLQEQQSGLYYLSTTVKEMSKKAPSEISRKYQSEFEEIEGRWKKLSSQLVEHCQKLEEQMNKLRKIQNHIQTLKKWMAEVDVFLKEEWPALGDSEILKKQLKQCRLLVSDIQTIQPSLNSVNEGGQKIKNEAEPEFASRLETELKELNTQWDHMCQQVYARKEALKGGLEKTVSLQKDLSEMHEWMTQAEEEYLERDFEYKTPDELQKAVEEMKRAKEEAQQKEAKVKLLTESVNSVIAQAPPVAQEALKKELETLTTNYQWLCTRLNGKCKTLEEVWACWHELLSYLEKANKWLNEVEFKLKTTENIPGGAEEISEVLDSLENLMRHSEDNPNQIRILAQTLTDGGVMDELINEELETFNSRWRELHEEAVRRQKLLEQSIQSAQETEKSLHLIQESLTFIDKQLAAYIADKVDAAQMPQEAQKIQSDLTSHEISLEEMKKHNQGKEAAQRVLSQIDVAQKKLQDVSMKFRLFQKPANFELRLQESKMILDEVKMHLPALETKSVEQEVVQSQLNHCVNLYKSLSEVKSEVEMVIKTGRQIVQKKQTENPKELDERVTALKLHYNELGAKVTERKQQLEKCLKLSRKMRKEMNVLTEWLAATDMELTKRSAVEGMPSNLDSEVAWGKATQKEIEKQKVHLKSITEVGEALKTVLGKKETLVEDKLSLLNSNWIAVTSRAEEWLNLLLEYQKHMETFDQNVDHITKWIIQADTLLDESEKKKPQQKEDVLKRLKAELNDIRPKVDSTRDQAANLMANRGDHCRKLVEPQISELNHRFAAISHRIKTGKASIPLKELEQFNSDIQKLLEPLEAEIQQGVNLKEEDFNKDMNEDNEGTVKELLQRGDNLQQRITDERKREEIKIKQQLLQTKHNALKDLRSQRRKKALEISHQWYQYKRQADDLLKCLDDIEKKLASLPEPRDERKIKEIDRELQKKKEELNAVRRQAEGLSEDGAAMAVEPTQIQLSKRWREIESKFAQFRRLNFAQIHTVREETMMVMTEDMPLEISYVPSTYLTEITHVSQALLEVEQLLNAPDLCAKDFEDLFKQEESLKNIKDSLQQSSGRIDIIHSKKTAALQSATPVERVKLQEALSQLDFQWEKVNKMYKDRQGRFDRSVEKWRRFHYDIKIFNQWLTEAEQFLRKTQIPENWEHAKYKWYLKELQDGIGQRQTVVRTLNATGEEIIQQSSKTDASILQEKLGSLNLRWQEVCKQLSDRKKRLEEQKNILSEFQRDLNEFVLWLEEADNIASIPLEPGKEQQLKEKLEQVKLLVEELPLRQGILKQLNETGGPVLVSAPISPEEQDKLENKLKQTNLQWIKVSRALPEKQGEIEAQIKDLGQLEKKLEDLEEQLNHLLLWLSPIRNQLEIYNQPNQEGPFDVQETEIAVQAKQPDVEEILSKGQHLYKEKPATQPVKRKLEDLSSEWKAVNRLLQELRAKQPDLAPGLTTIGASPTQTVTLVTQPVVTKETAISKLEMPSSLMLEVPALADFNRAWTELTDWLSLLDQVIKSQRVMVGDLEDINEMIIKQKATMQDLEQRRPQLEELITAAQNLKNKTSNQEARTIITDRIERIQNQWDEVQEHLQNRRQQLNEMLKDSTQWLEAKEEAEQVLGQARAKLESWKEGPYTVDAIQKKITETKQLAKDLRQWQTNVDVANDLALKLLRDYSADDTRKVHMITENINASWRSIHKRVSEREAALEETHRLLQQFPLDLEKFLAWLTEAETTANVLQDATRKERLLEDSKGVKELMKQWQDLQGEIEAHTDVYHNLDENSQKILRSLEGSDDAVLLQRRLDNMNFKWSELRKKSLNIRSHLEASSDQWKRLHLSLQELLVWLQLKDDELSRQAPIGGDFPAVQKQNDVHRAFKRELKTKEPVIMSTLETVRIFLTEQPLEGLEKLYQEPRELPPEERAQNVTRLLRKQAEEVNTEWEKLNLHSADWQRKIDETLERLQELQEATDELDLKLRQAEVIKGSWQPVGDLLIDSLQDHLEKVKALRGEIAPLKENVSHVNDLARQLTTLGIQLSPYNLSTLEDLNTRWKLLQVAVEDRVRQLHEAHRDFGPASQHFLSTSVQGPWERAISPNKVPYYINHETQTTCWDHPKMTELYQSLADLNNVRFSAYRTAMKL

SEQ ID NO: 52 - protein, 296 aa, Homo sapiens
RRLQKALCLDLLSLSAACDALDQHNLKQNDQPMDILQIINCLTTIYDRLEQEHNNLVNVPLCVDMCLNWLLNVYDTGRTGRIRVLSFKTGIISLCKAHLEDKYRYLFKQVASSTGFCDQRRLGLLLHDSIQIPRQLGEVASFGGSNIEPSVRSCFQFANNKPEIEAALFLDWMRLEPQSMVWLPVLHRVAAAETAKHQAKCNICKECPIIGFRYRSLKHFNYDICQSCFFSGRVAKGHKMHYPMVEYCTPTTSGEDVRDFAKVLKNKFRTKRYFAKHPRMGYLPVQTVLEGDNMET

SEQ ID NO: 53 - protein, 277 aa, Homo sapiens
PVTLINFWPVDSAPASSPQLSHDDTHSRIEHYASRLAEMENSNGSYLNDSISPNESIDDEHLLIQHYCQSLNQDSPLSQPRSPAQILISLESEERGELERILADLEEENRNLQAEYDRLKQQHEHKGLSPLPSPPEMMPTSPQSPRDAELIAEAKLLRQHKGRLEARMQILEDHNKQLESQLHRLRQLLEQPQAEAKVNGTTVSSPSTSLQRSDSSQPMLLRVVGSQTSDSMGEEDLLSPPQDTSTGLEEVMEQLNNSFPSSRGRNTPGKPMREDTM

SEQ ID NO: 54 - protein, 15 aa, Homo sapiens
LLNSRWECLRVASME

SEQ ID NO: 55 - protein, 15 aa, Homo sapiens
QRLTEEQCLFSAWLS

SEQ ID NO: 56 - protein, 15 aa, Homo sapiens
WLDNFARCWDNLVQK

SEQ ID NO: 57 - protein, 8 aa, Homo sapiens
CLKLSRKM

SEQ ID NO: 58 - protein, 110 aa, Homo sapiens
EISYVPSTYLTEITHVSQALLEVEQLLNAPDLCAKDFEDLFKQEESLKNIKDSLQQSSGRIDIIHSKKTAALQSATPVERVKLQEALSQLDFQWEKVNKMYKDRQGRFDR

SEQ ID NO: 59 - protein, 21 aa, Homo sapiens
PSTYLTEITHVSQALLEVEQL

SEQ ID NO: 60 - protein, 309 aa, Homo sapiens
SIQSAQETEKSLHLIQESLTFIDKQLAAYIADKVDAAQMPQEAQKIQSDLTSHEISLEEMKKHNQGKEAAQRVLSQIDVAQKKLQDVSMKFRLFQKPANFELRLQESKMILDEVKMHLPALETKSVEQEVVQSQLNHCVNLYKSLSEVKSEVEMVIKTGRQIVQKKQTENPKELDERVTALKLHYNELGAKVTERKQQLEKCLKLSRKMRKEMNVLTEWLAATDMELTKRSAVEGMPSNLDSEVAWGKATQKEIEKQKVHLKSITEVGEALKTVLGKKETLVEDKLSLLNSNWIAVTSRAEEWLNLLLE

SEQ ID NO: 61 - protein, 331 aa, Homo sapiens
SEVNLDRYQTALEEVLSWLLSAEDTLQAQGEISNDVEVVKDQFHTHEGYMMDLTAHQGRVGNILQLGSKLIGTGKLSEDEETEVQEQMNLLNSRWECLRVASMEKQSNLHRVLMDLQNQKLKELNDWLTKTEERTRKMEEEPLGPDLEDLKRQVQQHKVLQEDLEQEQVRVNSLTHMVVVVDESSGDHATAALEEQLKVLGDRWANICRWTEDRWVLLQDILLKWQRLTEEQCLFSAWLSEKEDAVNKIHTTGFKDQNEMLSSLQKLAVLKADLEKKKQSMGKLYSLKQDLLSTLKNKSVTQKTEAWLDNFARCWDNLVQKLEKSTAQISQ

SEQ ID NO: 62 - protein, 4 aa, Homo sapiens
GGSG

SEQ ID NO: 63 - protein, 4 aa, Homo sapiens
GGGS

SEQ ID NO: 64 - protein, 5 aa, Homo sapiens
GGGGS

SEQ ID NO: 65 - protein, 4 aa, Homo sapiens
GSAT

SEQ ID NO: 66 - protein, 96 aa, Mus musculus
LLLQRRRVTVRKADAGGLGISIKGGRENKMPILISKIFKGLAADQTEALFVGDAILSVNGEDLSSATHDEAVQALKKTGKEVVLEVKYMKEVSPYF

SEQ ID NO: 67 - protein, 96 aa, Homo sapiens
LLLQRRRVTVRKADAGGLGISIKGGRENKMPILISKIFKGLAADQTEALFVGDAILSVNGEDLSSATHDEAVQVLKKTGKEVVLEVKYMKDVSPYF